European Patent Application EP 4 166 667 A2, published April 19, 2023. Title: COMPOSITIONS FOR MODULATING C9ORF72 EXPRESSION. Applicant: Ionis Pharmaceuticals, Inc. Application EP. The sequence listing filed with the application follows.

SEQUENCE LISTING (1548 sequences)

SEQ ID NO: 1 - RNA, 3339 nt, Homo sapiens
  source 1..3339: mol_type = mRNA
acgtaacctacggtgtcccgctaggaaagagaggtgcgtcaaacagcgacaagttccgcccacgtaaaagatgacgcttggtgtgtcagccgtccctgctgcccggttgcttctcttttgggggcggggtctagcaagagcaggtgtgggtttaggagatatctccggagcatttggataatgtgacagttggaatgcagtgatgtcgactctttgcccaccgccatctccagctgttgccaagacagagattgctttaagtggcaaatcacctttattagcagctacttttgcttactgggacaatattcttggtcctagagtaaggcacatttgggctccaaagacagaacaggtacttctcagtgatggagaaataacttttcttgccaaccacactctaaatggagaaatccttcgaaatgcagagagtggtgctatagatgtaaagttttttgtcttgtctgaaaagggagtgattattgtttcattaatctttgatggaaactggaatggggatcgcagcacatatggactatcaattatacttccacagacagaacttagtttctacctcccacttcatagagtgtgtgttgatagattaacacatataatccggaaaggaagaatatggatgcataaggaaagacaagaaaatgtccagaagattatcttagaaggcacagagagaatggaagatcagggtcagagtattattccaatgcttactggagaagtgattcctgtaatggaactgctttcatctatgaaatcacacagtgttcctgaagaaatagatatagctgatacagtactcaatgatgatgatattggtgacagctgtcatgaaggctttcttctcaatgccatcagctcacacttgcaaacctgtggctgttccgttgtagtaggtagcagtgcagagaaagtaaataagatagtcagaacattatgcctttttctgactccagcagagagaaaatgctccaggttatgtgaagcagaatcatcatttaaatatgagtcagggctctttgtacaaggcctgctaaaggattcaactggaagctttgtgctgcctttccggcaagtcatgtatgctccatatcccaccacacacatagatgtggatgtcaatactgtgaagcagatgccaccctgtcatgaacatatttataatcagcgtagatacatgagatccgagctgacagccttctggagagccacttcagaagaagacatggctcaggatacgatcatctacactgacgaaagctttactcctgatttgaatatttttcaagatgtcttacacagagacactctagtgaaagccttcctggatcaggtctttcagctgaaacctggcttatctctcagaagtactttccttgcacagtttctacttgtccttcacagaaaagccttgacactaataaaatatatagaagacgatacgcagaagggaaaaaagccctttaaatctcttcggaacctgaagatagaccttgatttaacagcagagggcgatcttaacataataatggctctggctgagaaaattaaaccaggcctacactcttttatctttggaagacctttctacactagtgtgcaagaacgagatgttctaatgactttttaaatgtgtaacttaataagcctattccatcacaatcatgatcgctggtaaagtagctcagtggtgtggggaaacgttcccctggatcatactccagaattctgctctcagcaattgcagttaagtaagttacactacagttctcacaagagcctgtgaggggatgtcaggtgcatcattacattgggtgtctcttttcctagatttatgcttttgggatacagacctatgtttacaatataataaatattattgctatcttttaaagatataataataggatgtaaacttgaccacaactactgtttttttgaaatacatgattcatggtttacatgtgtcaaggtgaaatctgagttggcttttacagatagttgactttctatcttttggcattctttggtgtgtagaattactgtaatacttctgcaatcaactgaaaactagagcctttaaatgatttcaattccacagaaagaaagtgagcttgaacataggatgagctttagaaagaaaattgatcaagcagatgtttaattggaattgattattagatcctactttgtggatttagtccctgggattcagtctgtagaaatgtctaatagttctctatagtccttgttcctggtgaaccacagttagggtgttttgtttattttattgttcttgctattgttgatattctatgtagttgagctctgtaaaaggaaattgtattttatgttttagtaattgttgccaactttttaaattaattttcattatttttgagccaaattgaaatgtgcacctcctgtgccttttttctccttagaaaatctaattacttggaacaagttcagatttcactggtcagtcattttcatcttgttttcttcttgctaagtcttaccatgtacctgctttggcaatcattgcaactctgagattataaaatgccttagagaatatactaactaataagatctttttttcagaaacagaaaatagttccttgagtacttccttcttgcatttctgcctatgtttttgaagttgttgctgtttgcctgcaataggctataaggaatagcaggagaaattttactgaagtgctgttttcctaggtgctactttggcagagctaagttatcttttgttttcttaatgcgtttggaccattttgctggctataaaataactgattaatataattctaacacaatgttgacattgtagttacacaaacacaaataaatattttatttaaaattctggaagtaatataaaagggaaaatatatttataagaaagggataaaggtaatagagcccttctgccccccacccaccaaatttacacaacaaaatgacatgttcgaatgtgaaaggtcataatagctttcccatcatgaatcagaaagatgtggacagcttgatgttttagacaaccactgaactagatgactgttgtactgtagctcagtcatttaaaaaatatataaatactaccttgtagtgtcccatactgtgttttttacatggtagattcttatttaagtgctaactggttattttctttggctggtttattgtactgttatacagaatgtaagttgtacagtgaaataagttattaaagcatgtgtaaacattgttatatatcttttctcctaaatggagaattttgaataaaatatatttgaaattttg

SEQ ID NO: 2 - DNA, 30001 bp, Homo sapiens
  source 1..30001: mol_type = genomic DNA
caaagaaaagggggaggttttgttaaaaaagagaaatgttacatagtgctctttgagaaaattcattggcactattaaggatctgaggagctggtgagtttcaactggtgagtgatggtggtagataaaattagagctgcagcaggtcattttagcaactattagataaaactggtctcaggtcacaacgggcagttgcagcagctggacttggagagaattacactgtgggagcagtgtcatttgtcctaagtgcttttctaccccctacccccactattttagttgggtataaaaagaatgacccaatttgtatgatcaactttcacaaagcatagaacagtaggaaaagggtctgtttctgcagaaggtgtagacgttgagagccattttgtgtatttattcctccctttcttcctcggtgaatgattaaaacgttctgtgtgatttttagtgatgaaaaagattaaatgctactcactgtagtaagtgccatctcacacttgcagatcaaaaggcacacagtttaaaaaacctttgtttttttacacatctgagtggtgtaaatgctactcatctgtagtaagtggaatctatacacctgcagaccaaaagacgcaaggtttcaaaaatctttgtgttttttacacatcaaacagaatggtacgtttttcaaaagttaaaaaaaaacaactcatccacatattgcaactagcaaaaatgacattccccagtgtgaaaatcatgcttgagagaattcttacatgtaaaggcaaaattgcgatgactttgcaggggaccgtgggattcccgcccgcagtgccggagctgtcccctaccagggtttgcagtggagttttgaatgcacttaacagtgtcttacggtaaaaacaaaatttcatccaccaattatgtgttgagcgcccactgcctaccaagcacaaacaaaaccattcaaaaccacgaaatcgtcttcactttctccagatccagcagcctcccctattaaggttcgcacacgctattgcgccaacgctcctccagagcgggtcttaagataaaagaacaggacaagttgccccgccccatttcgctagcctcgtgagaaaacgtcatcgcacatagaaaacagacagacgtaacctacggtgtcccgctaggaaagagaggtgcgtcaaacagcgacaagttccgcccacgtaaaagatgacgcttggtgtgtcagccgtccctgctgcccggttgcttctcttttgggggcggggtctagcaagagcaggtgtgggtttaggaggtgtgtgtttttgtttttcccaccctctctccccactacttgctctcacagtactcgctgagggtgaacaagaaaagacctgataaagattaaccagaagaaaacaaggagggaaacaaccgcagcctgtagcaagctctggaactcaggagtcgcgcgctaggggccggggccggggccggggcgtggtcggggcgggcccgggggcgggcccggggcggggctgcggttgcggtgcctgcgcccgcggcggcggaggcgcaggcggtggcgagtgggtgagtgaggaggcggcatcctggcgggtggctgtttggggttcggctgccgggaagaggcgcgggtagaagcgggggctctcctcagagctcgacgcatttttactttccctctcatttctctgaccgaagctgggtgtcgggctttcgcctctagcgactggtggaattgcctgcatccgggccccgggcttcccggcggcggcggcggcggcggcggcgcagggacaagggatggggatctggcctcttccttgctttcccgccctcagtacccgagctgtctccttcccggggacccgctgggagcgctgccgctgcgggctcgagaaaagggagcctcgggtactgagaggcctcgcctgggggaaggccggagggtgggcggcgcgcggcttctgcggaccaagtcggggttcgctaggaacccgagacggtccctgccggcgaggagatcatgcgggatgagatgggggtgtggagacgcctgcacaatttcagcccaagcttctagagagtggtgatgacttgcatatgagggcagcaatgcaagtcggtgtgctccccattctgtgggacatgacctggttgcttcacagctccgagatgacacagacttgcttaaaggaagtgactattgtgacttgggcatcacttgactgatggtaatcagttgtctaaagaagtgcacagattacatgtccgtgtgctcattgggtctatctggccgcgttgaacaccaccaggctttgtattcagaaacaggagggaggtcctgcactttcccaggaggggtggccctttcagatgcaatcgagattgttaggctctgggagagtagttgcctggttgtggcagttggtaaatttctattcaaacagttgccatgcaccagttgttcacaacaagggtacgtaatctgtctggcattacttctacttttgtacaaaggatcaaaaaaaaaaaagatactgttaagatatgatttttctcagactttgggaaacttttaacataatctgtgaatatcacagaaacaagactatcatataggggatattaataacctggagtcagaatacttgaaatacggtgtcatttgacacgggcattgttgtcaccacctctgccaaggcctgccactttaggaaaaccctgaatcagttggaaactgctacatgctgatagtacatctgaaacaagaacgagagtaattaccacattccagattgttcactaagccagcatttacctgctccaggaaaaaattacaagcaccttatgaagttgataaaatattttgtttggctatgttggcactccacaatttgctttcagagaaacaaagtaaaccaaggaggacttctgtttttcaagtctgccctcgggttctattctacgttaattagatagttcccaggaggactaggttagcctacctattgtctgagaaacttggaactgtgagaaatggccagatagtgatatgaacttcaccttccagtcttccctgatgttgaagattgagaaagtgttgtgaactttctggtactgtaaacagttcactgtccttgaagtggtcctgggcagctcctgttgtggaaagtggacggtttaggatcctgcttctctttgggctgggagaaaataaacagcatggttacaagtattgagagccaggttggagaaggtggcttacacctgtaatgccagagctttgggaggcggaggcaagaggatcacttgaagccaggagttcaagctcaacctgggcaacgtagaccctgtctctacaaaaaattaaaaacttagccgggcgtggtgatgtgcacctgtagtcctagctacttgggaggctgaggcaggagggtcatttgagcccaagagtttgaagttaccgagagctatgatcctgccagtgcattccagcctggatgacaaaacgagaccctgtctctaaaaaacaagaagtgagggctttatgattgtagaattttcactacaatagcagtggaccaaccacctttctaaataccaatcagggaagagatggttgattttttaacagacgtttaaagaaaaagcaaaacctcaaacttagcactctactaacagttttagcagatgttaattaatgtaatcatgtctgcatgtatgggattatttccagaaagtgtattgggaaacctctcatgaaccctgtgagcaagccaccgtctcactcaatttgaatcttggcttccctcaaaagactggctaatgtttggtaactctctggagtagacagcactacatgtacgtaagataggtacataaacaactattggttttgagctgatttttttcagctgcatttgcatgtatggatttttctcaccaaagacgatgacttcaagtattagtaaaataattgtacagctctcctgattatacttctctgtgacatttcatttcccaggctatttcttttggtaggatttaaaactaagcaattcagtatgatctttgtccttcattttctttcttattctttttgtttgtttgtttgtttgtttttttcttgaggcagagtctctctctgtcgcccaggctggagtgcagtggcgccatctcagctcattgcaacctctgccacctccgggttcaagagattctcctgcctcagcctcccgagtagctgggattacaggtgtccaccaccacacccggctaattttttgtatttttagtagaggtggggtttcaccatgttggccaggctggtcttgagctcctgacctcaggtgatccacctgcctcggcctaccaaagagctgggataacaggtgtgacccaccatgcccggcccattttttttttcttattctgttaggagtgagagtgtaactagcagtataatagttcaattttcacaacgtggtaaaagtttccctataattcaatcagattttgctccagggttcagttctgttttaggaaatacttttattttcagtttaatgatgaaatattagagttgtaatattgcctttatgattatccacctttttaacctaaaagaatgaaagaaaaatatgtttgcaatataattttatggttgtatgttaacttaattcattatgttggcctccagtttgctgttgttagttatgacagcagtagtgtcattaccatttcaattcagattacattcctatatttgatcattgtaaactgactgcttacattgtattaaaaacagtggatattttaaagaagctgtacggcttatatctagtgctgtctcttaagactattaaattgatacaacatatttaaaagtaaatattacctaaatgaatttttgaaattacaaatacacgtgttaaaactgtcgttgtgttcaaccatttctgtacatacttagagttaactgttttgccaggctctgtatgcctactcataatatgataaaagcactcatctaatgctctgtaaatagaagtcagtgctttccatcagactgaactctcttgacaagatgtggatgaaattctttaagtaaaattgtttactttgtcatacatttacagatcaaatgttagctcccaaagcaatcatatggcaaagataggtatatcatagtttgcctattagctgctttgtattgctattattataaatagacttcacagttttagacttgcttaggtgaaattgcaattctttttactttcagtcttagataacaagtcttcaattatagtacaatcacacattgcttaggaatgcatcattaggcgattttgtcattatgcaaacatcatagagtgtacttacacaaacctagatagtatagcctttatgtacctaggccgtatggtatagtctgttgctcctaggccacaaacctgtacaactgttactgtactgaatactatagacagttgtaacacagtggtaaatatttatctaaatatatgcaaacagagaaaaggtacagtaaaagtatggtataaaagataatggtatacctgtgtaggccacttaccacgaatggagcttgcaggactagaagttgctctgggtgagtcagtgagtgagtggtgaattaatgtgaaggcctagaacactgtacaccactgtagactataaacacagtacgctgaagctacaccaaatttatcttaacagtttttcttcaataaaaaattataactttttaactttgtaaactttttaattttttaacttttaaaatacttagcttgaaacacaaatacattgtatagctatacaaaaatattttttctttgtatccttattctagaagcttttttctattttctattttaaatttttttttttacttgttagtcgtttttgttaaaaactaaaacacacacactttcacctaggcatagacaggattaggatcatcagtatcactcccttccacctcactgccttccacctccacatcttgtcccactggaaggtttttaggggcaataacacacatgtagctgtcacctatgataacagtgctttctgttgaatacctcctgaaggacttgcctgaggctgttttacatttaacttaaaaaaaaaaaaagtagaaggagtgcactctaaaataacaataaaaggcatagtatagtgaatacataaaccagcaatgtagtagtttattatcaagtgttgtacactgtaataattgtatgtgctatactttaaataacttgcaaaatagtactaagaccttatgatggttacagtgtcactaaggcaatagcatattttcaggtccattgtaatctaatgggactaccatcatatatgcagtctaccattgactgaaacgttacatggcacataactgtatttgcaagaatgatttgttttacattaatatcacataggatgtacctttttagagtggtatgtttatgtggattaagatgtacaagttgagcaaggggaccaagagccctgggttctgtcttggatgtgagcgtttatgttcttctcctcatgtctgttttctcattaaattcaaaggcttgaacgggccctatttagcccttctgttttctacgtgttctaaataactaaagcttttaaattctagccatttagtgtagaactctctttgcagtgatgaaatgctgtattggtttcttggctagcatattaaatatttttatctttgtcttgatacttcaatgtcgttttaaacatcaggatcgggcttcagtattctcataaccagagagttcactgaggatacaggactgtttgcccattttttgttatggctccagacttgtggtatttccatgtctttttttttttttttttttttgaccttttagcggctttaaagtatttctgttgttaggtgttgtattacttttctaagattacttaacaaagcaccacaaactgagtggctttaaacaacagcaatttattctctcacaattctagaagctagaagtccgaaatcaaagtgttgacaggggcatgatcttcaagagagaagactctttccttgcctcttcctggcttctggtggttaccagcaatcctgagtgttcctttcttgccttgtagtttcaacaatccagtatctgccttttgtcttcacatggctgtctaccatttgtctctgtgtctccaaatctctctccttataaacacagcagttattggattaggccccactctaatccagtatgaccccattttaacatgattacacttatttctagataaggtcacattcacgtacaccaagggttaggaattgaacatatctttttgggggacacaattcaacccacaagtgtcagtctctagctgagcctttcccttcctgtttttctcctttttagttgctatgggttaggggccaaatctccagtcatactagaattgcacatggactggatatttgggaatactgcgggtctattctatgagctttagtatgtaacatttaatatcagtgtaaagaagcccttttttaagttatttctttgaatttctaaatgtatgccctgaatataagtaacaagttaccatgtcttgtaaaatgatcatatcaacaaacatttaatgtgcacctactgtgctagttgaatgtctttatcctgataggagataacaggattccacatctttgacttaagaggacaaaccaaatatgtctaaatcatttggggttttgatggatatctttaaattgctgaacctaatcattggtttcatatgtcattgtttagatatctccggagcatttggataatgtgacagttggaatgcagtgatgtcgactctttgcccaccgccatctccagctgttgccaagacagagattgctttaagtggcaaatcacctttattagcagctacttttgcttactgggacaatattcttggtcctagagtaaggcacatttgggctccaaagacagaacaggtacttctcagtgatggagaaataacttttcttgccaaccacactctaaatggagaaatccttcgaaatgcagagagtggtgctatagatgtaaagttttttgtcttgtctgaaaagggagtgattattgtttcattaatctttgatggaaactggaatggggatcgcagcacatatggactatcaattatacttccacagacagaacttagtttctacctcccacttcatagagtgtgtgttgatagattaacacatataatccggaaaggaagaatatggatgcataaggtaagtgatttttcagcttattaatcatgttaacctatctgttgaaagcttattttctggtacatataaatcttatttttttaattatatgcagtgaacatcaaacaataaatgttatttattttgcatttaccctattagatacaaatacatctggtctgatacctgtcatcttcatattaactgtggaaggtacgaaatggtagctccacattatagatgaaaagctaaagcttagacaaataaagaaacttttagaccctggattcttcttgggagcctttgactctaataccttttgtttccctttcattgcacaattctgtcttttgcttactactatgtgtaagtataacagttcaaagtaatagtttcataagctgttggtcatgtagcctttggtctctttaacctctttgccaagttcccaggttcataaaatgaggaggttgaatggaatggttcccaagagaattccttttaatcttacagaaattattgttttcctaaatcctgtagttgaatatataatgctatttacatttcagtatagttttgatgtatctaaagaacacattgaattctccttcctgtgttccagtttgatactaacctgaaagtccattaagcattaccagttttaaaaggcttttgcccaatagtaaggaaaaataatatcttttaaaagaataattttttactatgtttgcaggcttacttccttttttctcacattatgaaactcttaaaatcaggagaatcttttaaacaacatcataatgtttaatttgaaaagtgcaagtcattcttttcctttttgaaactatgcagatgttacattgactgttttctgtgaagttatctttttttcactgcagaataaaggttgttttgattttattttgtattgtttatgagaacatgcatttgttgggttaatttcctacccctgcccccattttttccctaaagtagaaagtatttttcttgtgaactaaattactacacaagaacatgtctattgaaaaataagcaagtatcaaaatgttgtgggttgtttttttaaataaattttctcttgctcaggaaagacaagaaaatgtccagaagattatcttagaaggcacagagagaatggaagatcaggtatatgcaaattgcatactgtcaaatgtttttctcacagcatgtatctgtataaggttgatggctacatttgtcaaggccttggagacatacgaataagcctttaatggagcttttatggaggtgtacagaataaactggaggaagatttccatatcttaaacccaaagagttaaatcagtaaacaaaggaaaatagtaattgcatctacaaattaatatttgctccctttttttttctgtttgcccagaataaattttggataacttgttcatagtaaaaataaaaaaaattgtctctgatatgttctttaaggtactacttctcgaacctttccctagaagtagctgtaacagaaggagagcatatgtacccctgaggtatctgtctggggtgtaggcccaggtccacacaatatttcttctaagtcttatgttgtatcgttaagactcatgcaatttacattttattccataactattttagtattaaaatttgtcagtgatatttcttaccctctcctctaggaaaatgtgccatgtttatcccttggctttgaatgcccctcaggaacagacactaagagtttgagaagcatggttacaagggtgtggcttcccctgcggaaactaagtacagactatttcactgtaaagcagagaagttcttttgaaggagaatctccagtgaagaaagagttcttcacttttacttccatttcctcttgtgggtgaccctcaatgctccttgtaaaactccaatattttaaacatggctgttttgcctttctttgcttctttttagcatgaatgagacagatgatactttaaaaaagtaattaaaaaaaaaaacttgtgaaaatacatggccataatacagaacccaatacaatgatctcctttaccaaattgttatgtttgtacttttgtagatagctttccaattcagagacagttattctgtgtaaaggtctgacttaacaagaaaagatttccctttacccaaagaatcccagtccttatttgctggtcaataagcagggtccccaggaatggggtaactttcagcaccctctaacccactagttattagtagactaattaagtaaacttatcgcaagttgaggaaacttagaaccaactaaaattctgcttttactgggattttgttttttcaaaccagaaacctttacttaagttgactactattaatgaattttggtctctcttttaagtgctcttcttaaaaatgttatcttactgctgagaagttcaagtttgggaagtacaaggaggaatagaaacttaagagattttcttttagagcctcttctgtatttagccctgtaggatttttttttttttttttttttttggtgttgttgagcttcagtgaggctattcattcacttatactgataatgtctgagatactgtgaatgaaatactatgtatgcttaaacctaagaggaaatattttcccaaaattattcttcccgaaaaggaggagttgccttttgattgagttcttgcaaatctcacaacgactttattttgaacaatactgtttggggatgatgcattagtttgaaacaacttcagttgtagctgtcatctgataaaattgcttcacagggaaggaaatttaacacggatctagtcattattcttgttagattgaatgtgtgaattgtaattgtaaacaggcatgataattattactttaaaaactaaaaacagtgaatagttagttgtggaggttactaaaggatggtttttttttaaataaaactttcagcattatgcaaatgggcatatggcttaggataaaacttccagaagtagcatcacatttaaattctcaagcaacttaataatatggggctctgaaaaactggttaaggttactccaaaaatggccctgggtctgacaaagattctaacttaaagatgcttatgaagactttgagtaaaatcatttcataaaataagtgaggaaaaacaactagtattaaattcatcttaaataatgtatgatttaaaaaatatgtttagctaaaaatgcatagtcatttgacaatttcatttatatctcaaaaaatttacttaaccaagttggtcacaaaactgatgagactggtggtggtagtgaataaatgagggaccatccatatttgagacactttacatttgtgatgtgttatactgaattttcagtttgattctatagactacaaatttcaaaattacaatttcaagatgtaataagtagtaatatcttgaaatagctctaaagggaatttttctgttttattgattcttaaaatatatgtgctgattttgatttgcatttgggtagattatacttttatgagtatggaggttaggtattgattcaagttttccttacctatttggtaaggatttcaaagtctttttgtgcttggttttcctcatttttaaatatgaaatatattgatgacctttaacaaattttttttatctcaaattttaaaggagatcttttctaaaagaggcatgatgacttaatcattgcatgtaacagtaaacgataaaccaatgattccatactctctaaagaataaaagtgagctttagggccgggcatggtcagaaatttgacaccaacctggccaacatggcgaaaccccgtctctactaaaaatacaaaaatcagccgggcatggtggcggcacctatagtcccagctacttgggaggatgagacaggagagtcacttgaacctgggaggagaggttgcagtgagctgagatcacgccattgcactccagcctgagcaatgaaagcaaaactccatctcaaaaaaaaaaaaagaaaagaaagaataaaagtgagctttggattgcatataaatcctttagacatgtagtagacttgtttgatactgtgtttgaacaaattacgaagtattttcatcaaagaatgttattgtttgatgttatttttattttttattgcccagcttctctcatattacgtgattttcttcacttcatgtcactttattgtgcagggtcagagtattattccaatgcttactggagaagtgattcctgtaatggaactgctttcatctatgaaatcacacagtgttcctgaagaaatagatgtaagtttaaatgagagcaattatacactttatgagttttttggggttatagtattattatgtatattattaatattctaattttaatagtaaggactttgtcatacatactattcacatacagtattagccactttagcaaataagcacacacaaaatcctggattttatggcaaaacagaggcatttttgatcagtgatgacaaaattaaattcattttgtttatttcattacttttataattcctaaaagtgggaggatcccagctcttataggagcaattaatatttaatgtagtgtcttttgaaacaaaactgtgtgccaaagtagtaaccattaatggaagtttacttgtagtcacaaatttagtttccttaatcatttgttgaggacgttttgaatcacacactatgagtgttaagagatacctttaggaaactattcttgttgttttctgattttgtcatttaggttagtctcctgattctgacagctcagaagaggaagttgttcttgtaaaaattgtttaacctgcttgaccagctttcacatttgttcttctgaagtttatggtagtgcacagagattgttttttggggagtcttgattctcggaaatgaaggcagtgtgttatattgaatccagacttccgaaaacttgtatattaaaagtgttatttcaacactatgttacagccagactaatttttttattttttgatgcattttagatagctgatacagtactcaatgatgatgatattggtgacagctgtcatgaaggctttcttctcaagtaagaatttttcttttcataaaagctggatgaagcagataccatcttatgctcacctatgacaagatttggaagaaagaaaataacagactgtctacttagattgttctagggacattacgtatttgaactgttgcttaaatttgtgttatttttcactcattatatttctatatatatttggtgttattccatttgctatttaaagaaaccgagtttccatcccagacaagaaatcatggccccttgcttgattctggtttcttgttttacttctcattaaagctaacagaatcctttcatattaagttgtactgtagatgaacttaagttatttaggcgtagaacaaaattattcatatttatactgatctttttccatccagcagtggagtttagtacttaagagtttgtgcccttaaaccagactccctggattaatgctgtgtacccgtgggcaaggtgcctgaattctctatacacctatttcctcatctgtaaaatggcaataatagtaatagtacctaatgtgtagggttgttataagcattgagtaagataaataatataaagcacttagaacagtgcctggaacataaaaacacttaataatagctcatagctaacatttcctatttacatttcttctagaaatagccagtatttgttgagtgcctacatgttagttcctttactagttgctttacatgtattatcttatattctgttttaaagtttcttcacagttacagattttcatgaaattttacttttaataaaagagaagtaaaagtataaagtattcacttttatgttcacagtcttttcctttaggctcatgatggagtatcagaggcatgagtgtgtttaacctaagagccttaatggcttgaatcagaagcactttagtcctgtatctgttcagtgtcagcctttcatacatcattttaaatcccatttgactttaagtaagtcacttaatctctctacatgtcaatttcttcagctataaaatgatggtatttcaataaataaatacattaattaaatgatattatactgactaattgggctgttttaaggctcaataagaaaatttctgtgaaaggtctctagaaaatgtaggttcctatacaaataaaagataacattgtgcttatagcttcggtgtttatcatataaagctattctgagttatttgaagagctcacctacttttttttgtttttagtttgttaaattgttttataggcaatgtttttaatctgttttctttaacttacagtgccatcagctcacacttgcaaacctgtggctgttccgttgtagtaggtagcagtgcagagaaagtaaataaggtagtttattttataatctagcaaatgatttgactctttaagactgatgatatatcatggattgtcatttaaatggtaggttgcaattaaaatgatctagtagtataaggaggcaatgtaatctcatcaaattgctaagacaccttgtggcaacagtgagtttgaaataaactgagtaagaatcatttatcagtttattttgatagctcggaaataccagtgtcagtagtgtataaatggttttgagaatatattaaaatcagatatataaaaaaaattactcttctatttcccaatgttatctttaacaaatctgaagatagtcatgtacttttggtagtagttccaaagaaatgttatttgtttattcatcttgatttcattgtcttcgctttccttctaaatctgtcccttctagggagctattgggattaagtggtcattgattattatactttattcagtaatgtttctgaccctttccttcagtgctacttgagttaattaaggattaatgaacagttacatttccaagcattagctaataaactaaaggattttgcacttttcttcactgaccattagttagaaagagttcagagataagtatgtgtatctttcaatttcagcaaacctaattttttaaaaaaagttttacataggaaatatgttggaaatgatactttacaaagatattcataatttttttttgtaatcagctactttgtatatttacatgagccttaatttatatttctcatataaccatttatgagagcttagtatacctgtgtcattatattgcatctacgaactagtgaccttattccttctgttacctcaaacaggtggctttccatctgtgatctccaaagccttaggttgcacagagtgactgccgagctgctttatgaagggagaaaggctccatagttggagtgtttttttttttttttttaaacatttttcccatcctccatcctcttgagggagaatagcttaccttttatcttgttttaatttgagaaagaagttgccaccactctaggttgaaaaccactcctttaacataataactgtggatatggtttgaatttcaagatagttacatgcctttttatttttcctaatagagctgtaggtcaaatattattagaatcagatttctaaatcccacccaatgacctgcttattttaaatcaaattcaataattaattctcttctttttggaggatctggacattctttgatatttcttacaacgaatttcatgtgtagacccactaaacagaagctataaaagttgcatggtcaaataagtctgagaaagtctgcagatgatataattcacctgaagagtcacagtatgtagccaaatgttaaaggttttgagatgccatacagtaaatttaccaagcattttctaaatttatttgaccacagaatccctattttaagcaacaactgttacatcccatggattccaggtgactaaagaatacttatttcttaggatatgttttattgataataacaattaaaatttcagatatctttcataagcaaatcagtggtctttttacttcatgttttaatgctaaaatattttcttttatagatagtcagaacattatgcctttttctgactccagcagagagaaaatgctccaggttatgtgaagcagaatcatcatttaaatatgagtcagggctctttgtacaaggcctgctaaaggtatagtttctagttatcacaagtgaaaccacttttctaaaatcatttttgagactctttatagacaaatcttaaatattagcatttaatgtatctcatattgacatgcccagagactgacttcctttacacagttctgcacatagactatatgtcttatggatttatagttagtatcatcagtgaaacaccatagaataccctttgtgttccaggtgggtccctgttcctacatgtctagcctcaggacttttttttttttaacacatgcttaaatcaggttgcacatcaaaaataagatcatttctttttaactaaatagatttgaattttattgaaaaaaaattttaaacatctttaagaagcttataggatttaagcaattcctatgtatgtgtactaaaatatatatatttctatatataatatatattagaaaaaaattgtatttttcttttatttgagtctactgtcaaggagcaaaacagagaaatgtaaattagcaattatttataatacttaaagggaagaaagttgttcaccttgttgaatctattattgttatttcaattatagtcccaagacgtgaagaaatagctttcctaatggttatgtgattgtctcatagtgactactttcttgaggatgtagccacggcaaaatgaaataaaaaaatttaaaaattgttgcaaatacaagttatattaggcttttgtgcattttcaataatgtgctgctatgaactcagaatgatagtatttaaatatagaaactagttaaaggaaacgtagtttctatttgagttatacatatctgtaaattagaacttctcctgttaaaggcataataaagtgcttaatacttttgtttcctcagcaccctctcatttaattatataattttagttctgaaagggacctataccagatgcctagaggaaatttcaaaactatgatctaatgaaaaaatatttaatagttctccatgcaaatacaaatcatatagttttccagaaaatacctttgacattatacaaagatgattatcacagcattataatagtaaaaaaatggaaatagcctctttcttctgttctgttcatagcacagtgcctcatacgcagtaggttattattacatggtaactggctaccccaactgattaggaaagaagtaaatttgttttataaaaatacatactcattgaggtgcatagaataattaagaaattaaaagacacttgtaattttgaatccagtgaatacccactgttaatatttggtatatctctttctagtctttttttcccttttgcatgtattttctttaagactcccacccccactggatcatctctgcatgttctaatctgcttttttcacagcagattctaagcctctttgaatatcaacacaaacttcaacaacttcatctatagatgccaaataataaattcatttttatttacttaaccacttcctttggatgcttaggtcattctgatgttttgctattgaaaccaatgctatactgaacacttctgtcactaaaactttgcacacactcatgaatagcttcttaggataaatttttagagatggatttgctaaatcagagaccattttttaaaattaaaaaacaattattcatatcgtttggcatgtaagacagtaaattttccttttattttgacaggattcaactggaagctttgtgctgcctttccggcaagtcatgtatgctccatatcccaccacacacatagatgtggatgtcaatactgtgaagcagatgccaccctgtcatgaacatatttataatcagcgtagatacatgagatccgagctgacagccttctggagagccacttcagaagaagacatggctcaggatacgatcatctacactgacgaaagctttactcctgatttgtacgtaatgctctgcctgctggtactgtagtcaagcaatatgaaattgtgtcttttacgaataaaaacaaaacagaagttgcatttaaaaagaaagaaatattaccagcagaattatgcttgaagaaacatttaatcaagcatttttttcttaaatgttcttctttttccatacaattgtgtttaccctaaaataggtaagattaacccttaaagtaaatatttaactatttgtttaataaatatatattgagctcctaggcactgttctaggtaccgggcttaatagtggccaaccagacagccccagccccagcccctacattgtgtatagtctattatgtaacagttattgaatggacttattaacaaaaccaaagaagtaattctaagtcttttttttcttgacatatgaatataaaatacagcaaaactgttaaaatatattaatggaacatttttttactttgcattttatattgttattcacttcttatttttttttaaaaaaaaaagcctgaacagtaaattcaaaaggaaaagtaatgataattaattgttgagcatggacccaacttgaaaaaaaaaatgatgatgataaatctataatcctaaaaccctaagtaaacacttaaaagatgttctgaaatcaggaaaagaattatagtatacttttgtgtttctcttttatcagttgaaaaaaggcacagtagctcatgcctgtaagaacagagctttgggagtgcaaggcaggcggatcacttgaggccaggagttccagaccagcctgggcaacatagtgaaaccccatctctacaaaaaataaaaaagaattattggaatgtgtttctgtgtgcctgtaatcctagctattccgaaagctgaggcaggaggatcttttgagcccaggagtttgaggttacagggagttatgatgtgccagtgtactccagcctggggaacaccgagactctgtcttatttaaaaaaaaaaaaaaaaaaatgcttgcaataatgcctggcacatagaaggtaacagtaagtgttaactgtaataacccaggtctaagtgtgtaaggcaatagaaaaattggggcaaataagcctgacctatgtatctacagaatcagtttgagcttaggtaacagacctgtggagcaccagtaattacacagtaagtgttaaccaaaagcatagaataggaatatcttgttcaagggacccccagccttatacatctcaaggtgcagaaagatgacttaatataggacccattttttcctagttctccagagtttttattggttcttgagaaagtagtaggggaatgttttagaaaatgaattggtccaactgaaattacatgtcagtaagtttttatatattggtaaattttagtagacatgtagaagttttctaattaatctgtgccttgaaacattttcttttttcctaaagtgcttagtattttttccgttttttgattggttacttgggagcttttttgaggaaatttagtgaactgcagaatgggtttgcaaccatttggtatttttgttttgttttttagaggatgtatgtgtattttaacatttcttaatcatttttagccagctatgtttgttttgctgatttgacaaactacagttagacagctattctcattttgctgatcatgacaaaataatatcctgaatttttaaattttgcatccagctctaaattttctaaacataaaattgtccaaaaaatagtattttcagccactagattgtgtgttaagtctattgtcacagagtcattttacttttaagtatatgtttttacatgttaattatgtttgttatttttaattttaactttttaaaataattccagtcactgccaatacatgaaaaattggtcactggaattttttttttgacttttattttaggttcatgtgtacatgtgcaggtgtgttatacaggtaaattgcgtgtcatgagggtttggtgtacaggtgatttcattacccaggtaataagcatagtacccaataggtagttttttgatcctcacccttctcccaccctcaagtaggccctggtgttgctgtttccttctttgtgtccatgtatactcagtgtttagctcccacttagaagtgagaacatgcggtagttggttttctgttcctggattagttcacttaggataatgacctctagctccatctggtttttatggctgcatagtattccatggtgtatatgtatcacattttctttatccagtctaccattgataggcatttaggttgattccctgtctttgttatcatgaatagtgctgtgatgaacatacacatgcatgtgtctttatggtagaaaaatttgtattcctttaggtacatatagaataatggggttgctagggtgaatggtagttctattttcagttatttgagaaatcttcaaactgcttttcataatagctaaactaatttacagtcccgccagcagtgtataagtgttcccttttctccacaaccttgccaacatctgtgattttttgactttttaataatagccattcctagagaattgatttgcaattctctattagtgatattaagcattttttcatatgctttttagctgtctgtatatattcttctgaaaaattttcatgtcctttgcccagtttgtagtggggtgggttgttttttgcttgttaattagttttaagttccttccagattctgcatatccctttgttggatacatggtttgcagatatttttctcccattgtgtaggttgtcttttactctgttgatagtttcttttgccatgcaggagctcgttaggtcccatttgtgtttgtttttgttgcagttgcttttggcgtcttcatcataaaatctgtgccagggcctatgtccagaatggtatttcctaggttgtcttccagggtttttacaattttagattttacgtttatgtctttaatccatcttgagttgatttttgtatatggcacaaggaaggggtccagtttcactccaattcctatggctagcaattatcccagcaccatttattgaatacggagtcctttccccattgcttgttttttgtcaactttgttgaagatcagatggttgtaagtgtgtggctttatttcttggctctctattctccattggtctatgtgtctgtttttataacagtaccctgctgttcaggttcctatagccttttagtataaaatcggctaatgtgatgcctccagctttgttctttttgcttaggattgctttggctatttgggctcctttttgggtccatattaattttaaaacagttttttctggttttgtgaaggatatcattggtagtttataggaatagcattgaatctgtagattgctttgggcagtatggccattttaacaatattaattcttcctatctatgaatatggaatgtttttccatgtgtttgtgtcatctctttatacctgatgtataaagaaaagctggtattattcctactcaatctgttccaaaaaattgaggaggaggaactcttccctaatgaggccagcatcattctgataccaaaacctggcagagacacaacagaaaaaagaaaacttcaggccaatatccttgatgaatatagatgcaaaaatcctcaacaaaatactagcaaaccaaatccagcagcacatcaaaaagctgatctactttgatcaagtaggctttatccctgggatgcaaggttggttcaacatacacaaatcaataagtgtgattcatcacataaacagagctaaaaacaaaaaccacaagattatctcaataggtagagaaaaggttgtcaataaaatttaacatcctccatgttaaaaaccttcagtaggtcaggtgtagtgactcacacctgtaatcccagcactttgggaggccaaggcgggcatatctcttaagcccaggagttcaagacgagcctaggcagcatggtgaaaccccatctctacaaaaaaaaaaaaaaaaaaaaattagcttggtatggtgacatgcacctatagtcccagctattcaggaggttgaggtgggaggattgtttgagcccgggaggcagaggttggcagcgagctgagatcatgccaccgcactccagcctgggcaacggagtgagaccctgtctcaaaaaagaaaaatcacaaacaatcctaaacaaactaggcattgaaggaacatgcctcaaaaaaataagaaccatctatgacagacccatagccaatatcttaccaaatgggcaaaagctggaagtattctccttgagaaccgtaacaagacaaggatgtccactctcaccactccttttcagcatagttctggaagtcctagccagagcaatcaggaaagagaaagaaagaaagacattcagataggaagagaagaagtcaaactatttctgtttgcaggcagtataattctgtacctagaaaatctcatagtctctgcccagaaactcctaaatctgttaaaaatttcagcaaagttttggcattctctatactccaacaccttccaaagtgagagcaaaatcaagaacacagtcccattcacaatagccgcaaaacgaataaaatacctaggaatccagctaaccagggaggtgaaagatctctatgagaattacaaaacactgctgaaagaaatcagagatgacacaaacaaatggaaatgttcttttttaacaccttgctttatctaattcacttatgatgaagatactcattcagtggaacaggtataataagtccactcgattaaatataagccttattctctttccagagcccaagaaggggcactatcagtgcccagtcaataatgacgaaatgctaatatttttcccctttacggtttctttcttctgtagtgtggtacactcgtttcttaagataaggaaacttgaactaccttcctgtttgcttctacacatacccattctctttttttgccactctggtcaggtataggatgatccctaccactttcagttaaaaactcctcctcttactaaatgttctcttaccctctggcctgagtagaacctagggaaaatggaagagaaaaagatgaaagggaggtggggcctgggaagggaataagtagtcctgtttgtttgtgtgtttgctttagcacctgctatatcctaggtgctgtgttaggcacacattattttaagtggccattatattactactactcactctggtcgttgccaaggtaggtagtactttcttggatagttggttcatgttacttacagatggtgggcttgttgaggcaaacccagtggataatcatcggagtgtgttctctaatctcactcaaatttttcttcacattttttggtttgttttggtttttgatggtagtggcttatttttgttgctggtttgttttttgtttttttttgagatggcaagaattggtagttttatttattaattgcctaagggtctctactttttttaaaagatgagagtagtaaaatagattgatagatacatacatacccttactggggactgcttatattctttagagaaaaaattacatattagcctgacaaacaccagtaaaatgtaaatatatccttgagtaaataaatgaatgtatattttgtgtctccaaatatatatatctatattcttacaaatgtgtttatatgtaatatcaatttataagaacttaaaatgttggctcaagtgagggattgtggaaggtagcattatatggccatttcaacatttgaacttttttcttttcttcattttcttcttttcttcaggaatatttttcaagatgtcttacacagagacactctagtgaaagccttcctggatcaggtaaatgttgaacttgagattgtcagagtgaatgatatgacatgttttcttttttaatatatcctacaatgcctgttctatatatttatattcccctggatcatgccccagagttctgctcagcaattgcagttaagttagttacactacagttctcagaagagtctgtgagggcatgtcaagtgcatcattacattggttgcctcttgtcctagatttatgcttcgggaattcagacctttgtttacaatataataaatattattgctatcttttaaagatataataataagatataaagttgaccacaactactgttttttgaaacatagaattcctggtttacatgtatcaaagtgaaatctgacttagcttttacagatataatatatacatatatatatcctgcaatgcttgtactatatatgtagtacaagtatatatatatgtttgtgtgtgtatatatatatagtacgagcatatatacatattaccagcattgtaggatatatatatgtttatatattaaaaaaaagttataaacttaaaaccctattatgttatgtagagtatatgttatatatgatatgtaaaatatataacatatactctatgatagagtgtaatatattttttatatatattttaacatttataaaatgatagaattaagaattgagtcctaatctgttttattaggtgctttttgtagtgtctggtctttctaaagtgtctaaatgatttttccttttgacttattaatggggaagagcctgtatattaacaattaagagtgcagcattccatacgtcaaacaacaaacattttaattcaagcattaacctataacaagtaagttttttttttttttttgagaaagggaggttgtttatttgcctgaaatgactcaaaaatatttttgaaacatagtgtacttatttaaataacatctttattgtttcattcttttaaaaaatatctacttaattacacagttgaaggaaatcgtagattatatggaacttatttcttaatatattacagtttgttataataacattctggggatcaggccaggaaactgtgtcatagataaagctttgaaataatgagatccttatgtttactagaaattttggattgagatctatgaggtctgtgacatattgcgaagttcaaggaaaattcgtaggcctggaatttcatgcttctcaagctgacataaaatccctcccactctccacctcatcatatgcacacattctactcctacccacccactccaccccctgcaaaagtacaggtatatgaatgtctcaaaaccataggctcatcttctaggagcttcaatgttatttgaagatttgggcagaaaaaattaagtaatacgaaataacttatgtatgagttttaaaagtgaagtaaacatggatgtattctgaagtagaatgcaaaatttgaatgcatttttaaagataaattagaaaacttctaaaaactgtcagattgtctgggcctggtggcttatgcctgtaatcccagcactttgggagtccgaggtgggtggatcacaaggtcaggagatcgagaccatcctgccaacatggtgaaaccccgtctctactaagtatacaaaaattagctgggcgtggcagcgtgtgcctgtaatcccagctacctgggaggctgaggcaggagaatcgcttgaacccaggaggtgtaggttgcagtgagtcaagatcgcgccactgcactttagcctggtgacagagctagactccgtctcaaaaaaaaaaaaaaatatcagattgttcctacacctagtgcttctataccacactcctgttagggggcatcagtggaaatggttaaggagatgtttagtgtgtattgtctgccaagcactgtcaacactgtcatagaaacttctgtacgagtagaatgtgagcaaattatgtgttgaaatggttcctctccctgcaggtctttcagctgaaacctggcttatctctcagaagtactttccttgcacagtttctacttgtccttcacagaaaagccttgacactaataaaatatatagaagacgatacgtgagtaaaactcctacacggaagaaaaacctttgtacattgtttttttgttttgtttcctttgtacattttctatatcataatttttgcgcttcttttttttttttttttttttttttttccattatttttaggcagaagggaaaaaagccctttaaatctcttcggaacctgaagatagaccttgatttaacagcagagggcgatcttaacataataatggctctggctgagaaaattaaaccaggcctacactcttttatctttggaagacctttctacactagtgtgcaagaacgagatgttctaatgactttttaaatgtgtaacttaataagcctattccatcacaatcatgatcgctggtaaagtagctcagtggtgtggggaaacgttcccctggatcatactccagaattctgctctcagcaattgcagttaagtaagttacactacagttctcacaagagcctgtgaggggatgtcaggtgcatcattacattgggtgtctcttttcctagatttatgcttttgggatacagacctatgtttacaatataataaatattattgctatcttttaaagatataataataggatgtaaacttgaccacaactactgtttttttgaaatacatgattcatggtttacatgtgtcaaggtgaaatctgagttggcttttacagatagttgactttctatcttttggcattctttggtgtgtagaattactgtaatacttctgcaatcaactgaaaactagagcctttaaatgatttcaattccacagaaagaaagtgagcttgaacataggatgagctttagaaagaaaattgatcaagcagatgtttaattggaattgattattagatcctactttgtggatttagtccctgggattcagtctgtagaaatgtctaatagttctctatagtccttgttcctggtgaaccacagttagggtgttttgtttattttattgttcttgctattgttgatattctatgtagttgagctctgtaaaaggaaattgtattttatgttttagtaattgttgccaactttttaaattaattttcattatttttgagccaaattgaaatgtgcacctcctgtgccttttttctccttagaaaatctaattacttggaacaagttcagatttcactggtcagtcattttcatcttgttttcttcttgctaagtcttaccatgtacctgctttggcaatcattgcaactctgagattataaaatgccttagagaatatactaactaataagatctttttttcagaaacagaaaatagttccttgagtacttccttcttgcatttctgcctatgtttttgaagttgttgctgtttgcctgcaataggctataaggaatagcaggagaaattttactgaagtgctgttttcctaggtgctactttggcagagctaagttatcttttgttttcttaatgcgtttggaccattttgctggctataaaataactgattaatataattctaacacaatgttgacattgtagttacacaaacacaaataaatattttatttaaaattctggaagtaatataaaagggaaaatatatttataagaaagggataaaggtaatagagcccttctgccccccacccaccaaatttacacaacaaaatgacatgttcgaatgtgaaaggtcataatagctttcccatcatgaatcagaaagatgtggacagcttgatgttttagacaaccactgaactagatgactgttgtactgtagctcagtcatttaaaaaatatataaatactaccttgtagtgtcccatactgtgttttttacatggtagattcttatttaagtgctaactggttattttctttggctggtttattgtactgttatacagaatgtaagttgtacagtgaaataagttattaaagcatgtgtaaacattgttatatatcttttctcctaaatggagaattttgaataaaatatatttgaaattttgcctctttcagttgttcattcagaaaaaaatactatgatatttgaagactgatcagcttctgttcagctgacagtcatgctggatctaaactttttttaaaattaattttgtcttttcaaagaaaaaatatttaaagaagctttataatataatcttatgttaaaaaaactttctgcttaactctctggatttcattttgatttttcaaattatatattaatatttcaaatgtaaaatactatttagataaattgtttttaaacattcttattattataatattaatataacctaaactgaagttattcatcccaggtatctaatacatgtatccaaagtaaaaatccaaggaatctgaacactttcatctgcaaagctaggaataggtttgacattttcactccaagaaaaagtttttttttgaaaatagaatagttgggatgagaggtttctttaaaagaagactaactgatcacattactatgattctcaaagaagaaaccaaaacttcatataatactataaagtaaatataaaatagttccttctatagtatatttctataatgctacagtttaaacagatcactcttatataatactattttgattttgatgtagaattgcacaaattgatatttctcctatgatctgcagggtatagcttaaagtaacaaaaacagtcaaccacctccatttaacacacagtaacactatgggactagttttattacttccattttacaaatgaggaaactaaagcttaaagatgtgtaatacaccgcccaaggtcacacagctggtaaaggtggatttcatcccagacagttacagtcattgccatgggcacagctcctaacttagtaactccatgtaactggtactcagtgtagctgaattgaaaggagagtaaggaagcaggttttacaggtctacttgcactattcagagcccgagtgtgaatccctgctgtgctgcttggagaagttacttaacctatgcaaggttcattttgtaaatattggaaatggagtgataatacgtacttcaccagaggatttaatgagaccttatacgatccttagttcagtacctgactagtgcttcataaatgctttttcatccaatctgacaatctccagcttgtaattggggcatttagaacatttaatatgattattggcatggtaggttaaagctgtcatcttgctgttttctatttgttctttttgttttctccttacttttggatttttttattctactatgtcttttctattgtcttattaactatactctttgatttattttagtggttgttttagggttatacctctttctaatttaccagtttataaccagtttatatactacttgacatatagcttaagaaacttactgttgttgtctttttgctgttatggtcttaacgtttttatttctacaaacattataaactccacactttattgttttttaattttacttatacagtcaattatcttttaaagatatttaaatataaacattcaaaacaccccaat

SEQ ID NO: 3 - RNA, 1031 nt, Homo sapiens
  source 1..1031: mol_type = mRNA
attcccgggatacgtaacctacggtgtcccgctaggaaagagaggtgcgtcaaacagcgacaagttccgcccacgtaaaagatgacgcttggtgtgtcagccgtccctgctgcccggttgcttctcttttgggggcggggtctagcaagagcaggtgtgggtttaggagatatctccggagcatttggataatgtgacagttggaatgcagtgatgtcgactctttgcccaccgccatctccagctgttgccaagacagagattgctttaagtggcaaatcacctttattagcagctacttttgcttactgggacaatattcttggtcctagagtaaggcacatttgggctccaaagacagaacaggtacttctcagtgatggagaaataacttttcttgccaaccacactctaaatggagaaatccttcgaaatgcagagagtggtgctatagatgtaaagttttttgtcttgtctgaaaagggagtgattattgtttcattaatctttgatggaaactggaatggggatcgcagcacatatggactatcaattatacttccacagacagaacttagtttctacctcccacttcatagagtgtgtgttgatagattaacacatataatccggaaaggaagaatatggatgcataaggaaagacaagaaaaatgtccagaagattatcttagaaggcacagagagaatggaagatcagggtcagagtattattccaatgcttactggagaagtgattcctgtaatggaaactgctttcctctatgaaattcccccgggttcctggaggaaatagatataggctgatacagttacccaatgatggatgaatattgggggaccgcctggtcattgaaaggctttcttttctccaggaaagaaatttttttccttttccataaaaagcttgggaatggaagacaacaattcccattctttttttgcgttccacccctatgtgacaacagaaatttttggggaaacaacaacgaaaaaattttatcccgcgcgca

SEQ ID NO: 4 - RNA, 3244 nt, Homo sapiens
  source 1..3244: mol_type = mRNA
gggcggggctgcggttgcggtgcctgcgcccgcggcggcggaggcgcaggcggtggcgagtggatatctccggagcatttggataatgtgacagttggaatgcagtgatgtcgactctttgcccaccgccatctccagctgttgccaagacagagattgctttaagtggcaaatcacctttattagcagctacttttgcttactgggacaatattcttggtcctagagtaaggcacatttgggctccaaagacagaacaggtacttctcagtgatggagaaataacttttcttgccaaccacactctaaatggagaaatccttcgaaatgcagagagtggtgctatagatgtaaagttttttgtcttgtctgaaaagggagtgattattgtttcattaatctttgatggaaactggaatggggatcgcagcacatatggactatcaattatacttccacagacagaacttagtttctacctcccacttcatagagtgtgtgttgatagattaacacatataatccggaaaggaagaatatggatgcataaggaaagacaagaaaatgtccagaagattatcttagaaggcacagagagaatggaagatcagggtcagagtattattccaatgcttactggagaagtgattcctgtaatggaactgctttcatctatgaaatcacacagtgttcctgaagaaatagatatagctgatacagtactcaatgatgatgatattggtgacagctgtcatgaaggctttcttctcaatgccatcagctcacacttgcaaacctgtggctgttccgttgtagtaggtagcagtgcagagaaagtaaataagatagtcagaacattatgcctttttctgactccagcagagagaaaatgctccaggttatgtgaagcagaatcatcatttaaatatgagtcagggctctttgtacaaggcctgctaaaggattcaactggaagctttgtgctgcctttccggcaagtcatgtatgctccatatcccaccacacacatagatgtggatgtcaatactgtgaagcagatgccaccctgtcatgaacatatttataatcagcgtagatacatgagatccgagctgacagccttctggagagccacttcagaagaagacatggctcaggatacgatcatctacactgacgaaagctttactcctgatttgaatatttttcaagatgtcttacacagagacactctagtgaaagccttcctggatcaggtctttcagctgaaacctggcttatctctcagaagtactttccttgcacagtttctacttgtccttcacagaaaagccttgacactaataaaatatatagaagacgatacgcagaagggaaaaaagccctttaaatctcttcggaacctgaagatagaccttgatttaacagcagagggcgatcttaacataataatggctctggctgagaaaattaaaccaggcctacactcttttatctttggaagacctttctacactagtgtgcaagaacgagatgttctaatgactttttaaatgtgtaacttaataagcctattccatcacaatcatgatcgctggtaaagtagctcagtggtgtggggaaacgttcccctggatcatactccagaattctgctctcagcaattgcagttaagtaagttacactacagttctcacaagagcctgtgaggggatgtcaggtgcatcattacattgggtgtctcttttcctagatttatgcttttgggatacagacctatgtttacaatataataaatattattgctatcttttaaagatataataataggatgtaaacttgaccacaactactgtttttttgaaatacatgattcatggtttacatgtgtcaaggtgaaatctgagttggcttttacagatagttgactttctatcttttggcattctttggtgtgtagaattactgtaatacttctgcaatcaactgaaaactagagcctttaaatgatttcaattccacagaaagaaagtgagcttgaacataggatgagctttagaaagaaaattgatcaagcagatgtttaattggaattgattattagatcctactttgtggatttagtccctgggattcagtctgtagaaatgtctaatagttctctatagtccttgttcctggtgaaccacagttagggtgttttgtttattttattgttcttgctattgttgatattctatgtagttgagctctgtaaaaggaaattgtattttatgttttagtaattgttgccaactttttaaattaattttcattatttttgagccaaattgaaatgtgcacctcctgtgccttttttctccttagaaaatctaattacttggaacaagttcagatttcactggtcagtcattttcatcttgttttcttcttgctaagtcttaccatgtacctgctttggcaatcattgcaactctgagattataaaatgccttagagaatatactaactaataagatctttttttcagaaacagaaaatagttccttgagtacttccttcttgcatttctgcctatgtttttgaagttgttgctgtttgcctgcaataggctataaggaatagcaggagaaattttactgaagtgctgttttcctaggtgctactttggcagagctaagttatcttttgttttcttaatgcgtttggaccattttgctggctataaaataactgattaatataattctaacacaatgttgacattgtagttacacaaacacaaataaatattttatttaaaattctggaagtaatataaaagggaaaatatatttataagaaagggataaaggtaatagagcccttctgccccccacccaccaaatttacacaacaaaatgacatgttcgaatgtgaaaggtcataatagctttcccatcatgaatcagaaagatgtggacagcttgatgttttagacaaccactgaactagatgactgttgtactgtagctcagtcatttaaaaaatatataaatactaccttgtagtgtcccatactgtgttttttacatggtagattcttatttaagtgctaactggttattttctttggctggtttattgtactgttatacagaatgtaagttgtacagtgaaataagttattaaagcatgtgtaaacattgttatatatcttttctcctaaatggagaattttgaataaaatatatttgaaattttg

SEQ ID NO: 5 - RNA, 761 nt, Homo sapiens
  source 1..761: mol_type = mRNA
cacgaggctttgatatttcttacaacgaatttcatgtgtagacccactaaacagaagctataaaagttgcatggtcaaataagtctgagaaagtctgcagatgatataattcacctgaagagtcacagtatgtagccaaatgttaaaggttttgagatgccatacagtaaatttaccaagcattttctaaatttatttgaccacagaatccctattttaagcaacaactgttacatcccatggattccaggtgactaaagaatacttatttcttaggatatgttttattgataataacaattaaaatttcagatatctttcataagcaaatcagtggtctttttacttcatgttttaatgctaaaatattttcttttatagatagtcagaacattatgcctttttctgactccagcagagagaaaatgctccaggttatgtgaagcagaatcatcatttaaatatgagtcagggctctttgtacaaggcctgctaaaggattcaactggaagctttgtgctgcctttccggcaagtcatgtatgctccatatcccaccacacacatagatgtggatgtcaatactgtgaagcagatgccaccctgtcatgaacatatttataatcagcgtagatacatgagatccgagctgacagccttctggagagccacttcagaagaagacatggctcangatacgatcatctacactgacgaaagctntactcctgatttgaatatttttcaagatgtcttacacag

SEQ ID NO: 6 - RNA, 1901 nt, Homo sapiens
  source 1..1901: mol_type = mRNA
acgtaacctacggtgtcccgctaggaaagagaggtgcgtcaaacagcgacaagttccgcccacgtaaaagatgacgcttgatatctccggagcatttggataatgtgacagttggaatgcagtgatgtcgactctttgcccaccgccatctccagctgttgccaagacagagattgctttaagtggcaaatcacctttattagcagctacttttgcttactgggacaatattcttggtcctagagtaaggcacatttgggctccaaagacagaacaggtacttctcagtgatggagaaataacttttcttgccaaccacactctaaatggagaaatccttcgaaatgcagagagtggtgctatagatgtaaagttttttgtcttgtctgaaaagggagtgattattgtttcattaatctttgatggaaactggaatggggatcgcagcacatatggactatcaattatacttccacagacagaacttagtttctacctcccacttcatagagtgtgtgttgatagattaacacatataatccggaaaggaagaatatggatgcataaggaaagacaagaaaatgtccagaagattatcttagaaggcacagagagaatggaagatcagggtcagagtattattccaatgcttactggagaagtgattcctgtaatggaactgctttcatctatgaaatcacacagtgttcctgaagaaatagatatagctgatacagtactcaatgatgatgatattggtgacagctgtcatgaaggctttcttctcaagtaagaatttttcttttcataaaagctggatgaagcagataccatcttatgctcacctatgacaagatttggaagaaagaaaataacagactgtctacttagattgttctagggacattacgtatttgaactgttgcttaaatttgtgttatttttcactcattatatttctatatatatttggtgttattccatttgctatttaaagaaaccgagtttccatcccagacaagaaatcatggccccttgcttgattctggtttcttgttttacttctcattaaagctaacagaatcctttcatattaagttgtactgtagatgaacttaagttatttaggcgtagaacaaaattattcatatttatactgatctttttccatccagcagtggagtttagtacttaagagtttgtgcccttaaaccagactccctggattaatgctgtgtacccgtgggcaaggtgcctgaattctctatacacctatttcctcatctgtaaaatggcaataatagtaatagtacctaatgtgtagggttgttataagcattgagtaagataaataatataaagcacttagaacagtgcctggaacataaaaacacttaataatagctcatagctaacatttcctatttacatttcttctagaaatagccagtatttgttgagtgcctacatgttagttcctttactagttgctttacatgtattatcttatattctgttttaaagtttcttcacagttacagattttcatgaaattttacttttaataaaagagaagtaaaagtataaagtattcacttttatgttcacagtcttttcctttaggctcatgatggagtatcagaggcatgagtgtgtttaacctaagagccttaatggcttgaatcagaagcactttagtcctgtatctgttcagtgtcagcctttcatacatcattttaaatcccatttgactttaagtaagtcacttaatctctctacatgtcaatttcttcagctataaaatgatggtatttcaataaataaatacattaattaaatgatattatactgactaattgggctgttttaaggcaaaaaaaaaaaaaaaaaaaaaaaaaaaa

SEQ ID NO: 7 - RNA, 562 nt, Homo sapiens
  source 1..562: mol_type = mRNA
agacgtaacctacggtgtcccgctaggaaagagagatatctccggagcatttggataatgtgacagttggaatgcagtgatgtcgactctttgcccaccgccatctccagctgttgccaagacagagattgctttaagtggcaaatcacctttattagcagctacnttttgcttactgggacaatattcttggtcctagagtaaggcacatttgggctccaaagacagaacaggtacttctcagtgatggagaaataacttttcttgccaaccacactctaaatggagaaatccttcgaaatgcagagagtggtgctatagatgtaaagttttttgtcttgtctgaaaagggagtgattattgtttcattaatctttgatggaaactggaatggggatcgcagcacatatggactatcaattatacttccacagacagaacttagtttctacctcccacttcatagagtgtgtgttgatagattaacacatataatccggaaaggaagaatatggatgcataaggaaagacaagaaaatgtccagaagattatcttagaagg

SEQ ID NO: 8 - RNA, 798 nt, Homo sapiens
  source 1..798: mol_type = mRNA
gggctctcttttgggggcggggtctagcaagagcagatatctccggagcatttggataatgtgacagttggaatgcagtgatgtcgactctttgcccaccgccatctccagctgttgccaagacagagattgctttaagtggcaaatcacctttattagcagctacttttgcttactgggacaatattcttggtcctagagtaaggcacatttgggctccaaagacagaacaggtacttctcagtgatggagaaataacttttcttgccaaccacactctaaatggagaaatccttcgaaatgcagagagtggtgctatagatgtaaagttttttgtcttgtctgaaaagggagtgattattgtttcattaatctttgatggaaactggaatggggatcgcagcacatatggactatcaattatacttccacagacagaacttagtttctacctcccacttcatagagtgtgtgttgatagattaacacatataatccggaaaggaagaatatggatgcataaggaaagacaagaaaatgtccagaagattatcttagaaggcacagagagaatggaagatcagggtcagagtattattccaatgcttactggagaagtgattcctgtaatgggactgctttcatctatgaaatcacacagtgttcctgaagaaatagatatagctgatacagtactccatgatgatgatatttggtgacagctgtcatgaaaggctttcttctcaagtaggaattttttcttttcataaaagctgggatgaagccagattcccatct

SEQ ID NO: 9 - RNA, 169 nt, Homo sapiens
  source 1..169: mol_type = mRNA
aaacagcgacaagttccgcccacgtaaaagatgatgcttggtgtgtcagccgtccctgctgcccggttgcttctcttttgggggcggggtctagcaagagcagatatctccggagcatttggataatgtgacagttggaatgcggtgatgtcgactctttgcccaccgc

SEQ ID NO: 10 - RNA, 176 nt, Homo sapiens
  source 1..176: mol_type = mRNA
aaaacgtcatcgcacatagaaaacagacagacgtaacctacggtgtcccgctaggaaagagaggtgcgtcaaacagcgacaagttccgcccacgtaaaagatgacgcttgatatctccggagcatttggataatgtgacagttggaatgcagtgatgtcgactctttgcccaccgc

SEQ ID NO: 11 - DNA, 38001 bp, Mus musculus
  source 1..38001: mol_type = genomic DNA
tgtctctaggtaaaattttgaaggaaaaaaaaaacactaagaaggtatattccttcaaagttccagtcttattctgaagtgtaatgttatgttagtttgactcacagacaggttttaaagaagggcttacttcaagaggacaccaaacaaataccttctattcctagtgggctctggaatcacagaaaactgacccaatcaattacattgatagctctggcttactacagacaagcaaattatcttaagtgtgcatgcatgcgcgtgtatgtgtgttagtacctaacacccacctgggaacttttcagcttttcagtgtgggatatagtataaacgtctattcctcgtgttgtggattagctgactggcctcactcagctgccttccttacctgcaaactcacccactttgactacagcatcgcactcttaaccctagccttccaaacatggtcctatgctatttctgtgtgtctggatgtatttttaactctcagatgtatacttcatttatgagatatacatctgaagaccacggtacaaaacactgtaagaacttgatagaatgacaactgctaggtaaaaaaaaaaaaaaaaaaaaaaaaaaaaaaaaaaaaaagcatacaatacctggtgagagttctatttttaccgaaggtggtattgataggtattctgttattaatgcctttcttttccctataaatgatgaaaagttgctggaaaataataaacactactcatctgtagtgaaaagccacaatacagttacaaaccaatcaatcaatcaataaatcagacgtcatggtgttcttttcccaaaggttaaaaaacaaagtgcactgtgctatttggcaaaaatgacgtttagaagaaaacacggtgactacgcacagagggtgggggaatcattgtgcttgttgcggagtgaacacgtacagtgtgcacgcagacttacggcatttaaccgtgtcatagggaccaaaggaaatccactcactcactaaatatttgttgagcacccactacctgccaactcccaaacaaaacaaagcaaaactacttacaaccacaaactacgcttcgtaacctagatagataacgcaggtgacactatctatctaggttgagctcagctctgcccatgcttttcctgagcggctcttggaagaaaagctacaaagcccatgacagcctccgcctggccagctgccactggcatctcaaggctggcaaagcaaagtgaaagcgccaacccggaacttacggagtcccacgagggaaccgcggcgcgtcaagcagagacgagttccgcccacgtgaaagatggcgtttgtagtgacagccatcccaattgccctttccttctaggtggaaagtggtgtctagacagtccagggagggtgtgcgagggaggtgcgttttggttgcctcagctcgcaacttaactccacaacggtgaccaaggacaaaagaaggaaacaagactgcagagatccgcaccggggagccctgcagattctgggtctgctgtggactgggggcgggactgcgactgggcgggcctgggggcgtgtccggggcggggcggtcccggggcggggcccggagcgggctgcggttgcggtccctgcgccggcggtgaaggcgcagcagcggcgagtgggtgagtgagacgcgcgggcggaggggggctgctgccacggtcggctcgcgggccggccggctccgggtaccagcggggtttttttctccttcgaggtgaactcctccctgtcccccgggcgaaagagcccttggccttgcaggagttgcgggggccgcggcggtgcggaggggatggggatgggcctcatctttgctgtccgcccgcgctccccgatcccgacccggagcgtctcccgggcccttgagggaaccctccgggagtacggcgagcgcggcccccaccgccacaagcctgggccccaggggcctggcccggcgacagctggtgggtcctgcgacccagtcaggtctcccgagggtccccgcccgggaggagaaagcgccggtgggatggagtaaggacggacagaacaacacgcaggcaggatttcgcagaagtttgcaaggagtgcggatgcccacttacatgggctgctactcttaccaggttgttccccagttctgtgggacgtgacctggttgcctcacagctccgcggttgtacagacttattaaaggaagtgaccattgtgacttgggcatcacttgactgatggtaatcagttgcagagagagaagtgcactgattaagtctgtccacacagggtctgtctggccaggagtgcatttgcctgggagggattggttgcgctttctggtgtggggactattaggctcttgtagagttttgtcccggcagatggataaatttcttgttacactgttcccgttcgtcaccagttgagaaaaacgggtacacagtctgtctcagtagtacttttactttatattaagggcccaaaagggactggaaaatactttaagatagaatcgttagtccacttggaaaacttaaaatatgagagagagaggggggggggagagagagagagagagagagagagaaaggaaggaagaaggaggaagaggaggaggaaagagattgagattatgttaataatatggaatcagaatatttgaaatatagtaagcgtcccctcagttaaagaggacattccaggaggcccccagtatagcctgaaatctcaggaaacgcctacatacacccatcgtgtggatataggtgttttcccttcattacatttcatacacagatgttaaagtttagaaagtaggcacaataagagattacaaataactgataataaagtcgagccattgcagctgctctgtaaaagtcctgtgaatgtgatcgctttgtgtttcaaagtaacttactgtacttcacccctgttaagcaaaacaagattcacctgaacgcaggcaccttggtaccttggcagacaccagatctgataaccaagaggatggagaagtagtggcagacagtgtggagagcatgaatatgctagacaaaagggtgaatcataacctaggagcagaaagcaggtatttcatcatcctccacagtaaaaacctatgtcacgtaaaaaacctacaagtagtttttcttttactctttttgaatgaaagcttgctacaggcactgaaagttaaaataatctgtggatcaggaggaacaggggttttctgtctgagtcactgctgactagcacctcagtgaccattggcactgtgggaaaccccagagtcagttggaaacttcgaaactaaaggtgacggtgttcttatttcatagaacacaaaaaataagaggggttacagcctgcgctgcagactggacattcaacaagcatttaaatttctgggagacaaatgtaaatataactttaaaagttggtaaaatactctgtttggctatgttggccatccaatgtttgcttttagaaaatgactgaatggataaaacgtctatcttttgagcctgccctagacccccatgttgagtgaatactgtccaagtgttaggttagccggcctgagaaacttggatctaggcaagatggcacagtcctggtgtcatgagtatgcatgtgagttttggctgaaattgaacatttgtagagaatgacaaaggctggtctggcaagtagtccactgtctttacagtggtcttggttagttcctgtttggctgagagggctggttgatggctgtcctgcccctcttcccacaagtggaagccttatggtataattcttgatcacagtagcagtaggcaaatgaacttcctcaaagcagcctggaaagctgatttttttttctttctttctcttttttttttttttttcacaaggttaaagaaaaaacaaagggcttcaaatgtgccagtctgctaacagtgttaacatgtttattaacataaataaactttattagtttttggaagtattggttaagccctcgtgacccctgaactcggtttatagagtgatgagtcgtagcctcactctggtttggactctggcttctctcagaagactctgtggctaatgttaaccttctgaagtagccagaaaacatataagcaaaagtctgtgaggttgaaatgaattttttggccacatttgtatatgggttcccaccaatgctaacttcaggtgttagtaatatcagactcacagcttccctgattacacttcgctataagactttattttttaggtcataggaatttcccctttttcatgattcctaaatcatgaaataacatagtctaaaaatacggtattcctgaaataaacaatttctaagttttaagctgcgtgctattctgaacagtctgatgccctcttgtagcttttactgtgtcctaccccgggcatggttgattcctttgtccaaacatctgtctgttgtatccacactggattgcaccacctgcgtgctagtcagtcactcagacattttagttataaggtagcttatatttactccttattttatttaataatggcctcatagcaaggcggtaatgatactggtaatttgggtttgcttaagaggagccatgaagtagttttaaatgaaaaggtgaaaattcccactatagtttggagggggaggctatactggtactactacgattcacggtaagactaaatcttctgtgaaattatgaaggagaaaaagttacactggtctggtcttgctgttggattaattttatagttataaccactgtacatgataaataaccctaaaacaatgaatttgtaggtggatggcataatctgaaaaccatgttctgagcagttgatggcagcaggctgtgctggaagtgttaggcatatttatagatttcagcccaagttctgaagaggctggagagatggctcagtggttaagagtgcttgctattgcagaggacctaggttcctctacaggcaccaggcaagcgtgggacacactgagatacatacagacaaaacataaaattaaataaattgtgcataataatactagtaatatatgagtaaaataaggataaatacacatcataattaaataaataaattgtaaagttccctagaagtgagggtcaccaagccattcacaagatggctgcgctgatgcagggatatatgtgaactagaaaaaggtcaaacttaacagagaagttccaaggcatgctactgcaggcttggctagcatgcttgacctgcagaaatgctgacggccactgggaggttttcacaaatgaggaattagaagaactttttttactaatctccagaaaaaaaaaagggaagaagaaactgaagcagcctgtgatgtggaccagaaacgcagtgacagtaacatgtgtgacattgcaaaggcatgaaaggacagagctgtggaatacagacctcaggtggagctcagcatagagtcattcggggattatgcctgctgcagcaacaaaaggatgagctcaaaagagacaccgacttctgaatgcagtgggtgtttgttttgttttgtttcaaatgaattgggcagaaaactttccagctgtggaagcttctgaaccgtcccttgctgctgacatctaagcgtccgctgtgtcccagctcagtgatctagggtcttccaaacagatggtccggtgctgagcactttgaatctcaatcctgagtttctaccacgcctttggccatttaattcccagataaaagacacatacaacctttatatttataataaaccttagtcagcacaagagctgagcaaatatctgtcctctatgctattatatctattacccagccaataaccccattctataatttgctgtgcttcatctgggctgctcttaacttcagtcagccagcccacgtggccattattttaagatttttttaccccatagtgtcttctcactttactttacatttttctctctctcctcatggttctcctctgaccccaagcctaggaaccctaaaccccacccatgtctcttctgcccatctattggctgtaggcatctttattcaccaatcaggataacttggaggcaaggttaagtagtctcctgggtctaggtgctgtctctgggagcaaccagtatttagcatagcaaaagaccagacctccacaatgatcactctgaccatcggggcagaaggcacctactagcctgtgccactcacctcactttgttgaatcacatcttatcctgtagtgtgtatcactgcctgttatcacaggaaaaagtgagtcccatcaaataagatgtttcagaaagagaccatgttcatataattatcattctggtaagcttttaatggttatattttgttattaatctctttgttcctattttgcaaattataccttacagtaaatatatatgcatccaatggggtctttgaattcctccccggggagtaggaggactctttgaggatgggctgcatttaaagctaaacaacgcaacatgacctttagtccttatagatagcctagagatgagactaaataaaagaaatggtatataatgctttaagtttcccaatcagcttaaaagcttttcctataaatctttaagattatgctctggggctcaatactgcttcaagaagggcttttcttttgtatttagaattattcacctttttaaacaaaaggagaaaatggaatagaaatatgtttgcaacataattttatgactatgtgtttatttcgcgtgttctgtgggcctgcagtttgctgctgttaatgaggacaacagtggcaccaatacagtttccactcagattacattctctgttccctttctgaaagctgccctctccactgggcccaaaagagtcagtatcttaaacaagctgtacaacttagataaccatggtctcttcagactagttaattgacatatattaaaaagtaaatagtaccaaagtgaatttctgaaattaaaaatgaacatttaaaaactctaggtaaactattccttagagttaagtgttttgccaagttctgtaatcataatatgatagaaacgctcactcagcattctaaatatagaagttactccttcgcatgacactctaattcttgataaggtggagaaagagagagagagagggggagagacagaaaatatggtggttcaaggaccatttgagggaattagttatgttcttccgtcctctgtggatcttaggggttgaatacagtcattgagctcggtggatggctgtcctgttgaaaggtctgcccagcagagcaaatagacttttttatttacatggacatccgtttgtgactaatctaatgttcactcccaaagtaatcacacagacagagaggtagcttccttcagtactcttaccttacatgaatcctaccattttgttattttttttccactttaaatctttgattatgtgtttttaattagaaaatttgcatacaaatttccatacagtatgtagaattgactgtgtttgaatgggtgaagatccacatgtgtaaccctagctctggactggctctgagcttgtttgctcttctcttttgtgttctgagtaactgaaactctttcattttagcagcttagtatgcgcccttcacattgctgtgctgcctgctgcactaacattactcctttgcttatgttccccttcctgattcagtgtcattttaagcagtagtactggacctcagtaccttagccggagctcactgaggtgacagggctgaggctctgctgctgtcttttgagcttacctctttttaatgttttatggtatttctgctgccaggtttgggggttttgttttgttttgttttttgttttttgttttttttaattttctaggaacacctagaaaacacaaactaggaaacttaaaagagcagcgtcttgttccctgcgttctagaaagtccaagcctaatgccagtgtcatggttgtcaggaacatgagcctctgaaggcttcttgggaaacctttcttgtctcaacacctctggtggcaagcagtagtccatggtactctctctgtccacggtcagcatcccagtccctgccctttatctttgtgcagccgaccagctttgctttagtctgtctccttctcaggtctccttccccgctcctcttaagcacagcagtcattggattagagcccatccttccctcggatggcccatttgacctaattttacgtatttgtaactaaggtcccatttacttacacagggccctccccttcctgttttgttctttagctgaaatggtttggagaccaaatatccaatcattacaattgtgcacaagctatgttcatttggaggtaataaaggctcattctttgcttctattggtatgtgacatttttctaagtcacttggggtttgatagatatctttaaatggctgaacctgatcactgttcttttgtatgtccctgtttagctattgcaagcgttcggataatgtgagacctggaatgcagtgagacctgggatgcagggatgtcgactatctgccccccaccatctcctgctgttgccaagacagagattgctttaagtggtgaatcacccttgttggcggctacctttgcttactgggataatattcttggtcctagagtaaggcatatttgggctccaaagacagaccaagtgcttctcagtgatggagaaataacttttcttgccaaccacactctaaatggagaaattcttcgaaatgcagagagtggggctatagatgtaaaattttttgtcttatctgaaaaaggggtaattattgtttcattaatcttcgacggaaactggaatggagatcggagcacttatggactatcaattatactgccgcagacagagctgagcttctacctcccacttcacagagtgtgtgttgacaggctaacacacattattcgaaaaggaagaatatggatgcataaggtaaggggcttttgagcttgatcatggtagcctggccaatgaaagtttttttctggtacagttacacttaagttttggaaattatatgctgctaacaccagacagctgttatgttgtgtctcctgggcacagaaagccctgctctcatgcctggggtcttcacagtcctaatggaaagtaagatcttataaacattgtgtctgagtttgttctggaagctgtgactctaccttcttgttttcctttccctgtgtgactttgtcctttgcttacaacagtgcaaaagtataaatattctcagattttgataagctgtcagccacacagccttagtaactaagctgctgtcccacgctcccagttctgtataacgaggatggaccaattagattctaaggagttattcctttcaatttgcaaatttagctaaaggaaatattgttttctcctgatatttacattgcttttcattttcagcatatctaaagaacaaacctaattctccttcctactttctagtttaatataatcctaaaaatccattaaaacatgactaattctataaggcctctaacctacaaagggaagtagcattttgaaaagaatagttttctctattatacctattcatgcagacttccttccttatttctgacatacttaacaaaaatcatttagattcaaacagtttagctgcaggtgatattacagacaagtaatcccagtgctctatctagtctgaggcaaaaggatttgagctcagtgccagcctgttctatctacctggtgagttccagtcccataaataaacaaactaaaacaaccgttcctctgttcctcagatgcgagtcgatcttgtttgatttaaatagtgtgtaattattttcttttgaagctgcaggtgttatgtgggctgttttagactaaattctctctttactgtggagtaaagggtgctgtgattgtatttcatgttctctgcgagagcttgaacttgttgggctaatcgcttgtctccatcctgtctccccacctgcgtaaaaagtattttcctgtgagctgtacatgatagagcatatctacattgaaaaatgaacgagcatcaaaatggatttgttaaagtaaattttctttttcttaggaaagacaagaaaatgtccagaaaattgtcttggaaggcacagagaggatggaagatcaggtacagtgcatatcacatgctgcctgtggcaggtcctctttgcttatgtcggtataaagttggtgggtacttctggtaaggacctgaggatacattcatttgacggaaggagcctgaaaatgagtattcttgttaagctgtatagaatgaactgaataaaaatttctgcagcctaagtttgaattttaaaaaaatttaattacatctacaaattagtatttggccaccctttttcaatcagcaagaatatgtttgaggtcatttatttgtagtaaaattgcatgcagtttatttattttattgaaaataggttttttaaactatattttctgattatggttttccctcctctgaatcctcctagaacctccacctacccaaatctatatctgttctttctctctctcattaggatacaatcaggcatgtaaaataatagtagtagtagtagtaataataatgtaaaataagttaaagtaaaaacaaaccagagtaggacaacataaatagaagtagaaaagagccaaataagaaattcaagaaacacatatagacacagacacaatatttgcatacacagaaattgcataaaaccgcaagactggaaaccataatatgtatgtaaggtggagtgggaagccctgacagcacagtgagtaaagcactttcaaaaacaccactgactttgtgttgtgttgcctgtctgctgggcatgaggcctggccttagagagtggtgtgtatacccaggaagacttacataaacacttagcttttcatttgtgacctgatagcaattggaaatagtgtctgggctaggcattccggcttattgccacttcccctcagcactgaggccccatctgaatcggatccgtgcaacccttgtgcatatgcagttttaaaagttatcccttctgcaactatgctcacaggagttgccgtcttaagggagtgagcacacccctgaggcatggctccaggggtgcagagccagccataggcacagttttttttaaaaggtttatgttgtagttttgaaactcaaatttatgtgtatttgtggcagattgtttgaatgttgaaatttgccagtaacatcttttatcttcttccctttagcctggcatgccacccaccctcatttgtccttgtcaaactccagtaattaaacatggctatgtggccttttctctcattttccttagcatggctaaggagaatgggacttaaaaaataataatcatcattttaagtatgtctgagggtttgaggatatagtggtagaatatctgcctagcttccatagcttgatcctacatttgatccctggcaaaacacacacacacacacatatacacacacataaaatgacttttataaagttagtgtgctgtgctgtgatgaacagtgccataggaaatattcttggaaaagacctgaaactaaatgctctaaaaggtctaatctttacttgcttgctgatcgttaagcagagtctccaagtataaagtcactttcaccaacctctgcactggatttctggagtaattagggagagtcatttcaatataagaaaatttagtaccaaataaaattttcattcagtgaaattttgtttttgaaagtaagagcccactgtggtggtttgaatatgcttggcccagggagtgtcctgtaagatttttgttgttgttgaactccattgagacttatgttgacaataaatgcctgagagtccatgtctaaaatgctgtacctgtctgaacccaacggagataaaacttaccatttctgaaaaggatgaggtgttttatttacatagctgatgtaatgtgcttgcaacagctctattatgaatcttaatactacttcagtatatcacagcacttcaggaaatttaacatacattgtttaattccatgtcttaattgtatttgtaaacagacatttcagcagttactctaaaaagtagaaataatgagtggttgcttctggtcattaggatgaaatattgaaatgataaaattttctgggctggagagatggctcagaggttaagagcactgactgctcttccagagatcctgagttcaattcccagcaaccacatggtagctcacaaccatctgtaatggggatctgatgccctcttctggtgtgtctgaagacaactacagtgaactcatacaaataaaaataaataaatctttttttaaaaatctatatctgcataggcatttctagattaggataaattttccaaaggaaataagcacctccatgataagggcattggaaatgaagcccccgcccccacccccggtctgcacgtgtgttgaggatgagatctagggcctccttatacatgccaggcagctgttctgtcaccaagtggaatataatcctcaacccttaatttgaggttctaactttaaaatagatgtgaggggtttaaataatcatttcatgaaacttaaatgagcaagtttattactgaggtgagtataagtaattgataattttaaatatatttagctgagattgatagacacttggcaatgtcagcatcttatttaggtgatcataaactgatgggagaaatggtaaatgttagggggtgtcgctcatgtcacacaccgcagttatgctgcaaacaagatgccgggaaatagaaattcaaggtcttgttttgcgggtgcagactcttctgtctcactgattctatgtggtaacttcagtatgcatttggatagattatgtcccattttgaatgtggaagctggctgttgagaggagacttcctggtgaattcctttttctaagcattaccatctgtcttagtcagggtttctattcctgcacaaacattatgaccaagaagcacttggggaggaaagggtttattcagcttacacttccacactgctgttcatcaccaaggaagtcaggactggaacttaagcaggtcaggaagcaggagctgatgcagaggccacggagggatgttctttactggcttgcttccctggcttgctcagcctgctgtcttatagaacccaagactactagcctagggatggcaccacccacaatgggccctccccccttgatcactaattgagaaaatgccccacagctggatctcatggaggcatttcctcaactgaaactcctttctctgtgataactccagcctgtgtcaagttgacacacaaaaccagccagtacaacatcttttcacatttaatttttctcactttaaacgtggcctttaacaagcgcttataaaaatgcttaagcttaaatgttatttaagcttaatatacttaatatacagcactgtagcttaaatgttgcatgtgagagtatatgataagccatgctcaccaaggaaaagaagcttaaagagcataaaaaccctgacagcggtttctgagtgggaggctcggggactgtgctgagcaattccaaccaagggtgttttactctctgcctccatttgaaatgtttttcctgcacaacctacccaccctgtgatttcgttcactcgattatgtttgatctagggtcagagtatcattcccatgcttactggggaagtcattcctgtaatggagctgcttgcatctatgaaatcccacagtgttcctgaagacattgatgtaagtgtcatgtatcttttatgggttcccttgagtggtgagtgggtggatgtgtggtgcatgtgcgtgtgtgtgcttgcatactgggaattgaacccaagtcctcaggaagagcagccggtgctcttaagcactgagccatctcttcagaacctcttccaccagtttctttgaccatttgttgagaatattccagtcacacattttccgtgagtaaatctctctaatgctgatttgtcattaagctcagtctcctaattctgatagctaagaagggtaaattattaaaaagtgccctttactcttcctggccaattcccctttgttcttctgaaaagtgcatagacagcatcactttatagatcaccttgatgctcgtgagagggctggctcgtgctggctctagacttcggcacacttattaagagttctcccaacactgtaaacagactaatttttatattgtgcattttagatagctgatacagtgctcaatgatgatgacattggtgacagctgtcacgaaggctttcttctcaagtaagaattttacttctttttctgaatgctaagtaaagcagattaaaaatcttaatgctcacccatgacaagatttacagggaaaagatggtagaaaacctacttcctccaattatttagggtcaacatggcacatttgagcttacacgtgttgttctcacccatacaacagtggcatatctgacattactcttcccacagtctaaaaaggcagagtttccgtagtacccagggaagttctggtctgtgtttgggtctggtttcttctttcaattctcactaagtataacccttaggaatctatcaagttgagttgcattttaaattcctgtgaattcttcaggtctagaaatggaaatcattcatattttagactgacatttttcatcttcttgtgtaatttaacatttaagaacttgagctctaatatcagactgtctaggttacaactgggaaaacttggtgaagctacccaaagctgaacctccattttcttacctgtgaaatgtgaacagtgataacagctagtttcttgggtccttgtaggcaccaaatgacaggataatataaagcacctaggacagtggagccaatgagccaggagccagtgtgccctattatatctgctctaagaaagacagtaagtggaatagccaatactgactgtcttagtcaggctttctattcctgaacaaaaaacatcatgaccaagaagcaagctggggaggaaagggtttattcagcttacacttccacgttgctgttcctcaccaaaggaagtcaggactggaactcagatcaggaaacaggagcagatgcagaggccatggaggaatgttacttactagcttgctttcttatagaccccaagactaccagcccagagatggtcccacccacaagggaccctgcccccttgatcactaattgagaaaatgccccacagctggatctcatggaggcatttccccaactgaaactcctttctctatgataactccagcctgtttcaagttgacacaaaaccagccagtacgctgaccgagcagctgtgtgttcctctgcagggctgtgttctctgtttgtccctcatctcctgttgtagtctcctttacagttacagactgtcatcagtaacgagagagaagtgaataggattttgttaaagtgtttacttctatgtcacattcccttcctataataagctcacagtgaaataccaggtgaccgtgcttaacggcatctattacctaactggggtatctttttccttaaaatggatttaattttatgtgtgtttgaatacctgcatatgtgtatgtacaccatatttatgtatgcctggtacctgaaaaagggaaaagagggctttggctttcttgaaactagatggttgtgagtctccatgtgggttctggattgtctctgcaagagcggcaggcacactttagcagtgagccgctcctgtcccgagttgtcttaagacctgtgaaaggtccctaaaaaatgcagggttttacccgaataaaagatgacatcatgcagatggctttggtgttcatcaagctcttgtgtgttgtcctaaccttgctgggctttgtcgttgtgaagctgtaactccgtcaatgttttccttacctacagtgccatcagctcacacctgcagacctgtggctgttccgttgtagttggcagcagtgcagagaaagtaaataaggtaattcgttctacagttgaacatgatctgacttttatcatcactagcatatcatacattatcatctaaacagtaggctgcaattgaaataaccccatagtataaggaagcaatgtaattttaccaaatttctctgacaccctctagcagaactgactctaatagaatgagtaagaattcaattaccaaattaattttgatactcttttttatttttgttattacttttttattttattttaattaggtattttcttcatttacatttccaatgctatcccaaaagtttcccataccctcccacccactcccactcccctatccacccactcccctttggccttggcgttcacctgtactgagacatataaaatttgcaagaccaatgggcctctctttccaatgatggccaactagaccatcttctgatacatatgcagctagagacacgagctccagggggtactggttagttcatattgttgttccacctaaagggttgcagacccctttagctccttaggtactttctctagctcctccattgggggccctgtgatccatccaatagctgactgtgagcatccacttctctgtttgctaggccccagcatagcctcacaagagacagctatatcagggtccttttagcaaaatcttgctagtgtgtgcaatggtgtcagcgtttggaagctgattatgagatggatccccaggatggcagtatctagatcgtccatcctttcgtctcagttccaaactttgtctctgtaactccttccatgggtgttttgttcccaattctaagaagggacaaagtgtccacactttggttttcattcttcttgaatttcatgtgttttgcaaattgtatcttatatcttgggtatcctaagtttctgggctaatatccacttatcagtgagtacatattgtgtgagttcctttgtgattgggttacctcactcaggatgatgccctccaagtccatccatttgcctaggaatttcataaattcattctttttaatagctgagtagtactccattgtataaatgtaccacattttctgtatccattcctctgttgaaggacatctgggttctttccagcttctggctattataaataaggctgctatgaacatagtggagcatgtgaccttcttaccggttggaacatcttctggatatatgcccaggagaggtattgtgggatcctccggtagtactatgtccaattttctgaggaacggccagactgatttccagagtggttgtacaagcttgcaattccacgaacaatggaggagtattcctatttctccacatcctcgccagcatctgctgtcacctgaatttttcatcgtagccattctgactggtgtgaggtggaatctcagggttgttttgatttgcatttacctgatgattaaggatgctgagtttttttttcaggtgcttctctgccattcggtattcctcaggtgagaattcttggtttagctctgagccccatttttaatggggttatttgattttctggagtccaccttcttgagttctttatatatattggatattagtcccctatctgatttaggataggtaaagatcctttccaaatctgttggtgacctttttgtcttattgatggtgtcttttgccttacagaagctttgcaattttatgaggtaccatttgtcgattctcgctcttacagcacaagccattgatgttctattcaggaatttttcccctgagccaatatcttcgaggctgttccccactctctcctctataagcttcactgtctctggttttatgtggagttccttgatccacatggatttgacattagtacaaggaaataggaatggattaatttgcattcttctacatgatatccgccagttgtgctagcaccatttgttgaaaatgcttttttccactggatggttttagctcccttgtcaaagatcaagtgaccataggtgtgtgggttcatttctgggtcttcaattctattccattggtctacttgtctgtatataccactaccatgcagtttttatcacaattgccctgtagtacagctttaggtcaggcatggtgattccaccagaggatcttttatccttgagaagagtttttgctatcctaggttttttgttattccagatgaatttgcatattgccctttctaattcgttgaagaattgagttggaattttgatggggattgcattgaatctgtagattgcttttggcaagatagccatttttacaatgttgatcctgccaatccatgagcatgggagatctttccatcttctgagatcttctttaatttctttcttcagagactttaagttcttgtcatacagatctttcacttccttagagtcacgccaaggtattttatattatttgtgactattgagaagggtgttgttttcctaatttctttctcagcctgtttatcctttgtatagagaaaggccattacttgtttgagttaattttatatccagctacttcattgaagctgtttatcagatttaggagttctctggtggaattcttagggtcacttatatatactaccatatcatctgcaaaaagtgatattttgacttcttcctttccaatttgtatccccttgatctcctcttgttatcgaattgctctggctaagacttcaagtacagtgttgaatagggaggaagaaagtggacagccttgtctagtccctgattttagtggggttgcttccagcttctcaccatttactttgatgttggctactggtttgctgtagattgcttttatcatgtttaggtatgggccttgaattcctgatctttccaagacttttatcatgaatgggtgttggattttgacaaatgctttctcctcatctaacgagatgatcatgtggtttttgtctttgagtttatataatggattacattgatggatttccgtatattgaaccatctctgcatccctggaataaaacctacttggtcaggatggatgattgttttgatgagttcttggattcagttagtgagaattttactgagtatttttgcatcaatattcataagggaaattggtctgaagttctctatctttgttggttctttctgtggtttaggtatcagagtaattgtggcttcatagaatgagttgggtagagtaccttctgcttctgttttgtggaatagtttgtgaagaactggaattagatcttctttgaaggtctgatagaactctgcactaaacccatctggtcctgggattttttttggttgggagactattaatgactgcttctatttctttaggggatataggactgtttagatcattaacctgatcttgatttaactttggtacctggtatctgtctagaaacttgtccatttcatccaggttctccagttttgttgagtatagccttttgtagaaggatctgatggtgttttggatttcttcaggatctgttgttatgtctcccttttcatttctgattttgttaattagaatactttccctgtggcctctagtgagtctggctaagggtttatctatcttgttgattttctctaagaaccagctccttgattggttgattctttgaatagttcttcttgtttccacttggttgatttcacccctgagtttgattgtttcctgccgtctactcctcttgggtgaatttgcttctttttgttctagagcttttaggtgtgttgtcaagctgctaatgtgtgctctctctagtttccttttggaggcactcagagctatgagttttccccttagaaatgctatcattgtgtcccataagtttgggtatgtagtggcttcattttcattaaactccaaaaagtccttaatttctttcttcattccttccttgaccaaggtatcattgagaagactgttgttcagtttccacgtgaatgttggctttctattatttattttgttattgaagatcagccttagtccatggtgatctgataggatgcatgggacaatttcaatatttttgtatatgttgaggcttgtttttctgaccaattatgtggtcaattttggagaaggtaccatgaggtgctgagaagaaggtatatccttttgttttaggataaaatgttctgtagatatctgtcagatccatttgtttcattacttctgttagtttcactgtgtccctgtttagtttctgtttccacgatctgtccattggtgaaagtggccatctttatagtcactgaagacatacaaatacatattcatatcaactggaacaaacctaatttctttttaaatgttttacatggaaataagttaggggttgttatttgcattacaaagttactcatccctttccttcttttctttttttttttttttttttttttgagaacaagcctgtgtacttatatgaactttaatttgccaaattcataattcttattcaatcatttatgacagaatgctaaaactctcattatattttagctaggcatttagagctgttatgtgtaaccccaaaaagtagctttccacttgagatgctgaaggccttgggttccgtgggctgtcatcatggttggctgtatgaaaagagaaaggctccattgtttgggcatcacttaaatattttttcacctttcatcttcttttaggttaagtagcttgtccttgatcatttcatttttgagagacaacttgccactactctagttgaaaagtgctgtcttgacgctgtctctggctgtggtcagagtccagcagagctgcacagctggttacctttctctgtacagctctaggccaactcttcttactggcgaccatttctaaatccaccattcacttgttccccatgaaagtgagtagggttttttctgtggaagattttgggcagtcctgttgccactttgcatcagacaatagttccctcattgaaacacgcagtttattctccagagcggtctgcccactccaaaggcagtaggtgctgggtagagatatgccaagtatcacactaggctatgactgctcactcagatcactcggatgaagctttcatggccaaatacagttgagaaagaacaaatattcttcacttagagagcaacaagagttattcaagtgtaacaagttctgagattccatgcagttgatttaccagctacttcctaaacttaactggccacaaaatccctttgtaagcagtatgttgttttgacccatgccctgtcaaaggatactccttacttgggaactgttttaatgatggcaacaaaaatttctatttaaatttatttcataagcaagcaaagatctttttacttcacattccaatgttgactcttttcctctagatagtaagaacgctgtgcctttttctgacaccagcagagaggaaatgctccaggctgtgtgaagcagaatcgtcctttaagtacgaatcgggactctttgtgcaaggcttgctaaaggtacacttgccgatcatttatcatgtgtgacgcaacaagtagagatggagggtacaaataatcactgagaggctttggaaagtatattgttagcatttaatgtctcatagttttagttgtctgggtactggtttgttttcatcattctgagcatgaagtgtatgtcttagggatttatagttcgtatcatgtatgaaacaccatggggtaatatttatatttcacttggttccctctagctatgtgtctggccccagtgctttccttgtaaatgcatgcttgaatcagactgagctgatatgataatgttgatgctccttttgcttactgagtggctatgaatatgcaccatacttactcattgtaagaaattaaaatgtctcttaaggatgtaaacatagcaaaatgaagcaaaacaaaagcgatgctgttttaggtaccctaactgaccttgtgtattcaaggagcattcctacttctgtgatgcaaaagctgtctacactgggcagatctacaaccagcattaaaccaaatagggaatcactgaaatcacgttatcaaagatgagaaacaagataataatgtctactttcacggcttttattcaggtctagtgctataagtttttgccaaaacaaaaatgaaaacatagactctgggctgaggctttcccttagcagaaaagtgcttacttgttgtgtccggccagcagatcacagcctgggttctagcctggaaaggcattttggaaacctggaagagaagaggggctaggtaacgagagaaagaacggagccaagtcaaaagcaactctgatcaaagctcaattttactatatcagcacgcagttataaaggaggggaagggggggccaatagcaaggcggcaggttccagcagtgggcgtggcagaccgattgagccggcaagctccttccaggtgtaaacagtggagccctaaggctgggggaggggaggctacacttagcatgcctgatgccctagatgccacctaaatgacaaatccagtccagtacaggatgtagagcacccccccccaaaaaattattttttttgtataccagaaatgaaattgctgagaaaaaaaaatgaagaccataattatactcccagtagctacaaactaaacagccccatagatgaagtgagtgatgtctgctgtgacaattatgaaatgaaagaagtaaagatgaacaaatgaagggaagacatccagtactcaggactgaaagactgctgctaaaatgcctatccaacccagagctctctgcagactctggacagatccgctctagatgtgaagatggtcttttttttttttttttttttttggtttttcgagacagggtttctctgtgtagccctggctgtccaggaactcactctgtagaccaggctggcctcgaactcagaaatccgcctgcctctgcctcccgagtgctgggattaaaggcgtgcaccaccatacctggctttttgtgaagatgttcttaacagaactagaaagaagtaccccttggtttgctgcccttctgatgcagtatccccaaaggctcgcatgcactgaacatttcatcttacctggtgccactgttgggaagtgatggaaatgcgaggaattgtagcctcgttgagatgtttctcattaaggcactgggggcatacctatggagcatacagtaggaacctggtttgcaacctctcccctctccatccaggctctcccctgtgcacctggccttggtgttctgccactccatgaacccaaagtaaagtggactatgcccttagactgtaacagtgagtcagaagaaacatttcctctttaaagctgagttttctgggtgctttgtcatgttaatggagtctgattagtacagaccctgagtaggcagggcaatcttatgcagaaacatcaaagctggtagcatagacatacctaatttcacaatagacactgatggactcagtctggagtacttacagtaagaatatacagcagagatacggagctctcttacagtggtgctctgggagaactggccgtcctgtgaagaaaagccagagtggctcattctcaccagacacaaactgagctcataagacgcttgaacctgagatcctggtcagcagccactagaagaaaacttaggagaaaccattcaacacgtcagtctggggaaaagggtggttttggttttggttttggttttttagtatattccccaaatcaaaaacaacaaaacccaaacttgacagatgacatcacactgcaaagcttttgcacaaccaagaaagcaacctgcagagtgcagtaataacccacagaaggagaggagatacttgtgggcagttcatcacacaggtcaatataagcaagtactgatagtgtggccatctccaaagaagatatgaaaataactggtatatatgaagtagtacttagcattgctgcgtatatggtaaattcaaaaccatgatgagatattgccccacttagatggatattatcaaaacaacatcaaaaagtgacaaatgctttcaaggatatggggaaagtgtacttgcaggaatttaaattattaatttgccattcaagaggataggatggcagtttaaattaaaaaactagaagtggtagagcagtcgcctagaacatacaaggttcagcactataataaatgagcaattagacatttgaagcaacaatctcaccactaggcaagtcctaaaagaaatggactcgcttcttcttcttcgggaaaacaccaaatggcagatgacgccggtgcagcgggagggcccagaggacctgggggctcaggattaggaggccgcggcggcttccacggaggattcggcagcggtcttaggggccgtggtcgtggccgaggccgtggccgtggtcgaggccgcggggctcgtggaggtaaagctgaagacaaggagtggatccccgtcaccaagctgggccgcctggttaaggacatgaagatcaagtccttggaggagatctacctgttctccctgcgcattaaggagtctgagatcattgatttcttcctgggtgcgtccctaaaggatgaggttctgaaaatcatgccagtgcagaagcagactcgggctggccagcggaccaggttcaaggctttcgtcgctattggggactacaatggtcacgttggtcttggtgttaagtgctccaaggaggttgctactgccatccgaggggccatcatcttggccaagctttccatcgtccctgtgcggagaggctactgggggaacaagattggcaagccccacactgttccatgcaaggtgacaggccgctgtggctctgtgctggtgcgtctcatccctgcccccagaggcactggcattgtctctgctcctgaagctcctgatgatggccggtatagatgactgctacacttcagccagaggctgcactgccaccctgggcaactttgctaaggccacctttgatgccatctccaagacttacagctacctgacccccgacctctggaaagagactgtcttcaccaagtctccttatcaggaattcacggatcatcttgtgaaaacccacaccagagtctctgttcagaggacccaggctccagctgtggctaccacataagggtttttatatgagaaaaataaaagaattaagtctgctgaaaaaaaaaaaaaaagaaagaaagaaagaaaagaaatggactcggtatgtggatgaagcccaggcaccttcatctgtgttgcagcacgagtcaccatgcaggatcagtctaaacgcccatgcacaaatgaatggtacatagccacagtgaagtgtttgaccacaaaaaggaaagtcagttgtgataagtgaaacaagccaggcacagaaagataaatgctgcatgttatcattatgtgtaaaggctaaaacgtttatctcatacaagtagaaggtaaatacggagactaccagaacttataaagagttctaggaaaaagctatagagaggctcagggttgaataactaaaattatacctaaaataactaaaaggatagcttacaatattctgtagcactgtagaataattgtgacagtttgttgtatttttctggtttgtgtatgtgggagagaaagtatgtggacagaggttgatatcaagtgtctgactctgcactgcattattttaggcagggtctctctctaaccattgaatggactggctaggcagtggtgccctaacatctacctgtccgtacatctcccaatactaggttataagtacactgggttttaagtacaggctataggtatagatataggctacaggtatagatataggctgctgcaactgattacatgggtgctgggaacctaacataggttgggtcctcatgtttacacagaaatcagtactgtgcctactgagtcatttccccagttctagtatttgttttttaaatagctagtaattggaattgtgaatgttcctaacaaaagaaaatgataactatctgagatgctagttatgataccctgagtgaatcacactttgtgtgcatgtactgaaattcattgtaccctgaaaatacaaaaattgctctgtgttgattggctagatgcatgtgtattagtcagcaatctctagagtaataaaacttagatatatgggatgtattagacttttggccttacaggccaagatccagctaatccatcagtggcaggctgtgaacagtaagtctaagaatccaatagttgttcagtccacaaggccgggtggctcagctgccttctgtatacagtggaatcccaaagaaataggcgccaaagctagtgaggaatggtcttgctagcaaagcgaaggtgaaggtaatcaggcagaagacaagaccttcctttttccgtgtccttatataggctcctagcagaacaagtggcccagactagatgtggattaaatgttttgggtttggtttggtttgatttggtttggtttggtttggtttggtttggtttggtttggtttggtttggcttttcgagacagggtttctctgtatagccctggctgtcctgggttgtagaccaggctggcctcaaactcagaaatctcttgcctctgcttcccaagtgctgggattaaaggcgtgcacaccactacgcccggctcaatagcattaaatggcatgtcttttcctatctcaaatgatctggattaaaagagtgtcttcctacctcaaaggtctggattagaagtggatctttctacttcagattaagttaaactctctcacaggtgtgccctctacttttggatttttggttctagatggagtcaacatgacaaccaaaagtaactattacaagtccacccaatatcaacttgatacacaatcatatctccttatgtcataattaatttccaaatgaaaacaataaccatgtcataaaaacacctaaacatgaataactattccacatacaatcagaaatgcattcattatatatttaaccaagtcctaattatgcctaacgtgatataactattcttcatacaacagcaaacatgataaatttacaataggtggcaatgtcttattcttttaatatctcaaacttaaatatgataaccattgatgttatcttaattgatgttatatcatatgataaagaaattgatgaaagaaagcacaaatgtctgtataaatgctttcttaagaaaataggacagaaactctgtcaattataatcatcttttctgcaactagtcatgtggccttagtatttataactaccttcctctgctaaaccattttgtattttctccacccttggcaagaacctcagcaggtcttggctcttttcctggaggagtgacccataccttcattccttacatgtatgtgccctttgtcatcctgcctggaccaggttgttgtaacattgactttaatcacaggacatcgtagcaccaacacatgccccaaaggatctcctgccctatagacataacctttcttacctccatagtggggaggcagtcccagtcctccttggtagtctgcatcagtcacgcctcctaacactgttattcctttcttagccggttgacttaagggcatcagaaggccaaagttgccagaggaaaatctgagcttccagttcaatgaatgtaatgttgttctaggcaagcagaactgaaggtctcaggaataggaagcaaacacttcccatggatcactacagggtgagagtgagtagaattattctcttttctaccacttgactcctggacctatggatcctggtatcaaagaaaatgtctcatatattgtacactgattcagagcatgccttctggaaaaccctgccccagcccttcatactgctgccatcaaattgtcacctgtgtcttcctggtaccaacttttgtcctggttagggttactattgctgtgaggaaacaccatgagcaccaaagcaacttggggagaaatgggtttattcagcttatgcgtctacatcacagctcatcatcaaaggaagtcagaacaggagctcaagcagggcaggaatctggaggccgtggaggaaagctgctgactggctcgctccctaggcttgctcagactgcttatagaactcaggaccaccagctccagggtggccccaccccgcaatggattgggccctccctcaggaatcacaattgccccacagacttacctacagcctaggcattttggaggctttgagtctgcctcctctctgatgattctagcttttgtcaagttgaagcaaaagtagacaggccttaaactcacaacaacccacctgcctcaattttctgagtgctaatattatatcaatttaaaatttaaatataacatataaagggcaatagaaaggactagattcatgtaatggatacaagttatggaagatgtgtgtgtgtgtgtctgtctgtctgtgtgtgtgtttctagtttaattctgtcatgatttttttcttgtaggtggtaggtgagtgcatggaatacatttgatactgaaagggtaaattgaatgtggagcctcacagcttctgttccacatgcctatgataaccgtagaaattcatggattagtatagacgttgagtctggttaattttggtgtgtgatatttatatatatatgtatatatatatgtgtgtgtatgtatgtatgtatgtatatatatatatgtatatgtgtatatatatatatatatatatatatatgcaagatttcttataattaagtttacaaaattaaaaactatcttaaaaattgaattcttgcaaataaaaatttagcttttggtgattggattcttaatatggttgatgtttacctagaaagttaaaagccctgagttcagtctccactttcacccccaaaatgaaaatcagcttttgggtttcagatcatgagctcagaattaaagaaaacacatttctaactttgcttttacaaatcttaattttaccaatttcctttaaagtcacaatgagatacacagtacttcctagcaccccttgttcaattagataatgtgatttctgaaagagctccctctacacagggcacagggcaggtgcaaaactgtgattgggtgaaatacctgcgagctctccaagcaaagccaggcctatttgctttagctgccacatcgggttcttagacccgacatcccttcccacctgtatcctccctaattccttccaaccccacaacactaggtaggagagaaagaaggttagtggtggaagtttgcacacatctttttagactatttcctactgattaggggtgttaggtccttgagacaagtccagtcttcattgtcaggatatctccaacttcttcttctcatctctttgctcacaaagtttatcacaagttgataaactacaacaacaggaaccagcagtagcaaggacatcagagttgtatagctttccagaaaatactttgatatacagtaattatcctagcctttaagagtgaaagatttggcagcctctgtgttctacactcagcataataccttgtatactgcaggtatttgctgcatggtaagtggctgcccagctacctagaaagaggtaaatacttttctattaacatacatattcatttagatataggaagaagataaaacaatggagaaaggcagtcataattttacagaccagcaagtaaacgcattaacttggcataggtctttgtagtctttttctgcagtgcgtatttcctgcagtgcccacaccctacagttggattgcacgtggcatgttctgacccactttttatggtatactgtgtactgtcactgtcaacacaaatggtagtggctggatttttatacagtatcagcttgaaggttatttctgaacaagccctgtaccagattcacaggaatatgcatctcttatcattactatattcttttaacaattgcttctctcagttggcatgtggtcagtgagttctctcttccttctgacaggatgcaacaggcagttttgtcctacccttccggcaagttatgtatgccccgtaccccaccacgcacattgatgtggatgtcaacactgtcaagcagatgccaccgtgtcatgaacatatttataatcaacgcagatacatgaggtcagagctgacagccttctggagggcaacttcagaagaggacatggcgcaggacaccatcatctacacagatgagagcttcactcctgatttgtatgtgacgcttggccttaggtgtcattgttaaacaacataaaacttctcatttatgagtaaaaacagtgcaagttgtatttaaaagaaaagaaatatgacaagcacatactcaggcactttttctttattttcttaactttaaggtttttttttttttaagatttatttattattatatctaagtacactgtagctgtcttcagacacaccagaagagggcgtcagatctcattacaaatggttgtgagccaccatgtggttgctgggatttgaactcaggacctttggaagagcagtcagtgctcttacctgctgagccatcttgccacccccaactttaaattttttatactattatttttagacagtctcactgggcctaatgacttacataggtggcctggaactcactatatagatcaggctagccttcaactcccagatatccacctgcctctgccacccaaatacttggattaaaggcgtgtgcctccatacctagcctaaatcttcatttcttaaaatactgttttgctaagataggtaaagatttcctcttaaaaataaatacttagcaaatatataccgatctcctaattacttaatgaagggccagcttaatagttatcagtcagttatcagtgccagcccctactgctgggaatttagtgtataacgttcattgtatggtagactgaagtaattctaagtatttttttcttgggtgtgactatcaaacacagaaaagtatttgaaatttataaagagaacaggttttttctttgcattttatattttgctatttatttcttaccagaagatgcgagcagcaaagtaaaaggcagtaagtgctgatgggtttggaggaacttgggattttaattataaaacttcaagaaagcatttcaatggtgttctagagtctaaaaaagaatagtgagaccctattcctgttctctccgatcaaccaagagcttgaaatggtgctagtccttagtatacactgaaaagacgctaagtgtggtcatcccggttggagggctttaggaagcagtgaccctggaccaatgggtgtcaccgtgtgtctgaagaagaaagcagagctgaaacaagaggcgcatggtagggacaccagcagccacagtaaactgctgcccagaggtccctgtgtggggctgcagaattaaaagaacccattctacacagctctgctgtgctctgttagtgctgagaaaggttgagaggaattgtttcagaagaggaatcgttcaaattgaactcttatgtcactagttcacatactggcaatcttggaaaacatagaaattttctcactgagtctgcgtgcctgcgtcttcctcgtgactaatatacttgaagtcctgtttatttttttagttgattgtttagaatctcttctcaggaaatgaggtaaacttgaatggatttgcaccatgttagtgtttttgttttgaatatgtttgtttggaagatttgaagaaaaagcaattgttcagctattctggcatgacaaaatcatgtcatgaattttagaattttatttccagttctaagtaaatgttttgaatataaaattgtcagaaatattttcagccacaagattatatcttctattattgtgggctcatgatagtatcagtgtggtttaaataatattcacttttgagtctgggaggtttgaggtttcagattcagggactcacacactgggcaattactgtaccactatgcagttgcttattagtaccacagagtaattcccagttaagttacttttaattttaacctttttaagataaaagcagtctgatgatacattaaagtcggacatttccttgaagatagtctttccttttccagcttttgtgatccagatctcattcagtaaagcagaaattgggaaatagtggacttaagttctaagggacccacaaaccccgtgactgtgctgtccgttttcagccagtaaccatgaagtgctggcgtcccttccagcgcccctttctccatttggtgcactcatccctcaaggctgagaggcgtgctgctctcctgtctatttccctcttccccatggttcctgggcagtgatgttgtgatctctaccatctgagtcttgctttgcatttatcttactgtgaaaaatgttatattttccctctgacatgaatataatagcctagggaaagacagaagtaaaacactgaaagggaatgggggctgagaaaaaaacagtcattagcttctgtctggccagcatgctgaagtgggtcacctcagttggccattttgtctgaacgttacatgccagccaaccttagctgcggtagtaataagttatgctgctggctcatacttacagatggtaagtctcttgacctgaggcaaacgtgtaaggtgacggttctaaacacactgatggacaggcacatgccctgcctggatagcctcaaaacacaaacagtgtacaaatgtacccttgcgttaaagtggatctatgtgcgtttgtgtttattttctgtgcattaagtatgtatatgtatgtgtgtttatattgtgcacattgagtatatgcatgtgtgtttacactgaatactgaacccacggcctcctgcaaactaagtatgcattccaaatgcacacatctgtcttcttacacatctgtttataaaacttcaacttttttactagagcaagaagttgtggaatgtaactctgtaaaaccgtttaatatctgaacctttttcttcttaggaatattttccaagatgtcttacacagagacactctagtgaaagccttcctggatcaggtaaatatgatgccacccattgccagacaaaagaacatcatatattttcttttaaaatatgtcccacagtgcctacagaatatataaaaagcaccaaagaattaaagtgctagaggcctttctaaagtctgtaaacggattcctctttgaattattaatgggaaatagcctgtatattaaccgttaaagcagcattctccatcctagtggctgcttcaggtccaaccctctgcctttagaatttttgtggttggtgaagacaggggtgtgctttcatttgtgttaattgaattgaaaatattcttaaaacttaggttgcttctgcttaaatggtagcatccttattgtctctgtttttaaaagtatctgatgagtaaacatctggagatggtactggattctatgcgacttgtttctatacgtaagcagagctttgtcataatagcatgctgggaatcaggccaagatcctgtgccatagacatagagttgagatgaggagaacctcgtgttcactgggacttgtgggtctgggtctgtgtgaggtgaggacagcctgtaatcccaagtctctgaagctgaaaagtcccctcctctactccacacaacctgaagtcattgacttagttatttccataataaaataaggagatattttaaggtagaatacaagatctaagtgcattaaactagggaatctgaaaaggggacagtgggtttccagacatttgccgctaccagagtcttgccctttggaaatcggaagaaatggctgtaatgggtgttgtgtgtcagatcctgtcaacaatgtcgcggaagctgcactgtcttgtgtccctgcaggtcttccatttgaagcctggcctgtctctcaggagtactttccttgcacagttcctcctcattcttcacagaaaagccttgacactaatcaagtacatcgaggatgatacgtgagtcctgctcctctagaggaaagcctttatgcattgacagttgctgttcgttccctttgaacattgtctgtattataatgcgggggtttttgtctcttttgttttgtttataggcagaaggggaaaaagccctttaagtctcttcggaacctgaagatagatcttgatttaacagcagagggcgatcttaacataataatggctctagctgagaaaattaagccaggcctacactctttcatctttgggagacctttctacactagtgtacaagaacgtgatgttctaatgaccttttgaccgtgtggtttgctgtgtctgtctcttcacagtcacacctgctgttacagtgtctcagcagtgtgtgggcacatccttcctcccgagtcctgctgcaggacagggtacactacacttgtcagtagaagtctgtacctgatgtcaggtgcatcgttacagtgaatgactcttcctagaatagatgtactcttttagggccttatgtttacaattatcctaagtactattgctgtcttttaaagatatgaatgatggaatatacacttgaccataactgctgattggttttttgttttgttttgtttgttttcttggaaacttatgattcctggtttacatgtaccacactgaaaccctcgttagctttacagataaagtgtgagttgacttcctgcccctctgtgttctgtggtatgtccgattacttctgccacagctaaacattagagcatttaaagtttgcagttcctcagaaaggaacttagtctgactacagattagttcttgagagaagacactgatagggcagagctgtaggtgaaatcagttgttagcccttcctttatagacgtagtccttcagattcggtctgtacagaaatgccgaggggtcatgcatgggccctgagtatcgtgacctgtgacaagttttttgttggtttattgtagttctgtcaaagaaagtggcatttgtttttataattgttgccaacttttaaggttaattttcattatttttgagccgaattaaaatgcgcacctcctgtgcctttcccaatcttggaaaatataatttcttggcagagggtcagatttcagggcccagtcactttcatctgaccaccctttgcacggctgccgtgtgcctggcttagattagaagtccttgttaagtatgtcagagtacattcgctgataagatctttgaagagcagggaagcgtcttgcctctttcctttggtttctgcctgtactctggtgtttcccgtgtcacctgcatcataggaacagcagagaaatctgacccagtgctatttttctaggtgctactatggcaaactcaagtggtctgtttctgttcctgtaacgttcgactatctcgctagctgtgaagtactgattagtggagttctgtgcaacagcagtgtaggagtatacacaaacacaaatatgtgtttctatttaaaactgtggacttagcataaaaagggagaatatatttattttttacaaaagggataaaaatgggccccgttcctcacccaccagatttagcgagaaaaagctttctattctgaaaggtcacggtggctttggcattacaaatcagaacaacacacactgaccatgatggcttgtgaactaactgcaaggcactccgtcatggtaagcgagtaggtcccacctcctagtgtgccgctcattgctttacacagtagaatcttatttgagtgctaattgttgtctttgctgctttactgtgttgttatagaaaatgtaagctgtacagtgaataagttattgaagcatgtgtaaacactgttatatatcttttctcctagatggggaattttgaataaaatacctttgaaattctgtgtatgttttagttcattatttagggaaaacgctgctgtgaaagggggcgtgatcagcttcctattctgcgacagtcgtgttgaacggaacccattggttttcatcttcgctcccccccccttggtttttcgagacagggtttctctgtatagccctggctgtcctggacctcactctgtagaccaggctggcctcgaactcagaaatctacctgcctctgcctcccaagtgctgggaggcagttgccccaccaactagtcttcttttttcaaagaagatatttaaagctaacgaataatgctagactcttacatcttaaaaaaaaaagaagagaaaagaaaagaaaaggtaatcacactgcccagtgtgtagtgcatgcttctacttccggtccttgggagatgggggcaggatgagacgctccagaccggcttccaatacagagttcaagacccactgagctacgtgaggctacacgagcctgcctttaaaaacataaagctaaagctttcttcttaacttccagtattgcaccttgattcccccttcaaatttcacatacaaaataattcttaaattctcttttgaaaaatgttctactgaggccagagagacagttcgcttggtaaaggtgcctgttgccaaacgtgataacctgagttaaatcatagccccacatgggggaggaagaaacccccgcagcttgccctctgatgccatgtatgcactaaaacacgcacgtgtgtgcgcacacattttttaagttcctattacattgatagtaatataatttaaactgatttattctccccaagtcattgatacgggtgtccaacgtaaaatccagcggctgaacaaagcacttttaggcgctttaagttggaaagcaagaaacggagattgacactgtcactccaagagaaaactcttcgtagtagcgagatcggctgtggagtgaagatgctcagaggctgggaacgcacacagctcaggagtggatagcatcccccagcctcaactcctaacactgggaaagcgtagggctctcagatgaggaaacaaaaccatacaaagctgctgcaagctaaacagaaaaatagtggcattacactaactgttgtggaattgtacagaccgattctcctcccaatctgccgagtgtgggcggcttgagagaatgaagagagctactggcctcaggtaacagtgcttcccacaggactgtctcaggctgccaccaccataaatagcattttagacgtgacagagctaaggcttgacacacagccaaaagctactcacattccatttcatccccagctgttctgtcatcgctaagcacagagcattcagcacagctcttccctgtggtgggtactcagcactgttgagttgaaaggattgaaaaaactcaagactatgttctcaaacatttttttaagctctttttaaaaccaccttagaatgaaagcttttgacttcttattaacatgcactaacttcatatacacatttagtgttattgtacaggcacgaagcatactctggtcagaacctgtctcctttggtccaccctccccaccgttttcagcttctattccaccttccatacgtctcaagatccacatgtgagagggaacactcagagccttgtctttctgtatctgggatatctcacttaacatgatattctccagttctgttccatccatttcattgcaaagagcaagatttcactctacagccaaataacacatttgtccatgtatatccgtatttttccttattcatctgttgaatggcacaagactgatatcatgggtaatatctat

SEQ ID NO: 12 - RNA, 3435 nt, Rattus norvegicus
  source 1..3435: mol_type = mRNA
cgtttgtagtgtcagccatcccaattgcctgttccttctctgtgggagtggtgtctagacagtccaggcagggtatgctaggcaggtgcgttttggttgcctcagatcgcaacttgactccataacggtgaccaaagacaaaagaaggaaaccagattaaaaagaaccggacacagacccctgcagaatctggagcggccgtggttgggggcggggctacgacggggcggactcgggggcgtgggagggcggggccggggcggggcccggagccggctgcggttgcggtccctgcgccggcggtgaaggcgcagcggcggcgagtggctattgcaagcgtttggataatgtgagacctgggatgcagggatgtcgactatctgccccccaccatctcctgctgttgccaagacagagattgctttaagtggtgaatcacccttgttggcggctacctttgcttactgggataatattcttggtcctagagtaaggcacatttgggctccaaagacagaccaagtactcctcagtgatggagaaatcacttttcttgccaaccacactctgaatggagaaattcttcggaatgcggagagtggggcaatagatgtaaagttttttgtcttatctgaaaagggcgtcattattgtttcattaatcttcgacgggaactggaacggagatcggagcacttacggactatcaattatactgccgcagacggagctgagtttctacctcccactgcacagagtgtgtgttgacaggctaacgcacatcattcgaaaaggaaggatatggatgcacaaggaaagacaagaaaatgtccagaaaattgtcttggaaggcaccgagaggatggaagatcagggtcagagtatcatccctatgcttactggggaggtcatccctgtgatggagctgcttgcgtctatgagatcacacagtgttcctgaagacctcgatatagctgatacagtactcaatgatgatgacattggtgacagctgtcatgaaggctttcttctcaatgccatcagctcacatctgcagacctgcggctgttctgtggtggtaggcagcagtgcagagaaagtaaataagatagtaagaacactgtgcctttttctgacaccagcagagaggaagtgctccaggctgtgtgaagccgaatcgtcctttaaatacgaatctggactctttgtacaaggcttgctaaaggatgcgactggcagttttgtactacctttccggcaagttatgtatgccccttatcccaccacacacatcgatgtggatgtcaacactgtcaagcagatgccaccgtgtcatgaacatatttataatcaacgcagatacatgaggtcagagctgacagccttctggagggcaacttcagaagaggacatggctcaggacaccatcatctacacagatgagagcttcactcctgatttgaatattttccaagatgtcttacacagagacactctagtgaaagcctttctggatcaggtcttccatttgaagcctggcctgtctctcaggagtactttccttgcacagttcctcctcattcttcacagaaaagccttgacactaatcaagtacatagaggatgacacgcagaaggggaaaaagccctttaagtctcttcggaacctgaagatagatcttgatttaacagcagagggcgaccttaacataataatggctctagctgagaaaattaagccaggcctacactctttcatcttcgggagacctttctacactagtgtccaagaacgtgatgttctaatgactttttaaacatgtggtttgctccgtgtgtctcatgacagtcacacttgctgttacagtgtctcagcgctttggacacatccttcctccagggtcctgccgcaggacacgttacactacacttgtcagtagaggtctgtaccagatgtcaggtacatcgttgtagtgaatgtctcttttcctagactagatgtaccctcgtagggacttatgtttacaaccctcctaagtactagtgctgtcttgtaaggatacgaatgaagggatgtaaacttcaccacaactgctggttggttttgttgtttttgttttttgaaacttataattcatggtttacatgcatcacactgaaaccctagttagctttttacaggtaagctgtgagttgactgcctgtccctgtgttctctggcctgtacgatctgtggcgtgtaggatcacttttgcaacaactaaaaactaaagcactttgtttgcagttctacagaaagcaacttagtctgtctgcagattcgtttttgaaagaagacatgagaaagcggagttttaggtgaagtcagttgttggatcttcctttatagacttagtcctttagatgtggtctgtatagacatgcccaaccatcatgcatgggcactgaatatcgtgaactgtggtatgctttttgttggtttattgtacttctgtcaaagaaagtggcattggtttttataattgttgccaagttttaaggttaattttcattatttttgagccaaattaaaatgtgcacctcctgtgcctttcccaatcttggaaaatataatttcttggcagaaggtcagatttcagggcccagtcactttcgtctgacttccctttgcacagtccgccatgggcctggcttagaagttcttgtaaactatgccagagagtacattcgctgataaaatcttctttgcagagcaggagagcttcttgcctctttcctttcatttctgcctggactttggtgttctccacgttccctgcatcctaaggacagcaggagaactctgaccccagtgctatttctctaggtgctattgtggcaaactcaagcggtccgtctctgtccctgtaacgttcgtaccttgctggctgtgaagtactgactggtaaagctccgtgctacagcagtgtagggtatacacaaacacaagtaagtgttttatttaaaactgtggacttagcataaaaagggagactatatttattttttacaaaagggataaaaatggaaccctttcctcacccaccagatttagtcagaaaaaaacattctattctgaaaggtcacagtggttttgacatgacacatcagaacaacgcacactgtccatgatggcttatgaactccaagtcactccatcatggtaaatgggtagatccctccttctagtgtgccacaccattgcttcccacagtagaatcttatttaagtgctaagtgttgtctctgctggtttactctgttgttttagagaatgtaagttgtatagtgaataagttattgaagcatgtgtaaacactgttatacatcttttctcctagatggggaatttggaataaaatacctttaaaattcaaaaaaaaaaaaaaaaaaaaaaaa

SEQ ID NO: 13 - DNA, 20 bp, synthetic construct
  source 1..20: mol_type = other DNA
gggtctagcaagagcaggtg

SEQ ID NO: 14 - DNA, 21 bp, synthetic construct
  source 1..21: mol_type = other DNA
gtcttggcaacagctggagat

SEQ ID NO: 15 - DNA, 24 bp, synthetic construct
  source 1..24: mol_type = other DNA
tgatgtcgactctttgcccaccgc

SEQ ID NO: 16 - DNA, 22 bp, synthetic construct
  source 1..22: mol_type = other DNA
tgtgacagttggaatgcagtga

SEQ ID NO: 17 - DNA, 25 bp, synthetic construct
  source 1..25: mol_type = other DNA
gccacttaaagcaatctctgtcttg

SEQ ID NO: 18 - DNA, 21 bp, synthetic construct
  source 1..21: mol_type = other DNA
tcgactctttgcccaccgcca

SEQ ID NO: 19 - DNA, 30001 bp, Macaca mulatta
  source 1..30001: mol_type = genomic DNA
aatctctaagcaattttttggggaagaaagaattgcaattagggcatacgtgtagatcagatggtcttcggtatatccaacgacaaagaaaaggtgggaggtttcgttaaaaaagagaaatgttacatagtacttttagagaaaattcactggcactattaagggtctgaggagctggtaagtttcaattggtgagtgatggtggtagataaaattagagctgcagcaggtcatttcagcaactatcagataaaactggtctcaggtcacaacgggcagtttcagcagctagacttgaaagaattacactgcgggagcaatgtcatttgtcctgcatgcttttctaccccctacccccacttttttagttgggtataacaagaacgacccaaattgtatgatcaactttcacaaagcatagaacagtaggaaaagggtctgtttctgcagaagatgtagacgttgagagccattttatgtatttatttctccctttcttcatcggtgaatgattaaaatgttctgtatgatttttagtgatgagaaaggttaaacgccactcatctgtagtaagtgtaatctacacacttgcagaccaaaaggcataaggtttaaaaaacctttgtttttttacacatcaaacagagtggtataaatgctactcatctgtagtaagtgaaatctatacacctgcagaccaacgacgcaaggtttcaaaaatctttgtgttttttacacatcaaacagaatggtacatttttcaaaagtttaaaaaaaaaaaaaatccacatatcacaactagcaaaaatgacattccccagtgtgaaaatcatgcttgagagaattcttacatgtaaaggcaaaattgcagtgactttacaagggacctggggattcccgcccacagtgtggagctgtcccctaccagggtttgcggcggagttttgaatgtacttaacagtgtctcacggtaaaaacaaaacttcatccaccaaatatttgttgagcgcccactgcctgccaagcacaaacaaaaccattcaaaaccacgaaatcgtctgcactttctccggatccagcagcctctgcgattaaggtttgcacacgctattgcgccaacgctcctccagagcgcgtcttaagataaaagaatgggacaagttgcccctccccctttcacgggcctcgtgcgtcaacgtcatcgcatatagaaaacacacagacgtaacctacggtgtcccgctaggaaagagaggcgcgtcaaacagcgacaagttccgcccacgtaaaagatgacgcttggtgcgtcagccgtccctgctgcccggttccttctctctgggggcggggcctggctagagcaggtgtgggtttaggaggtgtgtgtttttgtttttcctaccctctcccctctacttgctctcacagtactcgctgagggtgaacaagaaaagacctgataaagattaaccagaagaaaacaaagagggaaacaactgcagcctgtagcgggctctggagcttaagagaggcgcgctaggcgccgggccgtgggcgtggtcggggcggggtcgggccaggggcggggctgcggttgcggtccctgcgcccgcggcggcggcggcggcggcagcggaggcgcaggcggtggcgagtgggtgagtgaagaggcggcgtcctggcgggtgtctgtttggcgtccggttgccgggaagagacgcgggtagcagccggggctctcctcagagctcgacacatttttactttccctctcgtttctctgaccgaagtcgggtgtccggctttcgcctctagcgactggtggaattgcctgcatctgggccccgggcttcgcggcggcgcagggacgagggatgggaatctggcctcttcctcgctttcccgcccgcagtgcgctgccccagctgtctccttcccggggacctgctgggagcgctgccgctacagactcgagagaaaggagcctcgggcactgagaggcctcgcccgggggaaggccggagggcgggcggcgggcggcgagcggctcctgcggaccaagtctgggttctctgggaacccgagacggtccctgatggcgaggagatcatgcggggtgctatgggggtgtggagacgtctgcagaattttagcccaagcttctaaggagtgctgatgacttgcatatgagggcagcaatgccagtcggtgtactccctattctgtgggacatgatgtggttgcttcacagctccgagatgacacagacttgcttaaaggaagtgaccattgtgacttgggcatcacttgactgatggtaatcagttgcagacagaagtgcacagattacatgtctgtgtccacactggatcagtctggccacgaggaacaccacaggctttgtattgagaaacaggagggaggtcctgcactttcccaggaggggtggccctttcagatgcaatcgagattgttaggctctggtagagtggttgcctggttgtggcagttggcaaattcctattcaaactgttgccgtgcgtcaccagttaacaacaagggtacacgatctgtctggcattacttctactttgtacaaaggatcaaaaatactgttagatatgatttttctcagactttgggaaacttttaacgtaatctgtgaatatcacagaagcaagactgtcatatagaggatattaataacctggagtcagaatacttgaaatatggtgtcatttgacacgggctctgttatcaccacctttgccaagccctttcacttgaggaaaaccctcaatcagttggaaactgcctcatgctgacagtacatctgaaacaaaaacgagagtagttaccacattccagattgttcactaaggcagcatttatctgctccaggaaaacattacaagcaacttatgaagttgataaaatattttgtttggctatgttggtactccaaaagttgctttcagagaaacaaagtaaaccaaggaggacttctgttgttcacgtctgcccttgggctctattctacgttaattaggtagttcccaggaggactagattagcctacctattgtctgagaaacttggatctgtgagaaatggccagatagtgatacgaacttcacctcccagtctttcctgatgtttaagattgagaaagtgttgtgaactttctggtgctgtaagcagttcactgtccttaaagtggtcctgggcagctcctgttgtggaaagtggaccgatttaggattctgcttggctttggactgggagaaaataaactgcatggttacaagtattgagagccaagttggagaaggtggcttacacctataatgccagagccttaggaggcaggggcaagaggatcactggaagtcaggagttcaagcccaacctgggcagcctagaccctgtctctacaaaaaattaaaaacttagccgggcgcggtggtgtgcacctgtagtcctagctacttgggaggctgaggcaggagggtcttttgagcccaggagtttgaagttacagggagctatgatcctgccagtgcactccagcctggatggcaaaacgagaccctgtctctaaaaaacaagaagtgagggctttatgatcgtagaaattttgcttacaatagcagtggaccaaccacctttctaaataccaatcagggaagacatagttgatttttaacaaacatttaaagaaaaagcaaaacctcaaacttagcactctactaacagttttagccgatgctaattaaggtaatcatgtctgcatatatgggattactttcagaaagtgtattgggaaacctctcatgaaccctgtgcaaccctgagcaagccaccgtctcactcagtttgaatcttggcttccctcaaaagactctgtggctaatgtttggtaactctctggagtagccagcactgcatgtacataggataggtacataaaacaattattggttttgagctgatttttttcagctgcatttgcgtgtatggatttttctcaccaaagacaatgacttcaagtgttaataaaataattgtacagctctcctaattatacttctctgtaacatttcatttctcagactatttcttttggtaggatttaaaactaaacaattcagtatgatctttgttcttcattttctttcttattcttttttttttcgagacagagtctccctctgttgtgccatctcagcccattgcaacctccgccacctgggttcaagtgattctcctgcctcagcctcctgagtagctgggattacaggtgcccgccaccacacctacctaattttttgtatttttagtagaggcggggtttcaccatgttggctaggctggtcttaaactcctgacctcagatgatccacctgcctcggcctcccaaagagctgggatgataggcgtgacccaccatgcccgccccattttttttcttattctgttaggagtgagagtgtaactagcagtctataatagttcaattttcacaacgtggtaaaaattttccctgtaattcaacgagattttgcttcagggctcagttctgttttaggaaatacttttattttcagtttgatgatgaaatattagagttgtgatattgcctttatgattacctacctttttaacctaaaagaatgaaagaaaaatatgtttacagtataattgtatggttgcgtgttaacttaattcattatgttggcctccagtttgctgttgttcgttatgacagcagtagtgtcattaccatttcaattcagattacattcctgtatttgatcattgtaaactgattgcttaaattgtattaaaaacagtggatattttaaacaagctgtactgcttatatccagtgctgtctcctaagactattaaattgatataacatatttaaaagtaaatatttcctaaatgaatttttgaaattaaaaatacacgtgttaaaactgtctttgtgttcaaccatttctgtacgtacttagagttaactgttttgccaggctctgtatgcctactcataatgtgataaaagcactcatctaatgctctataaatagaagtcagtgctttccatcagactgaacactcttggcaagatgtggataaaattatttaagtaaaattgtttactttgtcatacatttacagatcaaatgttagctcccaaagcaatcatatggcaaagataggcatatcataatttgcctattagctgctttgtattgctattatgatagatttcacagttttagatctgcttagatgaaaatgtaattctttttactgtcagtcttagatataagtcttcaattatagtacagtcacacattgcttaggaatgcatcattaggcgattttgtcattatgcaaacatcatagagtatacttacataaacctatatagtacagcctttacgtacgtaggccatatggtatagtctattgctcctaggctacaaatctgtacagctgttactgtactgaatactatagacagttgtaacacagtggtatttatttatctaaatatatccaaacatagaaaaggtacagttaaagtatggtataaaaaataatgatatacctatataggccacttaccgtgaatggagcttgcaggactagaagttgctctgggtgagtcagtaagtaagtggtgaatgaatgtgaaggcctagaacattactgtacacactgtagactttataaacacagtatgcttaagctacaccaaatttatctttacagtttttcttcaataaaaaattaatgtgaacctactataactttttaactttgtaaactttttaattttttaacttttaaaatacttagcttgaaacacaaacacgcatagctatacaaaaatattttttctttatatccttattctagaagctttttcctatttttaacttttttttttttacttgttagtcgtttttgttaaaaactaaaacacacacactttcacctaagcatagacaggattaggatcatcagtttcactcccttccacctcactgccttccacctccacatcttgtcccactggaacgtttttagggggaataacacacatgtagctgtcacctgctatgataacagtgctttctgttgaatacctcctgaaggacctgcctgaggctgttttacatttaacttaaaaaaaaaaataagtagaaggagtacactctaaaataacaataaaaggtatagtctagtgaatacataaaccagcaacatagtagtttattatcaagtgttgtatactgtaataattgtatgtgctatactttaaatgacttgaaaaattgtactaagaccttatgatggttacagtgtcactaaggcgatagcatattttcaggtccattgtaatctaatgggaccaccatcatatatgcagtccaccattgactgaaatgttacatggtacgtaactgtatttgcaagaatgatttgttttacattaatatcacataggatgtacctttttagagtgatatgtttatgtggattaagatgtacaagtggagcaaggggacaagagcccttggttctgtcttggatgtgagcttttatgctcttctcatcatgtctgttttcttattaaattcaaaggcttggacaggccctatttagcccttgttttctatgtgttctaaataactaaagcttttaaattctagccatttagtggagaactctctttgcaatggtaaaatgctgtattggtttcttgactagcatattaaatatatttatctttgtcttgatatttcaatgtcattttaaacatcaggattgggctttagtattctcatacccagagagttcactgaggatacaggactgtttgcccattttttgttatggctccagacttgtggtatttcgatgtcttttttttttttttttttttttaaccttttagcagctttaaagtatttctgttgttaggtgttgtattacttttctaagattactgtaacaaagcaccacaaactgagtggctttaaacaacagcaatttattctctcacaattctagaagctagaagtccgaaatggaagtgttgatggggcatgatcctcaaaagagagaagactctttccttgcctcttcctggcttctggtggttaccagcaatcctgagcgttcctttcttgcttcgtagtttcagcagtccagtatctgccttttgtcttcacatggatgtctaccccttgtctctgtgtctccagatctctctccttataaacacagaagttactggattaggccccactctaatccagtatgaccccattttaacacgattacacctatttctaaataaggtcacattcacatataccaagggttaggaattgagcatatcttttgcagggacacaattcaacccacaagtgtcagtctctagctgagcctttcccttcctggttttctcctttttagttgctgtgggttaggggccaaatctccagtcatactagacttgcacatggactggagatttgggaatactgcgggtctattctatgagctttagtatgtaacatttaatatcagtgtaaagaagccattttttcagttcactatttctttgaatttcttaatgtatgccctgaatataagtaacaagttactatgtctcataaaatgatcatatcaacaaacatttaatgtgcacctactgtgctagttgaatgtctttatcctgataggagataacaggcttccgcatctttgacttaagaggacaaaccaagtatgtctgaatcatttggggttttgatggatatctttaaattgctgaacctaatcattggttttatatgtcattgtttagatatctcaggagcatttggataatgtgacagttggaatgcagtgatgtcgactctttgcccaccgccatctccagctgttgccaagacagagattgctttaagtggtgaatcacctttattagcagctacttttgcttactgggacaatattcttggtcctagagtaaggcacatttgggctccaaagacagaacaggtacttctcagtgatggagaaataacttttcttgccaaccacactctaaatggagaaatccttcgaaatgcagagagtggtgctatagatgtaaagttttttgtcttgtctgaaaagggagtgattattgtttcattaatctttgatggaaactggaatggggatcgcagcacatacggactatcaattatacttccacagacagaacttagtttctacctcccacttcatagagtgtgtgttgatagattaacacatataatccggaaaggaagaatatggatgcataaggtaagtgatttttcagcttattaatcatgttaacctatcttttgaaagcttattttctgatacatataaatcttatttttaaattatatgcagtgaacatcaaacaatagatattatttattttgcatttatcctgttagatacaaatacatctggtctgatgcctgtcatcttcatattaactgtggaaggtaggaaatggtagctccacattacagatgaaaagctaaagcttaaacaaatgcagaaacttttagatcctggattcttcttgggagcctttgactctaataccttttgtttccctttcattgcacaatcctgtctttcgcttactactatgtgtaagtataacagttcaaaaaaatagtttcataagctgttggttatgtagcctttggtctctttaacctctttgccaagttcccaggttcataaaatgaggaggttgaaccgcatggttcccaagagaattccttttaattttacagaaattattgttttccccgaagtcctatagttcaatatataatgatatttacatttcagtatagttttggcatatctaaagaacacattaagttctccttcctgtgttccagtttgatactaacctggaagtccattaagcattaccaattttaaaaggcttttgcccaatagtaaggaaaaataatatcttttaaaagaataattttttactatgtttgcaggcttacttccttttttctcacattatgaaactcttaaaatcaggagaatcttttaaacatcataatgtttaatttgaaaagtgcaagtcattcttttcctttttgaaactatgcagatgttacattgactattttctgtgaagttatcttttttttccctgcagaataaagggtgttttgattttattttgtgttgtttataagaacatacattcgttgggttaatttcctgcccctgcccccgttttttccctaaagtagaaagtatttttcttgtgaactaaattactacacaagaacatgtctattgaaaaataagtatcaaaatgttgtgggttgtttttttaaataaattctttcttgctcaggaaagacaagaaaatgtccagaagattatcttagaaggcacagagagaatggaagatcaggtatatgcagattgcatactgtcaaatattattctcatggcatgtatctgtgtaaagttgatggctacatttgtgaaggccttggggacatacagagtaagccttaatggagcttttatggaggtgtacagaataaactagaggaagatttccatatcttagacctgaagagttaaatcagtaaacaaaggaaaatagtaattgcatctacaaattaatatttgctccctttttttttctgtttgaacagaataaattttggataacttgttactagtaaaaaatttaaaaattgtctgtgatatgttctttaaggtactacttctcgaactttttcctagaagtagctgtaacaggaggagagcatatgtacccctaaggtatctggggtataggcccatgtccaaacaatatttcttttaagtcttgtgttgtatctttaagactcatgcaatttacattttattccatgatataactattttaatattaaaatttgtcagtgatatttcttaccctctcctctaggaaaatgtgccatgtttatactttggctttgagtgcccctgaggaacagacactagagtttgagaagcatggttacacaggcgtggcttcccctgcagaaattaagtacagactatttcagtgtaaagcagagaagttcttttgaaggggaatctccagtgaagaaagggttcttcacttttacttccatttcctcttgagggtgaccctcattgctccttgtaaaactccgatattttaaacatggctgttttgctttcctctggttctttttaacatgagtgagacagatgatactttaaaaagtaattttaaaaaaaagtgttaaaatatatggccataatgcagaaccctatgctgtgatctcctttaccaaattgttgtgtttgtacttttgtagatagctttccagtccagagacagttattctgtgtaaaggtctgactcaacaagaaaagatttccctttacccaaagaatgccagtctttatttgctggtcaataagcagggtccccaggaaaggggtaactttcaccaccctctaacccactggttattagtaaactaattaagtagacttatctcaagatgaggaaacttaaaaccaagtaaaattctgcttttactgggattttattttttgaaaccagaaacgtttacttaagttgactactattaatgaattttggtctctcttttaagtactcttcttaaaaatgttatcctactgctgagaagttcaagtttgagaagtacaaggaggaatagaaacttgagagattttctttttcttttagagcctcttctgtatttagccctgtaggaattttttttttcccccaagattcttcttcgtgaaaaggaggagttgccttttgattgagttcttgcaaatctcacaacgactttattttgaacaatactgtttggggatgatgcatgagtctgaaacaacttcagttgtagctgtcatctgataaaattgcttcacagggaaggaaatttagcacggatctagtcattattcttgttagattgaatgtgttaatcataattgtaaacaggcatgataattattactttaaaaactgaaaacagtgaatagttagttgtggaggttactaaagcatgatttttttaaaataaaactttcagcattttgcaaatatgcatatggtttaggatagaacttccagaggtagcatcacatttaaattctcaagcaacttagtaatacgaggctctgaaaaactggttaaagttactccagaaatggccctgggtctgacagacattctaacttaaagatgcatatgaagactttgaataaaatcatttcatatgaagacattgaataaaatcatttcataaaataagtgaggaaaaacaactactattgaattcatcttaatgtatgattttaaaaatatgtttagctaaaaattcatagacatttgacaatttcgtttatatctcaaaaagttgacttacccaagttgatcacaaaactgatgagactggtggtggtagtgaataaatgagggaccacccatatttgagacactttacatttgtgatgtgttatactgaattttcagtttgattctataaactaccaatttcaaaattacaatttcaaggtgtaataagtagtggtattatcttgaaataggtctaaagggaacttttctgttttaaaatattcttaaactatatgtgctgattttgatttgcatttgggtagattatactcttatgaatcggggggctgggtattgattcaggttttccttacctatttggtaaggatttcaaagtctttttgtgcttgattttcctcgtttttaaatatgaaacatattgatgacttttaattaacaaatgtttttatctcgaataaattttaaaggagatcttttctaaaagaggtatgatgacttaattattgcatataacaataaatgagaaaccagtgattccatactctctaaagaataaaagtgagctttaggcccaggcatggtggctcatgcctgtaatcccagcactttggaaggccgaggcaggcggatcacctgaggtcaggaattcgacaccagcctggccaaatggcaaaaccctgtctctactacaaatacaaaaattagctgggcatggtggcagcccctatagtcccagctacttggaagactgagacaggagagtcactcgaacccgagaggcagaggttgcagtaagctgaaatcacaccattgcactccagcctgggcaacaagagcaaaactccgtctcaaaaaaaaaaaaaaaaaaaaaaaagaataaaagtgagctttggattgcgtataaatcctttagacaagtagtagacttgtttgatactgtgtttgaacaaattacaaagtattttcatcaaagaatgttattgtttgctgttatttttattttttattgcccagcttctctcatattcattatgtgattttcttcacttcatgttactttattgtgcagggtcagagtattattccaatgcttactggagaagtgattcctgtaatggaactgctttcatctatgaaatcacacagtgttcctgaagaaatagatgtaagtttttatatttttaaatgagagcaattataccctttatcagttttttggggttatattattattatgtatattattaatattctaattttaatactaagcacttcgtcgtacgtactatccacatgcagtattagccacttgaacagataagcacacacaaaatcctggattttatggcataacagaggcatttttgatcagtgatgacaaaactaaatttattttgtttatttcactacttttataattcctaaaagtgggaggatcccagctcttataggagcaattaatatttaatgcagtaccttttgaaacaaaactgtgtgccaaagcagtaaccattaatggaagttgacttatagtcacaaatttagtttccttaatcatttgttgaggatgttttgaatcacacactatgagtgttaagagatatctttaggacactattcttgttgttttattgtcatttaggttagtctcctgtctgacagctcagaagaggaagttgttcttgtaaaaattgtttacacaacctgattgaccagctttcacatttgttcttctgaaagctgatggtagtgcacagattgttttatggggagtcttgattctcagaaatgaaggcagtgtgttatattgaatccagacttcagaaaacttgtatattaaaagtgttttttcaacactatgttatagccagactaatttttttatttttttgatgcattttagatagctgatacagtactcaatgatgatgatattggtgacagttgtcatgaaggctttcttctcaagtaagaatttttcttttcataaaacctggatgaagcatatgttcacctatgacaagatttggaaggaagaaaataacagactgtctacttagattgttctagggacaacattgcatatttgaattgttgcttaaatttgtgttatttttcattcgttatatttctataatatatttgatgttattccatttgctatttaaagaaactgagtttccatatttcccagacaagaaatcatggccccttgcttgattctggtttcttgttttacttctcattaaagctaaaagaaccctttcaaattaagttgtactgtagatgaacttaagttatttaggcctagaaaaaaaaaattcatatttatactgatctttttccatccagcagtggagtttagtacttaagagtttgtgcccttaaaccagactccctgggttaatgctgtgtacctgtgggcaaggtccctgaattctctatacacctatttcctcatctgtaaaatggcaataataataatagtacctaatgtatagagttgttataagcattgagtaagataaataatataaagcacttagaacagtgcctggaacataagaacacttaataatagctaacattttctatttacatttcttctaaggaaaaggttaacagaaatagccaatatttgttcagtgcctacatgttagttcctatactaagtgctttacatgtattatcttatattctattttaatgtttcttcacagttgcagattatcatgaaattttattttttaaaaaagagaagtaaaaggataaagtattcacttttatgtccacagtcttttcctttaggctcatgatggagtatcagaggcatgaatgtgtttaacctaagagccttaatggcttgaatcagaagcactttagtcctgtatctgttcagtgtcagcctttcaaacatcattttaaatcccatttgactttaagtaaatcacttaatctctctacatgtcaatttcttcagctataaaatgatggtatttcaataaataaatacattaattaaatgatattttacaaactaattgggctgttttaaggctcaataagaaaatttctgtgaaaggtctctagcaaatgtagggttctatacaaataaaagataacattatgcttatatcttcggtgtttatcatgcaaagctcttctgagttttttgaagagctcacctactattttttgtttttagtttgttaaattgttttataggcaatgtttttaatctgttttctttaacttacagtgccatcagctcacacttgcaaacctgtggctgttccgttgtagtaggtagcagtgcagagaaagtaaataaggtagtttattttataatctagcaaatgatttgactctttaagactgatgatatatcatggattgtcatttaaatggtaggttgcaattaaaatgatctaatagtataaggaggcaatgtaatctcatcgaattgctgagacaacttgtggcaacagtgagtttgaaataaagtgaataggagtcatttatcagtttattttgataacttgtaaataccagtgtcagatgtgtataaatggttttgagaatatattaaaatcaggtatttaaaaaaacactattcttctatttcccaatgtaatctttaacaaatctgaaggtagtcatgtactttcggtactagttctgaagaaatgttatttgtttattcatcttgatttcattgtcttggctttccttctaaatctatcccttcttgggagctattgggattaagtggtcattgatgattatactttattcagtaatgtttctgaccctttccttcagtgctacttgagttaataaaggattaatgaacagttacatttccaagcattagctaataaactaaaggattttgcacttttcttcactgaccattagttaaaaacagttcagagataagtacatgtatctttcaattctagcaaacctaattttttaaaagaagttttacataggaaatatgttggaaatgattatttactttacaaagatattcataatttattttttctgtaactagctactttgtatatttacatgagccttaatttatcaaaattatatttctcatataaccatttatgagagcttagtattcctctgtcattatattgcgtctacggactagtgatcttactacttctgttacctcgaacaagtggcttcccgtctgtgacctccaaagccgtaggttccacagagtgactgctgagctgctttatgaagggagaaaggctccatagttgggtttttggttttgcttttgtttttgtttttaacatttttcctatcctccatcctcttgaggcagagtagcttaccttttatcttgttttaatttgagaaagaagttgccactgctctagattgaaaaccactgctttaacataataactctgaatatggtttgaatttcaagatagtgacatgcctttttatttttactaatagagctgtaggtcgaatattattagatttctaaaccccacccaatgacctccttattttaaatcaaatttaataattaattatcttcttattggaggatctggacattctttgatgtttcttacaatgaatttcacatgtagacccactaaacagaagttataaaggttccatggtcaaataagtctgagaaagtctgcatattatataattcacctaaagagtcacagtatgtacccaaatgttaaaggttttgagatgccatacagtaaatttaccaagcattttctaaatttatttgaccacagaatccctattttaagcaacaactgttatatcccataggttccaggtgactaaagaatacttattgcttaggatatgttttattgataataacaattaaaatgtcagatatctttcataagcagatcagtggtctttttaaaactttgtattttaatgctaaaatcttttcttttgtagatagtcagaacattatgcctttttctgactgcagcagagagaaaatgctccaggttatgtgaagcagaatcatcatttaaatatgagtcagggctctttgtacagggcctgctaaaggtatagtttctacttatcacaagggaaaccaattttctaaaatcatttttgagactctttgtagacaaatattaaatattagcatttaatgtatctcatattgacatgcccagtgactgacttcctttgcacagttctgcgcatagactatatgtcttatggatttatagttagtatcatcagtgtaacaccatagaataccctttgttttccaggtgggtccctgtacctacatgtctagcatcaggtgttgttttttttttttttttttaaaacatatgcttaaatcaggttgcacatctaaaataagatcatttctttttaactaaatagatttgaattttattgaaaaaaattttaaaacatctttaagaagcatataggatttaagcagttactatgtatgtgtactaaaatatatatatattcctaaatatatattcctatatataatatatgtatttctatatataatatatattagaaaaaacttagagttttctttcatttgagtctactgttcaaggagcaaaacagagaaatgtaaattagcaattatttacaataattaaagggaagaaagttgttcaccttgttggatctattattgttgttttaattatagtcccaagacgtgaagaaatagctttcctaatggttatgtgattgtctcatagtgactactttcttgaggatgtagccacagcaaaatgaaatttaaaaaatttaaaaattgttgcaaataaaagttatattaggcttttgtgcaatttcaataatgtgctgctatgaactcagaatgatagtatttaaatatagaaactagttaaaggaaacacagtttctatttgagttatacaaatctgtaaattagaacttctcctgttaaggcattataaagtgcttaatacttttgtttcctcagcaccctctcatttaattatataattttagctctgaaagggacctataccagatgtgtagaggaaatttcaaaactatgatctaatgaaaaaatatttaatagttctccatgcaaatacaaattatatagttttctggaaaatacctttgacattatacaaagatgattatcacagcattataatagtgaaaaaatggaaatagcctctttcttctgttctgttcacagcatatggcacagtacctcatatgcagtaggttattatgacctggtaactggctcccccaactgattaggaaagaagtaaatttgttatttataaaaatacgtgttcattgagatgcatagaataattaagaaattaaaagacacttgtaatttcaaatccagtgaatacccactgttaatatttggcatatctctttctagtctttttttcccttttgcatgtattttctttaagactcccacccccactggatcatctctgcatattctaatctgcttttttcacagcagattctaagcctttttgcatatcaacacaaacttcaacaacttcatctttagatgctaaataatgaattcatttttatttacttaaccactttctttggatgctcaggttattctgatgttttgccattaaaaccaatgctatactgaacacttctgtcactaaaacttgaacacactcatgaataatttcttaggataaatttttagagatggatttgctaaatcaaagaccattttttaaaaattgaaaaacaattatatcgtttggcatgtaagacagtacattttccttttattttgacaggattcaactggaagctttgtgctgcctttccggcaagtcatgtatgctccatatcccaccacacacatagatgtggatgtcaatactgtgaagcagatgccaccctgtcatgaacatatttataatcagcgtagatacatgagatccgagctgacagccttctggagagccacttcagaagaagacatggctcaggatacgatcatctacactgacgaaagctttactcctgatttgtacgtaatgctctgcgtgctggtactgtagtcaagcaatatgaaactgtgtcttttatgaataaaaacaaaacagaagttgcattcaaaaagaaagaaatattactagcagaattatgcttgaagaaacatttaatcaagcatttttttcttaaatgttcttctttttccatacgattgtgtttaccctaaaataagtaagattaacccttaaagtgaatatttaactatttgtttaataaatatatattgagctcctaagcactgttctaggtactgggcttaatagtggctaaccacacagctccagcccctacattgcatatagtctattgtataagttactgaatggacttactaacaaaaccagagaagtaattctaagtcttttttttcttgacatatgaatataaaatacaacaaaactggtaaaatatattaatagagcattcttttactttgcattttatattgttactcacttcgtatttaagaaaaacagtctgatcaggaaattcaaaaggaaaagtaatgataattaattgagcatagacccaacttgaaaagaaaaaaaaggatgatgataaatctataatcctaaaaccctaagtaaacacttaaatgatgttctgaaatcaggaaaagaattatagtatatttttgtggttctcttttattagttgaaaaaaggcacagtagctcatgcctataagaacagagctttgggattccaaggcaggcagatcacttgaggccaggagttccagaccagcctgggcaacatagtgaaaccccatctctacaaaaataaaaaagaattagttgaatgtgtttctgtgtgcctataatcctagctattcagaaagctgaggcaggaggatctcttgagcccaggagtttgaggttacatggagttatgatgtgccagtgtactccagcctgcgggacaatgagactctgtcttgttaaaaaaaaaagtgcttggaataatgtttggcatatagaaggtaacaacagtaaatgttaactgtaataacccaggtataagtgtgtaaggtgatagaaaaattggggcaaacaaccctgacctgtgtctctacagaataagtttgagttgaggcaacagacatgtggagcaccagtaattacacactaaatgttaaccaaaagcgttgaatagtaacatcttattcaagggacccccagccttatatatctcaaggtgcagaaagatgacttaatataggacccattttttccgagttctccagagtttttattggttcttgagaaagtagtgggggaattgttttagaaaatgaattggtcaaactgaaattccatgtcagtaagtttttacatattggtaaattttgatagacatgtagaagttttctaattaatctgcgccttgaaacattttcctttttcctaaagtgcttagtattttttcccttttttgattggttgcttgggagcttttttgaggaaatttagtgaactgcagaatgagtttgcaaccatttagtatttttgttttgtgttttagaggaggtatgtgtattttaacatttcttaatcatttttagccagctatgtttgttttgctgattgacaaactataattaaacagctattctcattttgctgatcatgacaaagtaatatcctgaatttttaaattttgcatccagctctaaattttctaaattttctaaacataaaattgttcaaaaaatagtatttttagccactagattgtgtgttgttaagtctgttgtcacagactcattttacttttcagtgtgtgtttttacatgttaattatgtttgtcatttttaattttaactttttaaaataattccagtcactgccaaaacatgaaaaattggtcactggaaattttttttttaacttttattttaggttcatgtgtacatgtgcaggtttgttatacaggtaaattgcgtgtcgtgagggtttggtgtacccaggtaataagggtagtacccaataggtagttttttgatccttacccttctcccacccttctttcaccctcgagtaggccttggtgttgctgtttccttctttgtgtccatgtgtactcaatggttagctcctacttagaagtgagaacatgcggtatttggttttctgttcctggattagttcactcaggataatggcctctagctccatctgttttttatggctgcatagtattccatggtgtatatgtatcatgttttctttatccagtctaccattgatagacatttaggttgattctctgtctttactatcatgaatagcgctgtgatgaacatatacacatgcatgtgtccttatggtggaacaatttgtattcctttaagtatatacagaataatggggttgctagggtgaatggtagttctattgtaagttatttgtgaaatcttcaaactgcttttcacaatagctaaactaatttacagtcccaccagcagtgtataagtgttcccttttctccacaaccttgccaacatgttatttttttacttttcaataataggcattcctagagaattgatttgcaattctctaatgattagtgatattgagcattttttcgtatgctttttagctgtgtgtatatattcttttgaaaaatgttaatgtcctttgcccagtttgtaatggggttgtttgtttttgcttgttaattaaagttccttccagattctggatatccctttgtcagatgcgtggtttgcagatatttttctccccttgtgtaggttgtctttttactctgttgatagtttcttttgccgggcaggagctcattaggtctcatttgtgtttgtttttgttgcagttgcttttggcgtcttcatcataaaatctgtgccagggcctatgtccagaatggtatttcctagtttgtcttccagggtttttacaattttagattttacgtttatgtctttaatccgtcttgagttgattaaggaaggggtccagtttcactctaattcctatggctaacaattatcccagcaccatttattgaatacggagtcctttccccattgcttgtttttgtcaattttgttgaagatctgatggttgtaggtgctatgtggctttatttcttggctctctattctccactggtctgtctgtttttataccagtaccctgctgttaaggttcctatagccttttagtataaggtcggctaatgtgatgcctccagctttgttctttttgcttaggattgctttggctatttgggctcctttttggttccatattaattttaaaatagttttttctagttttgtgaagaatgtcattgatagtttagaggaatagcgttgaatctgtagattgctttgggcaaatggccattttaacaatattgattcttcctatctatgaacatggaatgtttttccatgtgtttgtgtcatctctttatacctgatgtataaagaaaaaccagtattattgctactcaatctgttccaaaaaattgaggaggaggaactcttccctaatgagaccggcttccttctgataccaaaacctggcagagatacaacagaaaaaagaaaacttcaggccaatatccttgatgaatatagatgcaaaaatcctcaacaaaatactagcaaccaaatccagcagtacgtcaaaaagctaatctactttaagtaggctttatccctgggatgcaaggttggttcaacatacacaaatcaataagtgtgattcatcacataaacagagctaaaaacaaaaaccacaagattatctcaataggtgcagaaaaggctttcaatacaatttaacatccttcatgttaaaaaccttcagtaggtcaggtgcagtgactcacacctgtaatcccagcactttgggaggccaaggcggacgtatatcttaagcccaggagttcaagaccagcctaggcagcatggtgaaaccccatctctacaggaaaaaaaaaaaaaaaaaaaaaaaaaaaaaaaaagcttaatatggcggcatgcacctatagtcccagctactcaggaggttgaggtgggaggattgcttgagcccaggaggcagaggttgcagcgagctgagatcgtgccactgcactccaacctgggcaataaagtgagaccctgtctcaaaaagaaaaacaaaaataatcctaaaccaactaggcattgaaggaatatgcctcaaaaaaataagaaccatctatgacagacccacagccaatatcttaccaaatgggcaaaagctggaagtattctccttgagaaccgtaacaagacaaggatacacactctcatccctccttttcagcatagttctggaagtcctcgccagagcagtcaggaaagagaaagaaagaaaaggcattcagataggaagagaagaagtcaaactatttctgtttgcaggcagtataattctatacctagaaaatgccatagtttctgcccagaagctcctacatctgttaaaaatttcagcaaagttttagcattgtctgtattccaacagcttccagggtgagagtgaaatcaggaacacagtcccgttcacaatagccgcaaaaagaataaaataccttggaatccagctaaccagggaggtgaaacatctctacgagaattacaaaacgctgctgaaagaaatcagagatgacacaaacaaatggaaatgttgtttttaacaccttgctttatctaattcacttataactaagatattcattcagtggaacaggtataataagaccactcgacttaaatataagccttattctctttccagagcccaagaaggggcactatcagtgcccagtcaataatgataaaatgctgatatttttcccctttactgtttctttcttctgtagtgtggtacactcatttcttaagattagaaaacttgacctaccttcctgtttgcttctacacacccccattctctttttttgccactccggtcaggtataggatgatccctaccacttttagttaaaacctccttcccttattaaatgttctcttaccactctggcctgagtagaacctagggaaaatggaagagaaaagatgaaagggaggtgggggctgggaagggaatagtcttgtttgtgtgtttgctttagcacctactatatcctaggtgctgtgttaggcacacattattttaagtggccattatattgctacatctcactctggtcattgccaaggtaggtagtactttcttggatagttggttcatgttacttataggtggtggacttgttgaggcaaccccaatggataatcatctgagtgtgttctctaatctcagatttttcttcatattttttggtttgttttggtttttgatggtggtggttgtgtgcttatttttgttgctggcttgtttttttgttttgtttttgatatggcaagaattggtagttttatttattaattgcctaagggtctctactttttttaaaagatgagagtactaaaatagattgataggtacatacatacctttatgggggactgcttatattccttagagaaaaaaattacttattagcctgacaaacaccagtaaaatgtaaatatatccgtgagtaaataaatgaatgtatgctttgtatctccaaatatatacatctatattcttacaaatatgtttttatgtaataccaatttataagaacttaaaatgttggctcaagtgagggatggtggaaagtagcattatatagccatttcaacatttgaacttttttcttcattttcttcttttcttcaggaatatttttcaagatgtcttacacagagacactctagtgaaagccttcctggatcaggtaaatgttgaacttgagattgtcagagtgaatgatatgacatgttttcttttttaatatatcttacaatgcctgttctctctctctatatatatatatttatatatttccctggatcatgccccagagttctgctgagcaattgcagttaagttagttacactacagttctcacaagagtctgtgaggggatgtcaggtgcatcattacattggatgcctcttgtcctagatttatgtttcgggaattcagacctatgtttacaatataataaatattgttgctgccttttacagataaaataataagatataaacttgaccacaactactgttttttgaaacatagagttcatggtttacatgtatcaaagtgaaatctgagttagcttttacagatataatatatacatatatatatcctacaatgcttgtactatatatgtagtacaagtatatatatgtgtgtgtgtgtgtgtatatatattatggcactgtagtatatatatgtttatatgttaaaaaatatataaatatatgttacatatttaacataaacatatatacatatatgttaaatatataacatatactctatatatgacaaatagagtataatatatatttttattttttatatatatataaaacatgatagaattaagaattaagtcctaatctgttttattaggtgctttttgtagtgttcagtctttctaaagtgtctaaatgatttttccttttgacttattaatggggaagagcctctatattaacaattaaggctgcagcattgattacttcaaacaacaaacattttaattcaagcattaacctataactcaagtaagtttttttttttttttttttgagaaagggaggttgtttatttgcctgaattgagtcaaaaatatttttgaaacatcatgtactcatttaaatgataacatctttattgtttcattcttttaaaaaatatctacttaattacacagttgaaggaaattgtagattatatggaacttatttcttaatatattacagttttgttataataacattctggggatcaggccaggaaactgtgtcatagataaagctttgaaataatgagatccttatgtttactagaaattttggattgagatctatgtggtctgtgacatattgcaaagttcaaggaaaattcgtaggcatggaatttctcaaactgaaaatccctcccactgtccacctcatcacatgcacacattctactcttacccacccactccaccccttgcaaaagtacagatatatgaatgtctcaaaaccatgggctcatcttctagaagcttcaatgttatttgaagatttgggcagaggaagttaagaaatatgaaatagcttacatatgagttttaatagtgaaacaaacatggatgtattctgaagtagaatgcaaaatttgagtgcatttttttttttttgagactgagtctggctctgtcgcccaggctggagtgcagtggccggatctcagctcactgcaagctccacctcccgggtttacgccattctcctgcctcagcctcccgagtagctgggaccacaggcgcccgccacttcgcccggctagtttgtttgtattttttagtagagatggggtttcaccgtgttagccagggannnnnnnnnnnnnnnnnnnnnnnnnnnnnnnnnnnnnnnnnnnccattgagtgcatttttaaagataaatcagaaaacttcgaaaaactatcagattggccggacatggtggcttatgcctgtaatcctagcactttgggaggctgaggtgggtggatcacgaggtcaggagatcgagaccatcctgccaacatggtgaaaccccatctctactaagtatacaaaaattagctgggcgtgacagcacgtgcctgtaatcccagctacttgggaggctgaggcaggagaatcgcttgaacccgggaggtggaggttgcagtgagtcaagatcacaccactgcacttcagcttggtgacagagctagactccatatcaaaaaaaaaaaaaaaaaaaagaagtcagattgttcctacacccagtgcttctataccacactcctactagggggcatcagtggaaatggttaaggagatgtttagtgtgtattgtctgccaagcactgttaacactgtcctagaaacattgctgtacaagtagaatgtgagcaaattatgtattgaaatggttcctctccctgcaggtctttcagctgaaacctggcttatctctcaggagtactttccttgcacagtttttacttgtccttcacagaaaagccttgacactaataaaatatatagaagatgatacgtgagtacaactcctacatggaggaaaaaccttttgtacgttgttttttgttttatttcctttgtacattttctgtatcataatttttgctttttttttttttttttttttctccattactttcaggcagaagggaaaaaagccctttaaatctcttcggaacctgaagatagaccttgatttaacagcagagggcgatcttaacataataatggctctggctgagaaaattaaaccaggcctacactcttttatctttggaagacctttctacactagtgtacaagaacgagatgttctaatgactttttaaatgtgtaacttaataagcctattccatcacaatcgtgatcgctgctaaagtagctcggtggtgtggggaaacattcccctggatcatactccagagctctgctcggcagttgcagttaagttagttacactacagttctcacaagagtctgtgaggggatgtcaggtgcatcattacattggatgtctcttttcctagatttatgcttttgggatacagacctatgtttacaatataataggtattattgctgtcttttaaatatataataataggatataaacttgaccacaactgctgtttttttgaaatatatgattcatggtttacatgtattaaggtgaaatccgagttcgcttttacagatattagttgactttctatcttttggcattctttggtgtgtggaattactgtaatacttctgcaatcaactgaaaattagagcctttaaatgatttcagttccacagaaagaaagtgagcttcaacataggataagctttagaaagagaattgatcaagcagatgtttaattggaattgattattagatcctgctttgtggatttagccctcgggattcagtctgtagaaatgtctgatagttctctatagtccctgctcatggtgaaccacagttaggatgttttgtttgttttattgttgttgctattgttgatgttctatatagttgagctctataaaaggaaattgtattttatgttttagtagttgttgccaactttttaaattaattttcattatttttgagccaaattgaaatgtgcacctcctgtgccttttttttccttggaaaatcgaattacttggaagaagttcagatttcactggtcagtcgttttcatcttgttttcttcttgcagagtcttaccatgtacctgctttggcaatcattgtaactctgagattataaaatgcattagagaatatattaactaataagatcttttttttcaggaacagaaaatagttccttgagtacttccttcttacatttctgcccatgtttttgaagttgttgccatttgcctgcaataggctataaggaatagcaggagaaattttactgaagtgctatttttctaggtgctactttggcagagctaagtggtctgtttcttttgtttccttaatgcgtttggaccattttgctggctgtaaaataactgattaatataattctaacacaatattgacattgtagtgtacacaaacacaaatattttatttaaaactggaagtaacataaaagggaaaatatatttataagaaaggaataaaggtaatagagctcttctgtcccccagccaccaaatttacacaacaaaatcatatgttctaatgtgaaaggtcataatagctttcccatcattaatcagaaagatgtggcagcttgattttttagacaacccctgaactagatgactgttgtactgtagctcagtcatttaaaaaatatataaatactatctcgtagtgtcccatactatgttttttacatgatagattcttatttaagtgctaactggttattttctttggctggtttattgtactgttatatagaatgtaagttgtacagtgaaataagttattaaagcatgtgtaaacattgttatatatcttttctcctagatggagaattttgaataaaatatnnnnnnnnnnnnnnnnnnnnnnnnnnnnnnnnnnnnnnnnnnnnnnnnnnnnnnnnnnnnnnnnnnnnnnnnnnnnnnnnnnnnnnnnnnnnnnnnnnnnnnnnnnnnnnnnnnnnnnnnnnnnnnnnnnnnnnnnnnnnnnnnnnnnnnnnnnnnnnnnnnnnnnnnnnnnnnnnnnnnnnnnnnnnnnnnnnnnnnnnnnnnnnnnnnnnnnnnnnnnnnnnnnnnnnnnnnnnnnnnnnnnnnnnnnnnnnnnnnnnnnnnnnnnnnnnnnnnnnnnnnnnnnnnnnnnnnnnnnnnnnnnnnnnnnnnnnnnnnnnnnnnnnnnnnnnnnnnnnnnnnnnnnnnnnnnnnnnnnnnnnnnnnnnnnnnnnnnnnnnnnnnnnnnnnagaagactaattgatcatatcactatgattctcaaagaagaaccaaaacttcatataatactacaaatatgagatagttacttctgtagtatatttctgtaatgctacaggttaaacaggtcactcttatataacactattttgattttgatgtagaattgcacaaattgatatttcttctatgatctgtagggtatagcttaaagtagcaaaaacagtccaccacctccagttaacacacagtaacactatgggactagtattattatttccattttacaaaggaggaaactaaagcttaaagatgtgtaatatacagcccaaggtcacacagctggtaaaggtagatttcatcccagacagttacagtcattgccgtgggcacagctcctaacttattaactccatgtaactggtactcagtttagttgaattgaaaggagagtagggaagcaggtctgtttgcactattcagagcccaagtgtgaatccctgctgtgctgcttggagaagttacttaacctatgcaaggttcattttttaaatatttgaaacggaatgataatacatacttcaccagtgggtttaatgagaccttataagatcgttagttcagtacctgaccagtgcttcataaatgctttttcatccaatctgacaatctctagcttgtaattggggcatttagaacatttaatatgattattggcatggtaggttaaagttgtcatcttgctgttttctctttgttcttttttctcctttcttttggatttttttttaattttactgtgtcttctctgttgtcttattaa

SEQ ID NO: 20 - DNA, 20 bp, synthetic construct
  source 1..20: mol_type = other DNA
gccttactctaggaccaaga

SEQ ID NO: 21 - DNA, 20 bp, synthetic construct
  source 1..20: mol_type = other DNA
ctttcctagcgggacaccgt

SEQ ID NO: 22 - DNA, 20 bp, synthetic construct
  source 1..20: mol_type = other DNA
aaaagagaagcaaccgggca

SEQ ID NO: 23 - DNA, 20 bp, synthetic construct
  source 1..20: mol_type = other DNA
caaaagagaagcaaccgggc

SEQ ID NO: 24 - DNA, 20 bp, synthetic construct
  source 1..20: mol_type = other DNA
ccaaaagagaagcaaccggg

SEQ ID NO: 25 - DNA, 20 bp, synthetic construct
  source 1..20: mol_type = other DNA
cccaaaagagaagcaaccgg

SEQ ID NO: 26 - DNA, 20 bp, synthetic construct
  source 1..20: mol_type = other DNA
tctttcctagcgggacaccg

SEQ ID NO: 27 - DNA, 20 bp, synthetic construct
  source 1..20: mol_type = other DNA
ctctttcctagcgggacacc

SEQ ID NO: 28 - DNA, 20 bp, synthetic construct
  source 1..20: mol_type = other DNA
tctctttcctagcgggacac

SEQ ID NO: 29 - DNA, 20 bp, synthetic construct
  source 1..20: mol_type = other DNA
ctctctttcctagcgggaca

SEQ ID NO: 30 - DNA, 20 bp, synthetic construct
  source 1..20: mol_type = other DNA
cctctctttcctagcgggac

SEQ ID NO: 31 - DNA, 20 bp, synthetic construct
  source 1..20: mol_type = other DNA
acctctctttcctagcggga

SEQ ID NO: 32 - DNA, 20 bp, synthetic construct
  source 1..20: mol_type = other DNA
atccaaatgctccggagata

SEQ ID NO: 33 - DNA, 20 bp, synthetic construct
  source 1..20: mol_type = other DNA
cacctctctttcctagcggg

SEQ ID NO: 34 - DNA, 20 bp, synthetic construct
  source 1..20: mol_type = other DNA
gcacctctctttcctagcgg

SEQ ID NO: 35 - DNA, 20 bp, synthetic construct
  source 1..20: mol_type = other DNA
cgcacctctctttcctagcg

SEQ ID NO: 36 - DNA, 20 bp, synthetic construct
  source 1..20: mol_type = other DNA
gcgggacaccgtaggttacg

SEQ ID NO: 37 - DNA, 20 bp, synthetic construct
  source 1..20: mol_type = other DNA
acgcacctctctttcctagc

SEQ ID NO: 38 - DNA, 20 bp, synthetic construct
  source 1..20: mol_type = other DNA
gacgcacctctctttcctag

SEQ ID NO: 39 - DNA, 20 bp, synthetic construct
  source 1..20: mol_type = other DNA
tgacgcacctctctttccta

SEQ ID NO: 40 - DNA, 20 bp, synthetic construct
  source 1..20: mol_type = other DNA
ttgacgcacctctctttcct

SEQ ID NO: 41 - DNA, 20 bp, synthetic construct
  source 1..20: mol_type = other DNA
tttgacgcacctctctttcc

SEQ ID NO: 42 - DNA, 20 bp, synthetic construct
  source 1..20: mol_type = other DNA
gtttgacgcacctctctttc

SEQ ID NO: 43 - DNA, 20 bp, synthetic construct
  source 1..20: mol_type = other DNA
tgtttgacgcacctctcttt

SEQ ID NO: 44 - DNA, 20 bp, synthetic construct
  source 1..20: mol_type = other DNA
ctgtttgacgcacctctctt

SEQ ID NO: 45 - DNA, 20 bp, synthetic construct
  source 1..20: mol_type = other DNA
gctgtttgacgcacctctct

SEQ ID NO: 46 - DNA, 20 bp, synthetic construct
  source 1..20: mol_type = other DNA
cgctgtttgacgcacctctc

SEQ ID NO: 47 - DNA, 20 bp, synthetic construct
  source 1..20: mol_type = other DNA
agcgggacaccgtaggttac

SEQ ID NO: 48 - DNA, 20 bp, synthetic construct
  source 1..20: mol_type = other DNA
tcgctgtttgacgcacctct

SEQ ID NO: 49 - DNA, 20 bp, synthetic construct
  source 1..20: mol_type = other DNA
gtcgctgtttgacgcacctc

SEQ ID NO: 50 - DNA, 20 bp, synthetic construct
  source 1..20: mol_type = other DNA
tgtcgctgtttgacgcacct

SEQ ID NO: 51 - DNA, 20 bp, synthetic construct
  source 1..20: mol_type = other DNA
tggagcccaaatgtgcctta

SEQ ID NO: 52 - DNA, 20 bp, synthetic construct
  source 1..20: mol_type = other DNA
ttgtcgctgtttgacgcacc

SEQ ID NO: 53 - DNA, 20 bp, synthetic construct
  source 1..20: mol_type = other DNA
tctgtctttggagcccaaat

SEQ ID NO: 54 - DNA, 20 bp, synthetic construct
  source 1..20: mol_type = other DNA
cttgtcgctgtttgacgcac

SEQ ID NO: 55 - DNA, 20 bp, synthetic construct
  source 1..20: mol_type = other DNA
acttgtcgctgtttgacgca

SEQ ID NO: 56 - DNA, 20 bp, synthetic construct
  source 1..20: mol_type = other DNA
aacttgtcgctgtttgacgc

SEQ ID NO: 57 - DNA, 20 bp, synthetic construct
  source 1..20: mol_type = other DNA
gaacttgtcgctgtttgacg

SEQ ID NO: 58 - DNA, 20 bp, synthetic construct
  source 1..20: mol_type = other DNA
ggaacttgtcgctgtttgac

SEQ ID NO: 59 - DNA, 20 bp, synthetic construct
  source 1..20: mol_type = other DNA
cggaacttgtcgctgtttga

SEQ ID NO: 60 - DNA, 20 bp, synthetic construct
  source 1..20: mol_type = other DNA
tagcgggacaccgtaggtta

SEQ ID NO: 61 - DNA, 20 bp, synthetic construct
  source 1..20: mol_type = other DNA
gcggaacttgtcgctgtttg

SEQ ID NO: 62 - DNA, 20 bp, synthetic construct
  source 1..20: mol_type = other DNA
ggcggaacttgtcgctgttt

SEQ ID NO: 63 - DNA, 20 bp, synthetic construct
  source 1..20: mol_type = other DNA
gggcggaacttgtcgctgtt

SEQ ID NO: 64 - DNA, 20 bp, synthetic construct
  source 1..20: mol_type = other DNA
tgggcggaacttgtcgctgt

SEQ ID NO: 65 - DNA, 20 bp, synthetic construct
  source 1..20: mol_type = other DNA
gtgggcggaacttgtcgctg

SEQ ID NO: 66 - DNA, 20 bp, synthetic construct
  source 1..20: mol_type = other DNA
cgtgggcggaacttgtcgct

SEQ ID NO: 67 - DNA, 20 bp, synthetic construct
  source 1..20: mol_type = other DNA
ctagcgggacaccgtaggtt

SEQ ID NO: 68 - DNA, 20 bp, synthetic construct
  source 1..20: mol_type = other DNA
cctagcgggacaccgtaggt

SEQ ID NO: 69 - DNA, 20 bp, synthetic construct
  source 1..20: mol_type = other DNA
tcctagcgggacaccgtagg

SEQ ID NO: 70 - DNA, 20 bp, synthetic construct
  source 1..20: mol_type = other DNA
gacggctgacacaccaagcg

SEQ ID NO: 71 - DNA, 20 bp, synthetic construct
  source 1..20: mol_type = other DNA
ggacggctgacacaccaagc

SEQ ID NO: 72 - DNA, 20 bp, synthetic construct
  source 1..20: mol_type = other DNA
gggacggctgacacaccaag

SEQ ID NO: 73 - DNA, 20 bp, synthetic construct
  source 1..20: mol_type = other DNA
agggacggctgacacaccaa

SEQ ID NO: 74 - DNA, 20 bp, synthetic construct
  source 1..20: mol_type = other DNA
cagggacggctgacacacca

SEQ ID NO: 75 - DNA, 20 bp, synthetic construct
  source 1..20: mol_type = other DNA
ttcctagcgggacaccgtag

SEQ ID NO: 76 - DNA, 20 bp, synthetic construct
  source 1..20: mol_type = other DNA
gcagggacggctgacacacc

SEQ ID NO: 77 - DNA, 20 bp, synthetic construct
  source 1..20: mol_type = other DNA
agcagggacggctgacacac

SEQ ID NO: 78 - DNA, 20 bp, synthetic construct
  source 1..20: mol_type = other DNA
cagcagggacggctgacaca

SEQ ID NO: 79 - DNA, 20 bp, synthetic construct
  source 1..20: mol_type = other DNA
gcagcagggacggctgacac

SEQ ID NO: 80 - DNA, 20 bp, synthetic construct
  source 1..20: mol_type = other DNA
ggcagcagggacggctgaca

SEQ ID NO: 81 - DNA, 20 bp, synthetic construct
  source 1..20: mol_type = other DNA
tttcctagcgggacaccgta

SEQ ID NO: 82 - DNA, 20 bp, synthetic construct
  source 1..20: mol_type = other DNA
agaagcaaccgggcagcagg

SEQ ID NO: 83 - DNA, 20 bp, synthetic construct
  source 1..20: mol_type = other DNA
gagaagcaaccgggcagcag

SEQ ID NO: 84 - DNA, 20 bp, synthetic construct
  source 1..20: mol_type = other DNA
agagaagcaaccgggcagca

SEQ ID NO: 85 - DNA, 20 bp, synthetic construct
  source 1..20: mol_type = other DNA
aagagaagcaaccgggcagc

SEQ ID NO: 86 - DNA, 20 bp, synthetic construct
  source 1..20: mol_type = other DNA
aaagagaagcaaccgggcag

SEQ ID NO: 87 - DNA, 20 bp, synthetic construct
  source 1..20: mol_type = other DNA
gttttctatgtgcgatgacg

SEQ ID NO: 88 - DNA, 20 bp, synthetic construct
  source 1..20: mol_type = other DNA
tgttttctatgtgcgatgac

SEQ ID NO: 89 - DNA, 20 bp, synthetic construct
  source 1..20: mol_type = other DNA
ctgttttctatgtgcgatga

SEQ ID NO: 90 - DNA, 20 bp, synthetic construct
  source 1..20: mol_type = other DNA
tctgttttctatgtgcgatg

SEQ ID NO: 91 - DNA, 20 bp, synthetic construct
  source 1..20: mol_type = other DNA
gtctgttttctatgtgcgat

SEQ ID NO: 92 - DNA, 20 bp, synthetic construct
  source 1..20: mol_type = other DNA
tgtctgttttctatgtgcga

SEQ ID NO: 93 - DNA, 20 bp, synthetic construct
  source 1..20: mol_type = other DNA
ctgtctgttttctatgtgcg

SEQ ID NO: 94 - DNA, 20 bp, synthetic construct
  source 1..20: mol_type = other DNA
tctgtctgttttctatgtgc

SEQ ID NO: 95 - DNA, 20 bp, synthetic construct
  source 1..20: mol_type = other DNA
gtctgtctgttttctatgtg

SEQ ID NO: 96 - DNA, 20 bp, synthetic construct
  source 1..20: mol_type = other DNA
cgtctgtctgttttctatgt

SEQ ID NO: 97 - DNA, 20 bp, synthetic construct
  source 1..20: mol_type = other DNA
tacaggctgcggttgtttcc

SEQ ID NO: 98 - DNA, 20 bp, synthetic construct
  source 1..20: mol_type = other DNA
cccggcccctagcgcgcgac

SEQ ID NO: 99 - DNA, 20 bp, synthetic construct
  source 1..20: mol_type = other DNA
ccccaaaagagaagcaaccg

SEQ ID NO: 100 - DNA, 20 bp, synthetic construct
  source 1..20: mol_type = other DNA
cccccaaaagagaagcaacc

SEQ ID NO: 101 - DNA, 20 bp, synthetic construct
  source 1..20: mol_type = other DNA
gcccccaaaagagaagcaac

SEQ ID NO: 102 - DNA, 20 bp, synthetic construct
  source 1..20: mol_type = other DNA
cgcccccaaaagagaagcaa

SEQ ID NO: 103 - DNA, 20 bp, synthetic construct
  source 1..20: mol_type = other DNA
ccgcccccaaaagagaagca

SEQ ID NO: 104 - DNA, 20 bp, synthetic construct
  source 1..20: mol_type = other DNA
cccgcccccaaaagagaagc

SEQ ID NO: 105 - DNA, 20 bp, synthetic construct
  source 1..20: mol_type = other DNA
ccccgcccccaaaagagaag

SEQ ID NO: 106 - DNA, 20 bp, synthetic construct
  source 1..20: mol_type = other DNA
accccgcccccaaaagagaa

SEQ ID NO: 107 - DNA, 20 bp, synthetic construct
  source 1..20: mol_type = other DNA
gaccccgcccccaaaagaga

SEQ ID NO: 108 - DNA, 20 bp, synthetic construct
  source 1..20: mol_type = other DNA
agaccccgcccccaaaagag

SEQ ID NO: 109 - DNA, 20 bp, synthetic construct
  source 1..20: mol_type = other DNA
tagaccccgcccccaaaaga

SEQ ID NO: 110 - DNA, 20 bp, synthetic construct
  source 1..20: mol_type = other DNA
ctagaccccgcccccaaaag

SEQ ID NO: 111 - DNA, 20 bp, synthetic construct
  source 1..20: mol_type = other DNA
gctagaccccgcccccaaaa

SEQ ID NO: 112 - DNA, 20 bp, synthetic construct
  source 1..20: mol_type = other DNA
tgctagaccccgcccccaaa

SEQ ID NO: 113 - DNA, 20 bp, synthetic construct
  source 1..20: mol_type = other DNA
ttgctagaccccgcccccaa

SEQ ID NO: 114 - DNA, 20 bp, synthetic construct
  source 1..20: mol_type = other DNA
cttgctagaccccgccccca

SEQ ID NO: 115 - DNA, 20 bp, synthetic construct
  source 1..20: mol_type = other DNA
tcttgctagaccccgccccc

SEQ ID NO: 116 - DNA, 20 bp, synthetic construct
  source 1..20: mol_type = other DNA
ctcttgctagaccccgcccc

SEQ ID NO: 117 - DNA, 20 bp, synthetic construct
  source 1..20: mol_type = other DNA
gctcttgctagaccccgccc

SEQ ID NO: 118 - DNA, 20 bp, synthetic construct
  source 1..20: mol_type = other DNA
tgctcttgctagaccccgcc

SEQ ID NO: 119 - DNA, 20 bp, synthetic construct
  source 1..20: mol_type = other DNA
ctgctcttgctagaccccgc

SEQ ID NO: 120 - DNA, 20 bp, synthetic construct
  source 1..20: mol_type = other DNA
cctgctcttgctagaccccg

SEQ ID NO: 121 - DNA, 20 bp, synthetic construct
  source 1..20: mol_type = other DNA
acctgctcttgctagacccc

SEQ ID NO: 122 - DNA, 20 bp, synthetic construct
  source 1..20: mol_type = other DNA
cacctgctcttgctagaccc

SEQ ID NO: 123 - DNA, 20 bp, synthetic construct
  source 1..20: mol_type = other DNA
acacctgctcttgctagacc

SEQ ID NO: 124 - DNA, 20 bp, synthetic construct
  source 1..20: mol_type = other DNA
cacacctgctcttgctagac

SEQ ID NO: 125 - DNA, 20 bp, synthetic construct
  source 1..20: mol_type = other DNA
ccacacctgctcttgctaga

SEQ ID NO: 126 - DNA, 20 bp, synthetic construct
  source 1..20: mol_type = other DNA
cccacacctgctcttgctag

SEQ ID NO: 127 - DNA, 20 bp, synthetic construct
  source 1..20: mol_type = other DNA
acccacacctgctcttgcta

SEQ ID NO: 128 - DNA, 20 bp, synthetic construct
  source 1..20: mol_type = other DNA
aacccacacctgctcttgct

SEQ ID NO: 129 - DNA, 20 bp, synthetic construct
  source 1..20: mol_type = other DNA
aaacccacacctgctcttgc

SEQ ID NO: 130 - DNA, 20 bp, synthetic construct
  source 1..20: mol_type = other DNA
taaacccacacctgctcttg

SEQ ID NO: 131 - DNA, 20 bp, synthetic construct
  source 1..20: mol_type = other DNA
ctaaacccacacctgctctt

SEQ ID NO: 132 - DNA, 20 bp, synthetic construct
  source 1..20: mol_type = other DNA
cctaaacccacacctgctct

SEQ ID NO: 133 - DNA, 20 bp, synthetic construct
  source 1..20: mol_type = other DNA
tcctaaacccacacctgctc

SEQ ID NO: 134 - DNA, 20 bp, synthetic construct
  source 1..20: mol_type = other DNA
ctcctaaacccacacctgct

SEQ ID NO: 135 - DNA, 20 bp, synthetic construct
  source 1..20: mol_type = other DNA
gtacctgttctgtctttgga

SEQ ID NO: 136 - DNA, 20 bp, synthetic construct
  source 1..20: mol_type = other DNA
ccatcactgagaagtacctg

SEQ ID NO: 137 - DNA, 20 bp, synthetic construct
  source 1..20: mol_type = other DNA
ggcataatgttctgactatc

SEQ ID NO: 138 - DNA, 20 bp, synthetic construct
  source 1..20: mol_type = other DNA
cctcctaaacccacacctgc

SEQ ID NO: 139 - DNA, 20 bp, synthetic construct
  source 1..20: mol_type = other DNA
acctcctaaacccacacctg

SEQ ID NO: 140 - DNA, 20 bp, synthetic construct
  source 1..20: mol_type = other DNA
cacctcctaaacccacacct

SEQ ID NO: 141 - DNA, 20 bp, synthetic construct
  source 1..20: mol_type = other DNA
acacctcctaaacccacacc

SEQ ID NO: 142 - DNA, 20 bp, synthetic construct
  source 1..20: mol_type = other DNA
cacacctcctaaacccacac

SEQ ID NO: 143 - DNA, 20 bp, synthetic construct
  source 1..20: mol_type = other DNA
acacacctcctaaacccaca

SEQ ID NO: 144 - DNA, 20 bp, synthetic construct
  source 1..20: mol_type = other DNA
cacacacctcctaaacccac

SEQ ID NO: 145 - DNA, 20 bp, synthetic construct
  source 1..20: mol_type = other DNA
acacacacctcctaaaccca

SEQ ID NO: 146 - DNA, 20 bp, synthetic construct
  source 1..20: mol_type = other DNA
aacacacacctcctaaaccc

SEQ ID NO: 147 - DNA, 20 bp, synthetic construct
  source 1..20: mol_type = other DNA
aaacacacacctcctaaacc

SEQ ID NO: 148 - DNA, 20 bp, synthetic construct
  source 1..20: mol_type = other DNA
aaaacacacacctcctaaac

SEQ ID NO: 149 - DNA, 20 bp, synthetic construct
  source 1..20: mol_type = other DNA
aaaaacacacacctcctaaa

SEQ ID NO: 150 - DNA, 20 bp, synthetic construct
  source 1..20: mol_type = other DNA
caaaaacacacacctcctaa

SEQ ID NO: 151 - DNA, 20 bp, synthetic construct
  source 1..20: mol_type = other DNA
acaaaaacacacacctccta

SEQ ID NO: 152 - DNA, 20 bp, synthetic construct
  source 1..20: mol_type = other DNA
aacaaaaacacacacctcct

SEQ ID NO: 153 - DNA, 20 bp, synthetic construct
  source 1..20: mol_type = other DNA
aaacaaaaacacacacctcc

SEQ ID NO: 154 - DNA, 20 bp, synthetic construct
  source 1..20: mol_type = other DNA
aaaacaaaaacacacacctc

SEQ ID NO: 155 - DNA, 20 bp, synthetic construct
  source 1..20: mol_type = other DNA
gaaaaacaaaaacacacacc

SEQ ID NO: 156 - DNA, 20 bp, synthetic construct
  source 1..20: mol_type = other DNA
ggaaaaacaaaaacacacac

SEQ ID NO: 157 - DNA, 20 bp, synthetic construct
  source 1..20: mol_type = other DNA
tgggaaaaacaaaaacacac

SEQ ID NO: 158 - DNA, 20 bp, synthetic construct
  source 1..20: mol_type = other DNA
gtgggaaaaacaaaaacaca

SEQ ID NO: 159 - DNA, 20 bp, synthetic construct
  source 1..20: mol_type = other DNA
ggtgggaaaaacaaaaacac

SEQ ID NO: 160 - DNA, 20 bp, synthetic construct
  source 1..20: mol_type = other DNA
ctgtgagagcaagtagtggg

SEQ ID NO: 161 - DNA, 20 bp, synthetic construct
  source 1..20: mol_type = other DNA
actgtgagagcaagtagtgg

SEQ ID NO: 162 - DNA, 20 bp, synthetic construct
  source 1..20: mol_type = other DNA
tactgtgagagcaagtagtg

SEQ ID NO: 163 - DNA, 20 bp, synthetic construct
  source 1..20: mol_type = other DNA
gtactgtgagagcaagtagt

SEQ ID NO: 164 - DNA, 20 bp, synthetic construct
  source 1..20: mol_type = other DNA
agtactgtgagagcaagtag

SEQ ID NO: 165 - DNA, 20 bp, synthetic construct
  source 1..20: mol_type = other DNA
gagtactgtgagagcaagta

SEQ ID NO: 166 - DNA, 20 bp, synthetic construct
  source 1..20: mol_type = other DNA
cgagtactgtgagagcaagt

SEQ ID NO: 167 - DNA, 20 bp, synthetic construct
  source 1..20: mol_type = other DNA
gcgagtactgtgagagcaag

SEQ ID NO: 168 - DNA, 20 bp, synthetic construct
  source 1..20: mol_type = other DNA
agcgagtactgtgagagcaa

SEQ ID NO: 169 - DNA, 20 bp, synthetic construct
  source 1..20: mol_type = other DNA
cagcgagtactgtgagagca

SEQ ID NO: 170 - DNA, 20 bp, synthetic construct
  source 1..20: mol_type = other DNA
tcagcgagtactgtgagagc

SEQ ID NO: 171 - DNA, 20 bp, synthetic construct
  source 1..20: mol_type = other DNA
ctcagcgagtactgtgagag

SEQ ID NO: 172 - DNA, 20 bp, synthetic construct
  source 1..20: mol_type = other DNA
cctcagcgagtactgtgaga

SEQ ID NO: 173 - DNA, 20 bp, synthetic construct
  source 1..20: mol_type = other DNA
ccctcagcgagtactgtgag

SEQ ID NO: 174 - DNA, 20 bp, synthetic construct
  source 1..20: mol_type = other DNA
accctcagcgagtactgtga

SEQ ID NO: 175 - DNA, 20 bp, synthetic construct
  source 1..20: mol_type = other DNA
caccctcagcgagtactgtg

SEQ ID NO: 176 - DNA, 20 bp, synthetic construct
  source 1..20: mol_type = other DNA
tcaccctcagcgagtactgt

SEQ ID NO: 177 - DNA, 20 bp, synthetic construct
  source 1..20: mol_type = other DNA
ttcaccctcagcgagtactg

SEQ ID NO: 178 - DNA, 20 bp, synthetic construct
  source 1..20: mol_type = other DNA
gttcaccctcagcgagtact

SEQ ID NO: 179 - DNA, 20 bp, synthetic construct
  source 1..20: mol_type = other DNA
tgttcaccctcagcgagtac

SEQ ID NO: 180 - DNA, 20 bp, synthetic construct
  source 1..20: mol_type = other DNA
ttgttcaccctcagcgagta

SEQ ID NO: 181 - DNA, 20 bp, synthetic construct
  source 1..20: mol_type = other DNA
cttgttcaccctcagcgagt

SEQ ID NO: 182 - DNA, 20 bp, synthetic construct
  source 1..20: mol_type = other DNA
tcttgttcaccctcagcgag

SEQ ID NO: 183 - DNA, 20 bp, synthetic construct
  source 1..20: mol_type = other DNA
ttcttgttcaccctcagcga

SEQ ID NO: 184 - DNA, 20 bp, synthetic construct
  source 1..20: mol_type = other DNA
tttcttgttcaccctcagcg

SEQ ID NO: 185 - DNA, 20 bp, synthetic construct
  source 1..20: mol_type = other DNA
ttttcttgttcaccctcagc

SEQ ID NO: 186 - DNA, 20 bp, synthetic construct
  source 1..20: mol_type = other DNA
cttttcttgttcaccctcag

SEQ ID NO: 187 - DNA, 20 bp, synthetic construct
  source 1..20: mol_type = other DNA
tcttttcttgttcaccctca

SEQ ID NO: 188 - DNA, 20 bp, synthetic construct
  source 1..20: mol_type = other DNA
gtcttttcttgttcaccctc

SEQ ID NO: 189 - DNA, 20 bp, synthetic construct
  source 1..20: mol_type = other DNA
ggtcttttcttgttcaccct

SEQ ID NO: 190 - DNA, 20 bp, synthetic construct
  source 1..20: mol_type = other DNA
aggtcttttcttgttcaccc

SEQ ID NO: 191 - DNA, 20 bp, synthetic construct
  source 1..20: mol_type = other DNA
caggtcttttcttgttcacc

SEQ ID NO: 192 - DNA, 20 bp, synthetic construct
  source 1..20: mol_type = other DNA
tcaggtcttttcttgttcac

SEQ ID NO: 193 - DNA, 20 bp, synthetic construct
  source 1..20: mol_type = other DNA
atcaggtcttttcttgttca

SEQ ID NO: 194 - DNA, 20 bp, synthetic construct
  source 1..20: mol_type = other DNA
tatcaggtcttttcttgttc

SEQ ID NO: 195 - DNA, 20 bp, synthetic construct
  source 1..20: mol_type = other DNA
ttatcaggtcttttcttgtt

SEQ ID NO: 196 - DNA, 20 bp, synthetic construct
  source 1..20: mol_type = other DNA
tttatcaggtcttttcttgt

SEQ ID NO: 197 - DNA, 20 bp, synthetic construct
  source 1..20: mol_type = other DNA
ctttatcaggtcttttcttg

SEQ ID NO: 198 - DNA, 20 bp, synthetic construct
  source 1..20: mol_type = other DNA
tctttatcaggtcttttctt

SEQ ID NO: 199 - DNA, 20 bp, synthetic construct
  source 1..20: mol_type = other DNA
atctttatcaggtcttttct

SEQ ID NO: 200 - DNA, 20 bp, synthetic construct
  source 1..20: mol_type = other DNA
aatctttatcaggtcttttc

SEQ ID NO: 201 - DNA, 20 bp, synthetic construct
  source 1..20: mol_type = other DNA
taatctttatcaggtctttt

SEQ ID NO: 202 - DNA, 20 bp, synthetic construct
  source 1..20: mol_type = other DNA
ttaatctttatcaggtcttt

SEQ ID NO: 203 - DNA, 20 bp, synthetic construct
  source 1..20: mol_type = other DNA
gttaatctttatcaggtctt

SEQ ID NO: 204 - DNA, 20 bp, synthetic construct
  source 1..20: mol_type = other DNA
ggttaatctttatcaggtct

SEQ ID NO: 205 - DNA, 20 bp, synthetic construct
  source 1..20: mol_type = other DNA
tggttaatctttatcaggtc

SEQ ID NO: 206 - DNA, 20 bp, synthetic construct
  source 1..20: mol_type = other DNA
ctggttaatctttatcaggt

SEQ ID NO: 207 - DNA, 20 bp, synthetic construct
  source 1..20: mol_type = other DNA
tctggttaatctttatcagg

SEQ ID NO: 208 - DNA, 20 bp, synthetic construct
  source 1..20: mol_type = other DNA
ttctggttaatctttatcag

SEQ ID NO: 209 - DNA, 20 bp, synthetic construct
  source 1..20: mol_type = other DNA
cttctggttaatctttatca

SEQ ID NO: 210 - DNA, 20 bp, synthetic construct
  source 1..20: mol_type = other DNA
tcttctggttaatctttatc

SEQ ID NO: 211 - DNA, 20 bp, synthetic construct
  source 1..20: mol_type = other DNA
ttcttctggttaatctttat

SEQ ID NO: 212 - DNA, 20 bp, synthetic construct
  source 1..20: mol_type = other DNA
tttcttctggttaatcttta

SEQ ID NO: 213 - DNA, 20 bp, synthetic construct
  source 1..20: mol_type = other DNA
ttttcttctggttaatcttt

SEQ ID NO: 214 - DNA, 20 bp, synthetic construct
  source 1..20: mol_type = other DNA
gttttcttctggttaatctt

SEQ ID NO: 215 - DNA, 20 bp, synthetic construct
  source 1..20: mol_type = other DNA
tgttttcttctggttaatct

SEQ ID NO: 216 - DNA, 20 bp, synthetic construct
  source 1..20: mol_type = other DNA
ttgttttcttctggttaatc

SEQ ID NO: 217 - DNA, 20 bp, synthetic construct
  source 1..20: mol_type = other DNA
cttgttttcttctggttaat

SEQ ID NO: 218 - DNA, 20 bp, synthetic construct
  source 1..20: mol_type = other DNA
ccttgttttcttctggttaa

SEQ ID NO: 219 - DNA, 20 bp, synthetic construct
  source 1..20: mol_type = other DNA
tccttgttttcttctggtta

SEQ ID NO: 220 - DNA, 20 bp, synthetic construct
  source 1..20: mol_type = other DNA
ctccttgttttcttctggtt

SEQ ID NO: 221 - DNA, 20 bp, synthetic construct
  source 1..20: mol_type = other DNA
cctccttgttttcttctggt

SEQ ID NO: 222 - DNA, 20 bp, synthetic construct
  source 1..20: mol_type = other DNA
ccctccttgttttcttctgg

SEQ ID NO: 223 - DNA, 20 bp, synthetic construct
  source 1..20: mol_type = other DNA
tccctccttgttttcttctg

SEQ ID NO: 224 - DNA, 20 bp, synthetic construct
  source 1..20: mol_type = other DNA
ttccctccttgttttcttct

SEQ ID NO: 225 - DNA, 20 bp, synthetic construct
  source 1..20: mol_type = other DNA
tttccctccttgttttcttc

SEQ ID NO: 226 - DNA, 20 bp, synthetic construct
  source 1..20: mol_type = other DNA
gtttccctccttgttttctt

SEQ ID NO: 227 - DNA, 20 bp, synthetic construct
  source 1..20: mol_type = other DNA
tgtttccctccttgttttct

SEQ ID NO: 228 - DNA, 20 bp, synthetic construct
  source 1..20: mol_type = other DNA
ttgtttccctccttgttttc

SEQ ID NO: 229 - DNA, 20 bp, synthetic construct
  source 1..20: mol_type = other DNA
gttgtttccctccttgtttt

SEQ ID NO: 230 - DNA, 20 bp, synthetic construct
  source 1..20: mol_type = other DNA
ggttgtttccctccttgttt

SEQ ID NO: 231 - DNA, 20 bp, synthetic construct
  source 1..20: mol_type = other DNA
cggttgtttccctccttgtt

SEQ ID NO: 232 - DNA, 20 bp, synthetic construct
  source 1..20: mol_type = other DNA
gcggttgtttccctccttgt

SEQ ID NO: 233 - DNA, 20 bp, synthetic construct
  source 1..20: mol_type = other DNA
tgcggttgtttccctccttg

SEQ ID NO: 234 - DNA, 20 bp, synthetic construct
  source 1..20: mol_type = other DNA
ctgcggttgtttccctcctt

SEQ ID NO: 235 - DNA, 20 bp, synthetic construct
  source 1..20: mol_type = other DNA
gctgcggttgtttccctcct

SEQ ID NO: 236 - DNA, 20 bp, synthetic construct
  source 1..20: mol_type = other DNA
ggctgcggttgtttccctcc

SEQ ID NO: 237 - DNA, 20 bp, synthetic construct
  source 1..20: mol_type = other DNA
aggctgcggttgtttccctc

SEQ ID NO: 238 - DNA, 20 bp, synthetic construct
  source 1..20: mol_type = other DNA
caggctgcggttgtttccct

SEQ ID NO: 239 - DNA, 20 bp, synthetic construct
  source 1..20: mol_type = other DNA
acaggctgcggttgtttccc

SEQ ID NO: 240 - DNA, 20 bp, synthetic construct
  source 1..20: mol_type = other DNA
ctacaggctgcggttgtttc

SEQ ID NO: 241 - DNA, 20 bp, synthetic construct
  source 1..20: mol_type = other DNA
gctacaggctgcggttgttt

SEQ ID NO: 242 - DNA, 20 bp, synthetic construct
  source 1..20: mol_type = other DNA
tgctacaggctgcggttgtt

SEQ ID NO: 243 - DNA, 20 bp, synthetic construct
  source 1..20: mol_type = other DNA
ttgctacaggctgcggttgt

SEQ ID NO: 244 - DNA, 20 bp, synthetic construct
  source 1..20: mol_type = other DNA
cttgctacaggctgcggttg

SEQ ID NO: 245 - DNA, 20 bp, synthetic construct
  source 1..20: mol_type = other DNA
gcttgctacaggctgcggtt

SEQ ID NO: 246 - DNA, 20 bp, synthetic construct
  source 1..20: mol_type = other DNA
agcttgctacaggctgcggt

SEQ ID NO: 247 - DNA, 20 bp, synthetic construct
  source 1..20: mol_type = other DNA
gagcttgctacaggctgcgg

SEQ ID NO: 248 - DNA, 20 bp, synthetic construct
  source 1..20: mol_type = other DNA
agagcttgctacaggctgcg

SEQ ID NO: 249 - DNA, 20 bp, synthetic construct
  source 1..20: mol_type = other DNA
aaaaaacagtagttgtggtc

SEQ ID NO: 250 - DNA, 20 bp, synthetic construct
  source 1..20: mol_type = other DNA
gccaactcagatttcacctt

SEQ ID NO: 251 - DNA, 20 bp, synthetic construct
  source 1..20: mol_type = other DNA
ccagagcttgctacaggctg

SEQ ID NO: 252 - DNA, 20 bp, synthetic construct
  source 1..20: mol_type = other DNA
tccagagcttgctacaggct

SEQ ID NO: 253 - DNA, 20 bp, synthetic construct
  source 1..20: mol_type = other DNA
ttccagagcttgctacaggc

SEQ ID NO: 254 - DNA, 20 bp, synthetic construct
  source 1..20: mol_type = other DNA
gttccagagcttgctacagg

SEQ ID NO: 255 - DNA, 20 bp, synthetic construct
  source 1..20: mol_type = other DNA
agttccagagcttgctacag

SEQ ID NO: 256 - DNA, 20 bp, synthetic construct
  source 1..20: mol_type = other DNA
gagttccagagcttgctaca

SEQ ID NO: 257 - DNA, 20 bp, synthetic construct
  source 1..20: mol_type = other DNA
tgagttccagagcttgctac

SEQ ID NO: 258 - DNA, 20 bp, synthetic construct
  source 1..20: mol_type = other DNA
ctgagttccagagcttgcta

SEQ ID NO: 259 - DNA, 20 bp, synthetic construct
  source 1..20: mol_type = other DNA
cctgagttccagagcttgct

SEQ ID NO: 260 - DNA, 20 bp, synthetic construct
  source 1..20: mol_type = other DNA
tcctgagttccagagcttgc

SEQ ID NO: 261 - DNA, 20 bp, synthetic construct
  source 1..20: mol_type = other DNA
ctcctgagttccagagcttg

SEQ ID NO: 262 - DNA, 20 bp, synthetic construct
  source 1..20: mol_type = other DNA
actcctgagttccagagctt

SEQ ID NO: 263 - DNA, 20 bp, synthetic construct
  source 1..20: mol_type = other DNA
gactcctgagttccagagct

SEQ ID NO: 264 - DNA, 20 bp, synthetic construct
  source 1..20: mol_type = other DNA
cgactcctgagttccagagc

SEQ ID NO: 265 - DNA, 20 bp, synthetic construct
  source 1..20: mol_type = other DNA
gcgactcctgagttccagag

SEQ ID NO: 266 - DNA, 20 bp, synthetic construct
  source 1..20: mol_type = other DNA
cgcgactcctgagttccaga

SEQ ID NO: 267 - DNA, 20 bp, synthetic construct
  source 1..20: mol_type = other DNA
gcgcgactcctgagttccag

SEQ ID NO: 268 - DNA, 20 bp, synthetic construct
  source 1..20: mol_type = other DNA
cgcgcgactcctgagttcca

SEQ ID NO: 269 - DNA, 20 bp, synthetic construct
  source 1..20: mol_type = other DNA
gcgcgcgactcctgagttcc

SEQ ID NO: 270 - DNA, 20 bp, synthetic construct
  source 1..20: mol_type = other DNA
agcgcgcgactcctgagttc

SEQ ID NO: 271 - DNA, 20 bp, synthetic construct
  source 1..20: mol_type = other DNA
tagcgcgcgactcctgagtt

SEQ ID NO: 272 - DNA, 20 bp, synthetic construct
  source 1..20: mol_type = other DNA
ctagcgcgcgactcctgagt

SEQ ID NO: 273 - DNA, 20 bp, synthetic construct
  source 1..20: mol_type = other DNA
cctagcgcgcgactcctgag

SEQ ID NO: 274 - DNA, 20 bp, synthetic construct
  source 1..20: mol_type = other DNA
ccctagcgcgcgactcctga

SEQ ID NO: 275 - DNA, 20 bp, synthetic construct
  source 1..20: mol_type = other DNA
cccctagcgcgcgactcctg

SEQ ID NO: 276 - DNA, 20 bp, synthetic construct
  source 1..20: mol_type = other DNA
gcccctagcgcgcgactcct

SEQ ID NO: 277 - DNA, 20 bp, synthetic construct
  source 1..20: mol_type = other DNA
ggcccctagcgcgcgactcc

SEQ ID NO: 278 - DNA, 20 bp, synthetic construct
  source 1..20: mol_type = other DNA
cggcccctagcgcgcgactc

SEQ ID NO: 279 - DNA, 20 bp, synthetic construct
  source 1..20: mol_type = other DNA
ccggcccctagcgcgcgact

SEQ ID NO: 280 - DNA, 20 bp, synthetic construct
  source 1..20: mol_type = other DNA
ccccggcccctagcgcgcga

SEQ ID NO: 281 - DNA, 20 bp, synthetic construct
  source 1..20: mol_type = other DNA
gccccggcccctagcgcgcg

SEQ ID NO: 282 - DNA, 20 bp, synthetic construct
  source 1..20: mol_type = other DNA
ggccccggcccctagcgcgc

SEQ ID NO: 283 - DNA, 20 bp, synthetic construct
  source 1..20: mol_type = other DNA
cggccccggcccctagcgcg

SEQ ID NO: 284 - DNA, 20 bp, synthetic construct
  source 1..20: mol_type = other DNA
ccggccccggcccctagcgc

SEQ ID NO: 285 - DNA, 20 bp, synthetic construct
  source 1..20: mol_type = other DNA
cccggccccggcccctagcg

SEQ ID NO: 286 - DNA, 20 bp, synthetic construct
  source 1..20: mol_type = other DNA
ccccggccccggcccctagc

SEQ ID NO: 287 - DNA, 20 bp, synthetic construct
  source 1..20: mol_type = other DNA
gccccggccccggcccctag

SEQ ID NO: 288 - DNA, 20 bp, synthetic construct
  source 1..20: mol_type = other DNA
ggccccggccccggccccta

SEQ ID NO: 289 - DNA, 20 bp, synthetic construct
  source 1..20: mol_type = other DNA
acgccccggccccggccccg

SEQ ID NO: 290 - DNA, 20 bp, synthetic construct
  source 1..20: mol_type = other DNA
cacgccccggccccggcccc

SEQ ID NO: 291 - DNA, 20 bp, synthetic construct
  source 1..20: mol_type = other DNA
ccacgccccggccccggccc

SEQ ID NO: 292 - DNA, 20 bp, synthetic construct
  source 1..20: mol_type = other DNA
accacgccccggccccggcc

SEQ ID NO: 293 - DNA, 20 bp, synthetic construct
  source 1..20: mol_type = other DNA
gaccacgccccggccccggc

SEQ ID NO: 294 - DNA, 20 bp, synthetic construct
  source 1..20: mol_type = other DNA
cgaccacgccccggccccgg

SEQ ID NO: 295 - DNA, 20 bp, synthetic construct
  source 1..20: mol_type = other DNA
ccgaccacgccccggccccg

SEQ ID NO: 296 - DNA, 20 bp, synthetic construct
  source 1..20: mol_type = other DNA
cccgaccacgccccggcccc

SEQ ID NO: 297 - DNA, 20 bp, synthetic construct
  source 1..20: mol_type = other DNA
ccccgaccacgccccggccc

SEQ ID NO: 298 - DNA, 20 bp, synthetic construct
  source 1..20: mol_type = other DNA
gccccgaccacgccccggcc

SEQ ID NO: 299 - DNA, 20 bp, synthetic construct
  source 1..20: mol_type = other DNA
cgccccgaccacgccccggc

SEQ ID NO: 300 - DNA, 20 bp, synthetic construct
  source 1..20: mol_type = other DNA
ccgccccgaccacgccccgg

SEQ ID NO: 301 - DNA, 20 bp, synthetic construct
  source 1..20: mol_type = other DNA
cccgccccgaccacgccccg

SEQ ID NO: 302 - DNA, 20 bp, synthetic construct
  source 1..20: mol_type = other DNA
gcccgccccgaccacgcccc

SEQ ID NO: 303 - DNA, 20 bp, synthetic construct
  source 1..20: mol_type = other DNA
ggcccgccccgaccacgccc

SEQ ID NO: 304 - DNA, 20 bp, synthetic construct
  source 1..20: mol_type = other DNA
gggcccgccccgaccacgcc

SEQ ID NO: 305 - DNA, 20 bp, synthetic construct
  source 1..20: mol_type = other DNA
cgggcccgccccgaccacgc

SEQ ID NO: 306 - DNA, 20 bp, synthetic construct
  source 1..20: mol_type = other DNA
ccgggcccgccccgaccacg

SEQ ID NO: 307 - DNA, 20 bp, synthetic construct
  source 1..20: mol_type = other DNA
cccgggcccgccccgaccac

SEQ ID NO: 308 - DNA, 20 bp, synthetic construct
  source 1..20: mol_type = other DNA
ccccgggcccgccccgacca

SEQ ID NO: 309 - DNA, 20 bp, synthetic construct
  source 1..20: mol_type = other DNA
cccccgggcccgccccgacc

SEQ ID NO: 310 - DNA, 20 bp, synthetic construct
  source 1..20: mol_type = other DNA
gcccccgggcccgccccgac

SEQ ID NO: 311 - DNA, 20 bp, synthetic construct
  source 1..20: mol_type = other DNA
cgcccccgggcccgccccga

SEQ ID NO: 312 - DNA, 20 bp, synthetic construct
  source 1..20: mol_type = other DNA
cccgcccccgggcccgcccc

SEQ ID NO: 313 - DNA, 20 bp, synthetic construct
  source 1..20: mol_type = other DNA
gcccgcccccgggcccgccc

SEQ ID NO: 314 - DNA, 20 bp, synthetic construct
  source 1..20: mol_type = other DNA
ggcccgcccccgggcccgcc

SEQ ID NO: 315 - DNA, 20 bp, synthetic construct
  source 1..20: mol_type = other DNA
cgccccgggcccgcccccgg

SEQ ID NO: 316 - DNA, 20 bp, synthetic construct
  source 1..20: mol_type = other DNA
cccgccccgggcccgccccc

SEQ ID NO: 317 - DNA, 20 bp, synthetic construct
  source 1..20: mol_type = other DNA
ccccgccccgggcccgcccc

SEQ ID NO: 318 - DNA, 20 bp, synthetic construct
  source 1..20: mol_type = other DNA
gccccgccccgggcccgccc

SEQ ID NO: 319 - DNA, 20 bp, synthetic construct
  source 1..20: mol_type = other DNA
agccccgccccgggcccgcc

SEQ ID NO: 320 - DNA, 20 bp, synthetic construct
  source 1..20: mol_type = other DNA
cagccccgccccgggcccgc

SEQ ID NO: 321 - DNA, 20 bp, synthetic construct
  source 1..20: mol_type = other DNA
gcagccccgccccgggcccg

SEQ ID NO: 322 - DNA, 20 bp, synthetic construct
  source 1..20: mol_type = other DNA
cgcagccccgccccgggccc

SEQ ID NO: 323 - DNA, 20 bp, synthetic construct
  source 1..20: mol_type = other DNA
ctacacaccaaagaatgcca

SEQ ID NO: 324 - DNA, 20 bp, synthetic construct
  source 1..20: mol_type = other DNA
ggaataaggtcactagttcg

SEQ ID NO: 325 - DNA, 20 bp, synthetic construct
  source 1..20: mol_type = other DNA
cagagcttgctacaggctgc

SEQ ID NO: 326 - DNA, 20 bp, synthetic construct
  source 1..20: mol_type = other DNA
ccgcagccccgccccgggcc

SEQ ID NO: 327 - DNA, 20 bp, synthetic construct
  source 1..20: mol_type = other DNA
accgcagccccgccccgggc

SEQ ID NO: 328 - DNA, 20 bp, synthetic construct
  source 1..20: mol_type = other DNA
aaccgcagccccgccccggg

SEQ ID NO: 329 - DNA, 20 bp, synthetic construct
  source 1..20: mol_type = other DNA
caaccgcagccccgccccgg

SEQ ID NO: 330 - DNA, 20 bp, synthetic construct
  source 1..20: mol_type = other DNA
gcaaccgcagccccgccccg

SEQ ID NO: 331 - DNA, 20 bp, synthetic construct
  source 1..20: mol_type = other DNA
cgcaaccgcagccccgcccc

SEQ ID NO: 332 - DNA, 20 bp, synthetic construct
  source 1..20: mol_type = other DNA
ccgcaaccgcagccccgccc

SEQ ID NO: 333 - DNA, 20 bp, synthetic construct
  source 1..20: mol_type = other DNA
accgcaaccgcagccccgcc

SEQ ID NO: 334 - DNA, 20 bp, synthetic construct
  source 1..20: mol_type = other DNA
caccgcaaccgcagccccgc

SEQ ID NO: 335 - DNA, 20 bp, synthetic construct
  source 1..20: mol_type = other DNA
gcaccgcaaccgcagccccg

SEQ ID NO: 336 - DNA, 20 bp, synthetic construct
  source 1..20: mol_type = other DNA
ggcaccgcaaccgcagcccc

SEQ ID NO: 337 - DNA, 20 bp, synthetic construct
  source 1..20: mol_type = other DNA
aggcaccgcaaccgcagccc

SEQ ID NO: 338 - DNA, 20 bp, synthetic construct
  source 1..20: mol_type = other DNA
caggcaccgcaaccgcagcc

SEQ ID NO: 339 - DNA, 20 bp, synthetic construct
  source 1..20: mol_type = other DNA
gcaggcaccgcaaccgcagc

SEQ ID NO: 340 - DNA, 20 bp, synthetic construct
  source 1..20: mol_type = other DNA
cgcaggcaccgcaaccgcag

SEQ ID NO: 341 - DNA, 20 bp, synthetic construct
  source 1..20: mol_type = other DNA
gcgcaggcaccgcaaccgca

SEQ ID NO: 342 - DNA, 20 bp, synthetic construct
  source 1..20: mol_type = other DNA
ggcgcaggcaccgcaaccgc

SEQ ID NO: 343 - DNA, 20 bp, synthetic construct
  source 1..20: mol_type = other DNA
gggcgcaggcaccgcaaccg

SEQ ID NO: 344 - DNA, 20 bp, synthetic construct
  source 1..20: mol_type = other DNA
tctctctttcctagcgggac

SEQ ID NO: 345 - DNA, 20 bp, synthetic construct
  source 1..20: mol_type = other DNA
atctctctttcctagcggga

SEQ ID NO: 346 - DNA, 20 bp, synthetic construct
  source 1..20: mol_type = other DNA
tatctctctttcctagcggg

SEQ ID NO: 347 - DNA, 20 bp, synthetic construct
  source 1..20: mol_type = other DNA
atatctctctttcctagcgg

SEQ ID NO: 348 - DNA, 20 bp, synthetic construct
  source 1..20: mol_type = other DNA
gatatctctctttcctagcg

SEQ ID NO: 349 - DNA, 20 bp, synthetic construct
  source 1..20: mol_type = other DNA
agatatctctctttcctagc

SEQ ID NO: 350 - DNA, 20 bp, synthetic construct
  source 1..20: mol_type = other DNA
gagatatctctctttcctag

SEQ ID NO: 351 - DNA, 20 bp, synthetic construct
  source 1..20: mol_type = other DNA
ggagatatctctctttccta

SEQ ID NO: 352 - DNA, 20 bp, synthetic construct
  source 1..20: mol_type = other DNA
cggagatatctctctttcct

SEQ ID NO: 353 - DNA, 20 bp, synthetic construct
  source 1..20: mol_type = other DNA
ccggagatatctctctttcc

SEQ ID NO: 354 - DNA, 20 bp, synthetic construct
  source 1..20: mol_type = other DNA
tccggagatatctctctttc

SEQ ID NO: 355 - DNA, 20 bp, synthetic construct
  source 1..20: mol_type = other DNA
ctccggagatatctctcttt

SEQ ID NO: 356 - DNA, 20 bp, synthetic construct
  source 1..20: mol_type = other DNA
gctccggagatatctctctt

SEQ ID NO: 357 - DNA, 20 bp, synthetic construct
  source 1..20: mol_type = other DNA
tgctccggagatatctctct

SEQ ID NO: 358 - DNA, 20 bp, synthetic construct
  source 1..20: mol_type = other DNA
atgctccggagatatctctc

SEQ ID NO: 359 - DNA, 20 bp, synthetic construct
  source 1..20: mol_type = other DNA
aatgctccggagatatctct

SEQ ID NO: 360 - DNA, 20 bp, synthetic construct
  source 1..20: mol_type = other DNA
tctgctcttgctagaccccg

SEQ ID NO: 361 - DNA, 20 bp, synthetic construct
  source 1..20: mol_type = other DNA
atctgctcttgctagacccc

SEQ ID NO: 362 - DNA, 20 bp, synthetic construct
  source 1..20: mol_type = other DNA
tatctgctcttgctagaccc

SEQ ID NO: 363 - DNA, 20 bp, synthetic construct
  source 1..20: mol_type = other DNA
atatctgctcttgctagacc

SEQ ID NO: 364 - DNA, 20 bp, synthetic construct
  source 1..20: mol_type = other DNA
gatatctgctcttgctagac

SEQ ID NO: 365 - DNA, 20 bp, synthetic construct
  source 1..20: mol_type = other DNA
agatatctgctcttgctaga

SEQ ID NO: 366 - DNA, 20 bp, synthetic construct
  source 1..20: mol_type = other DNA
gagatatctgctcttgctag

SEQ ID NO: 367 - DNA, 20 bp, synthetic construct
  source 1..20: mol_type = other DNA
ggagatatctgctcttgcta

SEQ ID NO: 368 - DNA, 20 bp, synthetic construct
  source 1..20: mol_type = other DNA
cggagatatctgctcttgct

SEQ ID NO: 369 - DNA, 20 bp, synthetic construct
  source 1..20: mol_type = other DNA
ccggagatatctgctcttgc

SEQ ID NO: 370 - DNA, 20 bp, synthetic construct
  source 1..20: mol_type = other DNA
tccggagatatctgctcttg

SEQ ID NO: 371 - DNA, 20 bp, synthetic construct
  source 1..20: mol_type = other DNA
ctccggagatatctgctctt

SEQ ID NO: 372 - DNA, 20 bp, synthetic construct
  source 1..20: mol_type = other DNA
gctccggagatatctgctct

SEQ ID NO: 373 - DNA, 20 bp, synthetic construct
  source 1..20: mol_type = other DNA
tgctccggagatatctgctc

SEQ ID NO: 374 - DNA, 20 bp, synthetic construct
  source 1..20: mol_type = other DNA
atgctccggagatatctgct

SEQ ID NO: 375 - DNA, 20 bp, synthetic construct
  source 1..20: mol_type = other DNA
aatgctccggagatatctgc

SEQ ID NO: 376 - DNA, 20 bp, synthetic construct
  source 1..20: mol_type = other DNA
aaatgctccggagatatctg

SEQ ID NO: 377 - DNA, 20 bp, synthetic construct
  source 1..20: mol_type = other DNA
tgctccggagatatcaagcg

SEQ ID NO: 378 - DNA, 20 bp, synthetic construct
  source 1..20: mol_type = other DNA
atgctccggagatatcaagc

SEQ ID NO: 379 - DNA, 20 bp, synthetic construct
  source 1..20: mol_type = other DNA
aatgctccggagatatcaag

SEQ ID NO: 380 - DNA, 20 bp, synthetic construct
  source 1..20: mol_type = other DNA
aaatgctccggagatatcaa

SEQ ID NO: 381 - DNA, 20 bp, synthetic construct
  source 1..20: mol_type = other DNA
caaatgctccggagatatca

SEQ ID NO: 382 - DNA, 20 bp, synthetic construct
  source 1..20: mol_type = other DNA
ggtaacttcaaactcttggg

SEQ ID NO: 383 - DNA, 20 bp, synthetic construct
  source 1..20: mol_type = other DNA
gccatgatttcttgtctggg

SEQ ID NO: 384 - DNA, 20 bp, synthetic construct
  source 1..20: mol_type = other DNA
tctcctaaacccacacctgc

SEQ ID NO: 385 - DNA, 20 bp, synthetic construct
  source 1..20: mol_type = other DNA
atctcctaaacccacacctg

SEQ ID NO: 386 - DNA, 20 bp, synthetic construct
  source 1..20: mol_type = other DNA
tatctcctaaacccacacct

SEQ ID NO: 387 - DNA, 20 bp, synthetic construct
  source 1..20: mol_type = other DNA
atatctcctaaacccacacc

SEQ ID NO: 388 - DNA, 20 bp, synthetic construct
  source 1..20: mol_type = other DNA
gatatctcctaaacccacac

SEQ ID NO: 389 - DNA, 20 bp, synthetic construct
  source 1..20: mol_type = other DNA
agatatctcctaaacccaca

SEQ ID NO: 390 - DNA, 20 bp, synthetic construct
  source 1..20: mol_type = other DNA
gagatatctcctaaacccac

SEQ ID NO: 391 - DNA, 20 bp, synthetic construct
  source 1..20: mol_type = other DNA
ggagatatctcctaaaccca

SEQ ID NO: 392 - DNA, 20 bp, synthetic construct
  source 1..20: mol_type = other DNA
cggagatatctcctaaaccc

SEQ ID NO: 393 - DNA, 20 bp, synthetic construct
  source 1..20: mol_type = other DNA
ccggagatatctcctaaacc

SEQ ID NO: 394 - DNA, 20 bp, synthetic construct
  source 1..20: mol_type = other DNA
tccggagatatctcctaaac

SEQ ID NO: 395 - DNA, 20 bp, synthetic construct
  source 1..20: mol_type = other DNA
ctccggagatatctcctaaa

SEQ ID NO: 396 - DNA, 20 bp, synthetic construct
  source 1..20: mol_type = other DNA
gctccggagatatctcctaa

SEQ ID NO: 397 - DNA, 20 bp, synthetic construct
  source 1..20: mol_type = other DNA
tgctccggagatatctccta

SEQ ID NO: 398 - DNA, 20 bp, synthetic construct
  source 1..20: mol_type = other DNA
atgctccggagatatctcct

SEQ ID NO: 399 - DNA, 20 bp, synthetic construct
  source 1..20: mol_type = other DNA
aatgctccggagatatctcc

SEQ ID NO: 400 - DNA, 20 bp, synthetic construct
  source 1..20: mol_type = other DNA
aaatgctccggagatatctc

SEQ ID NO: 401 - DNA, 20 bp, synthetic construct
  source 1..20: mol_type = other DNA
gggacactacaaggtagtat

SEQ ID NO: 402-440 - skipped (39 entries)

SEQ ID NO: 441 - DNA, 20 bp, synthetic construct
  source 1..20: mol_type = other DNA
tcacattatccaaatgctcc

SEQ ID NO: 442 - DNA, 20 bp, synthetic construct
  source 1..20: mol_type = other DNA
ctgtcacattatccaaatgc

SEQ ID NO: 443 - DNA, 20 bp, synthetic construct
  source 1..20: mol_type = other DNA
caactgtcacattatccaaa

SEQ ID NO: 444 - DNA, 20 bp, synthetic construct
  source 1..20: mol_type = other DNA
ttccaactgtcacattatcc

SEQ ID NO: 445 - DNA, 20 bp, synthetic construct
  source 1..20: mol_type = other DNA
tgcattccaactgtcacatt

SEQ ID NO: 446 - DNA, 20 bp, synthetic construct
  source 1..20: mol_type = other DNA
cactgcattccaactgtcac

SEQ ID NO: 447 - DNA, 20 bp, synthetic construct
  source 1..20: mol_type = other DNA
catcactgcattccaactgt

SEQ ID NO: 448 - DNA, 20 bp, synthetic construct
  source 1..20: mol_type = other DNA
cgacatcactgcattccaac

SEQ ID NO: 449 - DNA, 20 bp, synthetic construct
  source 1..20: mol_type = other DNA
agtcgacatcactgcattcc

SEQ ID NO: 450 - DNA, 20 bp, synthetic construct
  source 1..20: mol_type = other DNA
aagagtcgacatcactgcat

SEQ ID NO: 451 - DNA, 20 bp, synthetic construct
  source 1..20: mol_type = other DNA
gcaaagagtcgacatcactg

SEQ ID NO: 452 - DNA, 20 bp, synthetic construct
  source 1..20: mol_type = other DNA
tgggcaaagagtcgacatca

SEQ ID NO: 453 - DNA, 20 bp, synthetic construct
  source 1..20: mol_type = other DNA
cggtgggcaaagagtcgaca

SEQ ID NO: 454 - DNA, 20 bp, synthetic construct
  source 1..20: mol_type = other DNA
tggcggtgggcaaagagtcg

SEQ ID NO: 455 - DNA, 20 bp, synthetic construct
  source 1..20: mol_type = other DNA
gagatggcggtgggcaaaga

SEQ ID NO: 456 - DNA, 20 bp, synthetic construct
  source 1..20: mol_type = other DNA
ctggagatggcggtgggcaa

SEQ ID NO: 457 - DNA, 20 bp, synthetic construct
  source 1..20: mol_type = other DNA
acagctggagatggcggtgg

SEQ ID NO: 458 - DNA, 20 bp, synthetic construct
  source 1..20: mol_type = other DNA
gcaacagctggagatggcgg

SEQ ID NO: 459 - DNA, 20 bp, synthetic construct
  source 1..20: mol_type = other DNA
ttggcaacagctggagatgg

SEQ ID NO: 460 - DNA, 20 bp, synthetic construct
  source 1..20: mol_type = other DNA
gtcttggcaacagctggaga

SEQ ID NO: 461 - DNA, 20 bp, synthetic construct
  source 1..20: mol_type = other DNA
tctgtcttggcaacagctgg

SEQ ID NO: 462 - DNA, 20 bp, synthetic construct
  source 1..20: mol_type = other DNA
tctctgtcttggcaacagct

SEQ ID NO: 463 - DNA, 20 bp, synthetic construct
  source 1..20: mol_type = other DNA
gcaatctctgtcttggcaac

SEQ ID NO: 464 - DNA, 20 bp, synthetic construct
  source 1..20: mol_type = other DNA
agcaatctctgtcttggcaa

SEQ ID NO: 465 - DNA, 20 bp, synthetic construct
  source 1..20: mol_type = other DNA
aaagcaatctctgtcttggc

SEQ ID NO: 466 - DNA, 20 bp, synthetic construct
  source 1..20: mol_type = other DNA
cttaaagcaatctctgtctt

SEQ ID NO: 467 - DNA, 20 bp, synthetic construct
  source 1..20: mol_type = other DNA
ccacttaaagcaatctctgt

SEQ ID NO: 468 - DNA, 20 bp, synthetic construct
  source 1..20: mol_type = other DNA
agctgctaataaaggtgatt

SEQ ID NO: 469 - DNA, 20 bp, synthetic construct
  source 1..20: mol_type = other DNA
agtagctgctaataaaggtg

SEQ ID NO: 470 - DNA, 20 bp, synthetic construct
  source 1..20: mol_type = other DNA
aaaagtagctgctaataaag

SEQ ID NO: 471 - DNA, 20 bp, synthetic construct
  source 1..20: mol_type = other DNA
agcaaaagtagctgctaata

SEQ ID NO: 472 - DNA, 20 bp, synthetic construct
  source 1..20: mol_type = other DNA
gtaagcaaaagtagctgcta

SEQ ID NO: 473 - DNA, 20 bp, synthetic construct
  source 1..20: mol_type = other DNA
ccagtaagcaaaagtagctg

SEQ ID NO: 474 - DNA, 20 bp, synthetic construct
  source 1..20: mol_type = other DNA
gtcccagtaagcaaaagtag

SEQ ID NO: 475 - DNA, 20 bp, synthetic construct
  source 1..20: mol_type = other DNA
tgtcccagtaagcaaaagta

SEQ ID NO: 476 - DNA, 20 bp, synthetic construct
  source 1..20: mol_type = other DNA
attgtcccagtaagcaaaag

SEQ ID NO: 477 - DNA, 20 bp, synthetic construct
  source 1..20: mol_type = other DNA
atattgtcccagtaagcaaa

SEQ ID NO: 478 - DNA, 20 bp, synthetic construct
  source 1..20: mol_type = other DNA
aatattgtcccagtaagcaa

SEQ ID NO: 479 - DNA, 20 bp, synthetic construct
  source 1..20: mol_type = other DNA
aagaatattgtcccagtaag

SEQ ID NO: 480 - DNA, 20 bp, synthetic construct
  source 1..20: mol_type = other DNA
accaagaatattgtcccagt

SEQ ID NO: 481 - DNA, 20 bp, synthetic construct
  source 1..20: mol_type = other DNA
aggaccaagaatattgtccc

SEQ ID NO: 482 - DNA, 20 bp, synthetic construct
  source 1..20: mol_type = other DNA
tctaggaccaagaatattgt

SEQ ID NO: 483 - DNA, 20 bp, synthetic construct
  source 1..20: mol_type = other DNA
tactctaggaccaagaatat

SEQ ID NO: 484 - DNA, 20 bp, synthetic construct
  source 1..20: mol_type = other DNA
ccttactctaggaccaagaa

SEQ ID NO: 485 - DNA, 20 bp, synthetic construct
  source 1..20: mol_type = other DNA
gtgccttactctaggaccaa

SEQ ID NO: 486 - DNA, 20 bp, synthetic construct
  source 1..20: mol_type = other DNA
aatgtgccttactctaggac

SEQ ID NO: 487 - DNA, 20 bp, synthetic construct
  source 1..20: mol_type = other DNA
agcccaaatgtgccttactc

SEQ ID NO: 488 - DNA, 20 bp, synthetic construct
  source 1..20: mol_type = other DNA
ctttggagcccaaatgtgcc

SEQ ID NO: 489 - DNA, 20 bp, synthetic construct
  source 1..20: mol_type = other DNA
tgtctttggagcccaaatgt

SEQ ID NO: 490 - DNA, 20 bp, synthetic construct
  source 1..20: mol_type = other DNA
ttctgtctttggagcccaaa

SEQ ID NO: 491 - DNA, 20 bp, synthetic construct
  source 1..20: mol_type = other DNA
gttctgtctttggagcccaa

SEQ ID NO: 492 - DNA, 20 bp, synthetic construct
  source 1..20: mol_type = other DNA
ctgttctgtctttggagccc

SEQ ID NO: 493 - DNA, 20 bp, synthetic construct
  source 1..20: mol_type = other DNA
tacctgttctgtctttggag

SEQ ID NO: 494 - DNA, 20 bp, synthetic construct
  source 1..20: mol_type = other DNA
aagtacctgttctgtctttg

SEQ ID NO: 495 - DNA, 20 bp, synthetic construct
  source 1..20: mol_type = other DNA
gagaagtacctgttctgtct

SEQ ID NO: 496 - DNA, 20 bp, synthetic construct
  source 1..20: mol_type = other DNA
actgagaagtacctgttctg

SEQ ID NO: 497 - DNA, 20 bp, synthetic construct
  source 1..20: mol_type = other DNA
tcactgagaagtacctgttc

SEQ ID NO: 498 - DNA, 20 bp, synthetic construct
  source 1..20: mol_type = other DNA
atcactgagaagtacctgtt

SEQ ID NO: 499 - DNA, 20 bp, synthetic construct
  source 1..20: mol_type = other DNA
tccatcactgagaagtacct

SEQ ID NO: 500 - DNA, 20 bp, synthetic construct
  source 1..20: mol_type = other DNA
tttctccatcactgagaagt

SEQ ID NO: 501 - DNA, 20 bp, synthetic construct
  source 1..20: mol_type = other DNA
ttatttctccatcactgaga

SEQ ID NO: 502 - DNA, 20 bp, synthetic construct
  source 1..20: mol_type = other DNA
aagttatttctccatcactg

SEQ ID NO: 503 - DNA, 20 bp, synthetic construct
  source 1..20: mol_type = other DNA
gaaaagttatttctccatca

SEQ ID NO: 504 - DNA, 20 bp, synthetic construct
  source 1..20: mol_type = other DNA
ggttggcaagaaaagttatt

SEQ ID NO: 505 - DNA, 20 bp, synthetic construct
  source 1..20: mol_type = other DNA
tgtggttggcaagaaaagtt

SEQ ID NO: 506 - DNA, 20 bp, synthetic construct
  source 1..20: mol_type = other DNA
gagtgtggttggcaagaaaa

SEQ ID NO: 507 - DNA, 20 bp, synthetic construct
  source 1..20: mol_type = other DNA
ttagagtgtggttggcaaga

SEQ ID NO: 508 - DNA, 20 bp, synthetic construct
  source 1..20: mol_type = other DNA
catttagagtgtggttggca

SEQ ID NO: 509 - DNA, 20 bp, synthetic construct
  source 1..20: mol_type = other DNA
ccatttagagtgtggttggc

SEQ ID NO: 510 - DNA, 20 bp, synthetic construct
  source 1..20: mol_type = other DNA
tttctccatttagagtgtgg

SEQ ID NO: 511 - DNA, 20 bp, synthetic construct
  source 1..20: mol_type = other DNA
ggatttctccatttagagtg

SEQ ID NO: 512 - DNA, 20 bp, synthetic construct
  source 1..20: mol_type = other DNA
cgccaccgcctgcgcctccg

SEQ ID NO: 513 - DNA, 20 bp, synthetic construct
  source 1..20: mol_type = other DNA
actcgccaccgcctgcgcct

SEQ ID NO: 514 - DNA, 20 bp, synthetic construct
  source 1..20: mol_type = other DNA
tccactcgccaccgcctgcg

SEQ ID NO: 515 - DNA, 20 bp, synthetic construct
  source 1..20: mol_type = other DNA
atatccactcgccaccgcct

SEQ ID NO: 516 - DNA, 20 bp, synthetic construct
  source 1..20: mol_type = other DNA
gagatatccactcgccaccg

SEQ ID NO: 517 - DNA, 20 bp, synthetic construct
  source 1..20: mol_type = other DNA
ttcgaaggatttctccattt

SEQ ID NO: 518 - DNA, 20 bp, synthetic construct
  source 1..20: mol_type = other DNA
catttcgaaggatttctcca

SEQ ID NO: 519 - DNA, 20 bp, synthetic construct
  source 1..20: mol_type = other DNA
ctgcatttcgaaggatttct

SEQ ID NO: 520 - DNA, 20 bp, synthetic construct
  source 1..20: mol_type = other DNA
tctctgcatttcgaaggatt

SEQ ID NO: 521 - DNA, 20 bp, synthetic construct
  source 1..20: mol_type = other DNA
cactctctgcatttcgaagg

SEQ ID NO: 522 - DNA, 20 bp, synthetic construct
  source 1..20: mol_type = other DNA
caccactctctgcatttcga

SEQ ID NO: 523 - DNA, 20 bp, synthetic construct
  source 1..20: mol_type = other DNA
agcaccactctctgcatttc

SEQ ID NO: 524 - DNA, 20 bp, synthetic construct
  source 1..20: mol_type = other DNA
tagcaccactctctgcattt

SEQ ID NO: 525 - DNA, 20 bp, synthetic construct
  source 1..20: mol_type = other DNA
ctatagcaccactctctgca

SEQ ID NO: 526 - DNA, 20 bp, synthetic construct
  source 1..20: mol_type = other DNA
catctatagcaccactctct

SEQ ID NO: 527 - DNA, 20 bp, synthetic construct
  source 1..20: mol_type = other DNA
actttacatctatagcacca

SEQ ID NO: 528 - DNA, 20 bp, synthetic construct
  source 1..20: mol_type = other DNA
aaaactttacatctatagca

SEQ ID NO: 529 - DNA, 20 bp, synthetic construct
  source 1..20: mol_type = other DNA
aagacaaaaaactttacatc

SEQ ID NO: 530 - DNA, 20 bp, synthetic construct
  source 1..20: mol_type = other DNA
caagacaaaaaactttacat

SEQ ID NO: 531 - DNA, 20 bp, synthetic construct
  source 1..20: mol_type = other DNA
gacaagacaaaaaactttac

SEQ ID NO: 532 - DNA, 20 bp, synthetic construct
  source 1..20: mol_type = other DNA
tcagacaagacaaaaaactt

SEQ ID NO: 533 - DNA, 20 bp, synthetic construct
  source 1..20: mol_type = other DNA
tttcagacaagacaaaaaac

SEQ ID NO: 534 - DNA, 20 bp, synthetic construct
  source 1..20: mol_type = other DNA
cttttcagacaagacaaaaa

SEQ ID NO: 535 - DNA, 20 bp, synthetic construct
  source 1..20: mol_type = other DNA
tcccttttcagacaagacaa

SEQ ID NO: 536 - DNA, 20 bp, synthetic construct
  source 1..20: mol_type = other DNA
cactcccttttcagacaaga

SEQ ID NO: 537 - DNA, 20 bp, synthetic construct
  source 1..20: mol_type = other DNA
aatcactcccttttcagaca

SEQ ID NO: 538 - DNA, 20 bp, synthetic construct
  source 1..20: mol_type = other DNA
aataatcactcccttttcag

SEQ ID NO: 539 - DNA, 20 bp, synthetic construct
  source 1..20: mol_type = other DNA
acaataatcactcccttttc

SEQ ID NO: 540 - DNA, 20 bp, synthetic construct
  source 1..20: mol_type = other DNA
aacaataatcactccctttt

SEQ ID NO: 541 - DNA, 20 bp, synthetic construct
  source 1..20: mol_type = other DNA
tgaaacaataatcactccct

SEQ ID NO: 542 - DNA, 20 bp, synthetic construct
  source 1..20: mol_type = other DNA
taatgaaacaataatcactc

SEQ ID NO: 543 - DNA, 20 bp, synthetic construct
  source 1..20: mol_type = other DNA
gattaatgaaacaataatca

SEQ ID NO: 544 - DNA, 20 bp, synthetic construct
  source 1..20: mol_type = other DNA
tcaaagattaatgaaacaat

SEQ ID NO: 545 - DNA, 20 bp, synthetic construct
  source 1..20: mol_type = other DNA
ccatcaaagattaatgaaac

SEQ ID NO: 546 - DNA, 20 bp, synthetic construct
  source 1..20: mol_type = other DNA
tttccatcaaagattaatga

SEQ ID NO: 547 - DNA, 20 bp, synthetic construct
  source 1..20: mol_type = other DNA
cagtttccatcaaagattaa

SEQ ID NO: 548 - DNA, 20 bp, synthetic construct
  source 1..20: mol_type = other DNA
ttccagtttccatcaaagat

SEQ ID NO: 549 - DNA, 20 bp, synthetic construct
  source 1..20: mol_type = other DNA
ccattccagtttccatcaaa

SEQ ID NO: 550 - DNA, 20 bp, synthetic construct
  source 1..20: mol_type = other DNA
tccccattccagtttccatc

SEQ ID NO: 551 - DNA, 20 bp, synthetic construct
  source 1..20: mol_type = other DNA
cgatccccattccagtttcc

SEQ ID NO: 552 - DNA, 20 bp, synthetic construct
  source 1..20: mol_type = other DNA
ctgcgatccccattccagtt

SEQ ID NO: 553 - DNA, 20 bp, synthetic construct
  source 1..20: mol_type = other DNA
gtgctgcgatccccattcca

SEQ ID NO: 554 - DNA, 20 bp, synthetic construct
  source 1..20: mol_type = other DNA
tatgtgctgcgatccccatt

SEQ ID NO: 555 - DNA, 20 bp, synthetic construct
  source 1..20: mol_type = other DNA
ggaagtataattgatagtcc

SEQ ID NO: 556 - DNA, 20 bp, synthetic construct
  source 1..20: mol_type = other DNA
tgtggaagtataattgatag

SEQ ID NO: 557 - DNA, 20 bp, synthetic construct
  source 1..20: mol_type = other DNA
gtctgtggaagtataattga

SEQ ID NO: 558 - DNA, 20 bp, synthetic construct
  source 1..20: mol_type = other DNA
tctgtctgtggaagtataat

SEQ ID NO: 559 - DNA, 20 bp, synthetic construct
  source 1..20: mol_type = other DNA
agttctgtctgtggaagtat

SEQ ID NO: 560 - DNA, 20 bp, synthetic construct
  source 1..20: mol_type = other DNA
ctaagttctgtctgtggaag

SEQ ID NO: 561 - DNA, 20 bp, synthetic construct
  source 1..20: mol_type = other DNA
aaactaagttctgtctgtgg

SEQ ID NO: 562 - DNA, 20 bp, synthetic construct
  source 1..20: mol_type = other DNA
tagaaactaagttctgtctg

SEQ ID NO: 563 - DNA, 20 bp, synthetic construct
  source 1..20: mol_type = other DNA
aggtagaaactaagttctgt

SEQ ID NO: 564 - DNA, 20 bp, synthetic construct
  source 1..20: mol_type = other DNA
gggaggtagaaactaagttc

SEQ ID NO: 565 - DNA, 20 bp, synthetic construct
  source 1..20: mol_type = other DNA
agtgggaggtagaaactaag

SEQ ID NO: 566 - DNA, 20 bp, synthetic construct
  source 1..20: mol_type = other DNA
tgaagtgggaggtagaaact

SEQ ID NO: 567 - DNA, 20 bp, synthetic construct
  source 1..20: mol_type = other DNA
ctatgaagtgggaggtagaa

SEQ ID NO: 568 - DNA, 20 bp, synthetic construct
  source 1..20: mol_type = other DNA
actctatgaagtgggaggta

SEQ ID NO: 569 - DNA, 20 bp, synthetic construct
  source 1..20: mol_type = other DNA
acactctatgaagtgggagg

SEQ ID NO: 570 - DNA, 20 bp, synthetic construct
  source 1..20: mol_type = other DNA
cacactctatgaagtgggag

SEQ ID NO: 571 - DNA, 20 bp, synthetic construct
  source 1..20: mol_type = other DNA
acacactctatgaagtggga

SEQ ID NO: 572 - DNA, 20 bp, synthetic construct
  source 1..20: mol_type = other DNA
acacacactctatgaagtgg

SEQ ID NO: 573 - DNA, 20 bp, synthetic construct
  source 1..20: mol_type = other DNA
tcaacacacactctatgaag

SEQ ID NO: 574 - DNA, 20 bp, synthetic construct
  source 1..20: mol_type = other DNA
ctatcaacacacactctatg

SEQ ID NO: 575 - DNA, 20 bp, synthetic construct
  source 1..20: mol_type = other DNA
aatctatcaacacacactct

SEQ ID NO: 576 - DNA, 20 bp, synthetic construct
  source 1..20: mol_type = other DNA
gttaatctatcaacacacac

SEQ ID NO: 577 - DNA, 20 bp, synthetic construct
  source 1..20: mol_type = other DNA
gtgttaatctatcaacacac

SEQ ID NO: 578 - DNA, 20 bp, synthetic construct
  source 1..20: mol_type = other DNA
tgtgttaatctatcaacaca

SEQ ID NO: 579 - DNA, 20 bp, synthetic construct
  source 1..20: mol_type = other DNA
tatgtgttaatctatcaaca

SEQ ID NO: 580 - DNA, 20 bp, synthetic construct
  source 1..20: mol_type = other DNA
atatgtgttaatctatcaac

SEQ ID NO: 581 - DNA, 20 bp, synthetic construct
  source 1..20: mol_type = other DNA
attatatgtgttaatctatc

SEQ ID NO: 582 - DNA, 20 bp, synthetic construct
  source 1..20: mol_type = other DNA
cggattatatgtgttaatct

SEQ ID NO: 583 - DNA, 20 bp, synthetic construct
  source 1..20: mol_type = other DNA
ttccggattatatgtgttaa

SEQ ID NO: 584 - DNA, 20 bp, synthetic construct
  source 1..20: mol_type = other DNA
cctttccggattatatgtgt

SEQ ID NO: 585 - DNA, 20 bp, synthetic construct
  source 1..20: mol_type = other DNA
cttcctttccggattatatg

SEQ ID NO: 586 - DNA, 20 bp, synthetic construct
  source 1..20: mol_type = other DNA
attcttcctttccggattat

SEQ ID NO: 587 - DNA, 20 bp, synthetic construct
  source 1..20: mol_type = other DNA
catattcttcctttccggat

SEQ ID NO: 588 - DNA, 20 bp, synthetic construct
  source 1..20: mol_type = other DNA
atccatattcttcctttccg

SEQ ID NO: 589 - DNA, 20 bp, synthetic construct
  source 1..20: mol_type = other DNA
atgcatccatattcttcctt

SEQ ID NO: 590 - DNA, 20 bp, synthetic construct
  source 1..20: mol_type = other DNA
ttatgcatccatattcttcc

SEQ ID NO: 591 - DNA, 20 bp, synthetic construct
  source 1..20: mol_type = other DNA
tccttatgcatccatattct

SEQ ID NO: 592 - DNA, 20 bp, synthetic construct
  source 1..20: mol_type = other DNA
ctttccttatgcatccatat

SEQ ID NO: 593 - DNA, 20 bp, synthetic construct
  source 1..20: mol_type = other DNA
tgtctttccttatgcatcca

SEQ ID NO: 594 - DNA, 20 bp, synthetic construct
  source 1..20: mol_type = other DNA
aggacctccctcctgtttct

SEQ ID NO: 595 - DNA, 20 bp, synthetic construct
  source 1..20: mol_type = other DNA
agaagtaatgccagacagat

SEQ ID NO: 596 - DNA, 20 bp, synthetic construct
  source 1..20: mol_type = other DNA
ctttgtttctctgaaagcaa

SEQ ID NO: 597 - DNA, 20 bp, synthetic construct
  source 1..20: mol_type = other DNA
gtggttggtccactgctatt

SEQ ID NO: 598 - DNA, 20 bp, synthetic construct
  source 1..20: mol_type = other DNA
ttgagggaagccaagattca

SEQ ID NO: 599 - DNA, 20 bp, synthetic construct
  source 1..20: mol_type = other DNA
agagctgtacaattatttta

SEQ ID NO: 600 - DNA, 20 bp, synthetic construct
  source 1..20: mol_type = other DNA
ggtaatgacactactgctgt

SEQ ID NO: 601 - DNA, 20 bp, synthetic construct
  source 1..20: mol_type = other DNA
gatcctaatcctgtctatgc

SEQ ID NO: 602 - DNA, 20 bp, synthetic construct
  source 1..20: mol_type = other DNA
acttgtgggttgaattgtgt

SEQ ID NO: 603 - DNA, 20 bp, synthetic construct
  source 1..20: mol_type = other DNA
taccttatgcatccatattc

SEQ ID NO: 604 - DNA, 20 bp, synthetic construct
  source 1..20: mol_type = other DNA
gatgttcactgcatataatt

SEQ ID NO: 605 - DNA, 20 bp, synthetic construct
  source 1..20: mol_type = other DNA
ccagatgtatttgtatctaa

SEQ ID NO: 606 - DNA, 20 bp, synthetic construct
  source 1..20: mol_type = other DNA
taatgtggagctaccatttc

SEQ ID NO: 607 - DNA, 20 bp, synthetic construct
  source 1..20: mol_type = other DNA
gctcccaagaagaatccagg

SEQ ID NO: 608 - DNA, 20 bp, synthetic construct
  source 1..20: mol_type = other DNA
acttacacatagtagtaagc

SEQ ID NO: 609 - DNA, 20 bp, synthetic construct
  source 1..20: mol_type = other DNA
aaagagaccaaaggctacat

SEQ ID NO: 610 - DNA, 20 bp, synthetic construct
  source 1..20: mol_type = other DNA
ggaattctcttgggaaccat

SEQ ID NO: 611 - DNA, 20 bp, synthetic construct
  source 1..20: mol_type = other DNA
tcttgtctttccttatgcat

SEQ ID NO: 612 - DNA, 20 bp, synthetic construct
  source 1..20: mol_type = other DNA
ttttcttgtctttccttatg

SEQ ID NO: 613 - DNA, 20 bp, synthetic construct
  source 1..20: mol_type = other DNA
tggacattttcttgtctttc

SEQ ID NO: 614 - DNA, 20 bp, synthetic construct
  source 1..20: mol_type = other DNA
ttctggacattttcttgtct

SEQ ID NO: 615 - DNA, 20 bp, synthetic construct
  source 1..20: mol_type = other DNA
atcttctggacattttcttg

SEQ ID NO: 616 - DNA, 20 bp, synthetic construct
  source 1..20: mol_type = other DNA
taatcttctggacattttct

SEQ ID NO: 617 - DNA, 20 bp, synthetic construct
  source 1..20: mol_type = other DNA
aagataatcttctggacatt

SEQ ID NO: 618 - DNA, 20 bp, synthetic construct
  source 1..20: mol_type = other DNA
tctaagataatcttctggac

SEQ ID NO: 619 - DNA, 20 bp, synthetic construct
  source 1..20: mol_type = other DNA
ccttctaagataatcttctg

SEQ ID NO: 620 - DNA, 20 bp, synthetic construct
  source 1..20: mol_type = other DNA
gtgccttctaagataatctt

SEQ ID NO: 621 - DNA, 20 bp, synthetic construct
  source 1..20: mol_type = other DNA
tctgtgccttctaagataat

SEQ ID NO: 622 - DNA, 20 bp, synthetic construct
  source 1..20: mol_type = other DNA
ctctctgtgccttctaagat

SEQ ID NO: 623 - DNA, 20 bp, synthetic construct
  source 1..20: mol_type = other DNA
attctctctgtgccttctaa

SEQ ID NO: 624 - DNA, 20 bp, synthetic construct
  source 1..20: mol_type = other DNA
tccattctctctgtgccttc

SEQ ID NO: 625 - DNA, 20 bp, synthetic construct
  source 1..20: mol_type = other DNA
tcttccattctctctgtgcc

SEQ ID NO: 626 - DNA, 20 bp, synthetic construct
  source 1..20: mol_type = other DNA
tgatcttccattctctctgt

SEQ ID NO: 627 - DNA, 20 bp, synthetic construct
  source 1..20: mol_type = other DNA
gaccctgatcttccattctc

SEQ ID NO: 628 - DNA, 20 bp, synthetic construct
  source 1..20: mol_type = other DNA
tctgaccctgatcttccatt

SEQ ID NO: 629 - DNA, 20 bp, synthetic construct
  source 1..20: mol_type = other DNA
tactctgaccctgatcttcc

SEQ ID NO: 630 - DNA, 20 bp, synthetic construct
  source 1..20: mol_type = other DNA
taatactctgaccctgatct

SEQ ID NO: 631 - DNA, 20 bp, synthetic construct
  source 1..20: mol_type = other DNA
gaataatactctgaccctga

SEQ ID NO: 632 - DNA, 20 bp, synthetic construct
  source 1..20: mol_type = other DNA
gcattggaataatactctga

SEQ ID NO: 633 - DNA, 20 bp, synthetic construct
  source 1..20: mol_type = other DNA
taagcattggaataatactc

SEQ ID NO: 634 - DNA, 20 bp, synthetic construct
  source 1..20: mol_type = other DNA
cagtaagcattggaataata

SEQ ID NO: 635 - DNA, 20 bp, synthetic construct
  source 1..20: mol_type = other DNA
ctccagtaagcattggaata

SEQ ID NO: 636 - DNA, 20 bp, synthetic construct
  source 1..20: mol_type = other DNA
cttctccagtaagcattgga

SEQ ID NO: 637 - DNA, 20 bp, synthetic construct
  source 1..20: mol_type = other DNA
tcacttctccagtaagcatt

SEQ ID NO: 638 - DNA, 20 bp, synthetic construct
  source 1..20: mol_type = other DNA
gaatcacttctccagtaagc

SEQ ID NO: 639 - DNA, 20 bp, synthetic construct
  source 1..20: mol_type = other DNA
caggaatcacttctccagta

SEQ ID NO: 640 - DNA, 20 bp, synthetic construct
  source 1..20: mol_type = other DNA
ttacaggaatcacttctcca

SEQ ID NO: 641 - DNA, 20 bp, synthetic construct
  source 1..20: mol_type = other DNA
ccattacaggaatcacttct

SEQ ID NO: 642 - DNA, 20 bp, synthetic construct
  source 1..20: mol_type = other DNA
aagcagttccattacaggaa

SEQ ID NO: 643 - DNA, 20 bp, synthetic construct
  source 1..20: mol_type = other DNA
tgaaagcagttccattacag

SEQ ID NO: 644 - DNA, 20 bp, synthetic construct
  source 1..20: mol_type = other DNA
agatgaaagcagttccatta

SEQ ID NO: 645 - DNA, 20 bp, synthetic construct
  source 1..20: mol_type = other DNA
catagatgaaagcagttcca

SEQ ID NO: 646 - DNA, 20 bp, synthetic construct
  source 1..20: mol_type = other DNA
tttcatagatgaaagcagtt

SEQ ID NO: 647 - DNA, 20 bp, synthetic construct
  source 1..20: mol_type = other DNA
gtgtgatttcatagatgaaa

SEQ ID NO: 648 - DNA, 20 bp, synthetic construct
  source 1..20: mol_type = other DNA
cactgtgtgatttcatagat

SEQ ID NO: 649 - DNA, 20 bp, synthetic construct
  source 1..20: mol_type = other DNA
gaacactgtgtgatttcata

SEQ ID NO: 650 - DNA, 20 bp, synthetic construct
  source 1..20: mol_type = other DNA
caggaacactgtgtgatttc

SEQ ID NO: 651 - DNA, 20 bp, synthetic construct
  source 1..20: mol_type = other DNA
tttcttcaggaacactgtgt

SEQ ID NO: 652 - DNA, 20 bp, synthetic construct
  source 1..20: mol_type = other DNA
ctatttcttcaggaacactg

SEQ ID NO: 653 - DNA, 20 bp, synthetic construct
  source 1..20: mol_type = other DNA
tatctatttcttcaggaaca

SEQ ID NO: 654 - DNA, 20 bp, synthetic construct
  source 1..20: mol_type = other DNA
ctatatctatttcttcagga

SEQ ID NO: 655 - DNA, 20 bp, synthetic construct
  source 1..20: mol_type = other DNA
cagctatatctatttcttca

SEQ ID NO: 656 - DNA, 20 bp, synthetic construct
  source 1..20: mol_type = other DNA
tatcagctatatctatttct

SEQ ID NO: 657 - DNA, 20 bp, synthetic construct
  source 1..20: mol_type = other DNA
ctgtatcagctatatctatt

SEQ ID NO: 658 - DNA, 20 bp, synthetic construct
  source 1..20: mol_type = other DNA
gtactgtatcagctatatct

SEQ ID NO: 659 - DNA, 20 bp, synthetic construct
  source 1..20: mol_type = other DNA
tgagtactgtatcagctata

SEQ ID NO: 660 - DNA, 20 bp, synthetic construct
  source 1..20: mol_type = other DNA
cattgagtactgtatcagct

SEQ ID NO: 661 - DNA, 20 bp, synthetic construct
  source 1..20: mol_type = other DNA
catcattgagtactgtatca

SEQ ID NO: 662 - DNA, 20 bp, synthetic construct
  source 1..20: mol_type = other DNA
catcatcattgagtactgta

SEQ ID NO: 663 - DNA, 20 bp, synthetic construct
  source 1..20: mol_type = other DNA
tatcatcatcattgagtact

SEQ ID NO: 664 - DNA, 20 bp, synthetic construct
  source 1..20: mol_type = other DNA
caatatcatcatcattgagt

SEQ ID NO: 665 - DNA, 20 bp, synthetic construct
  source 1..20: mol_type = other DNA
gtcaccaatatcatcatcat

SEQ ID NO: 666 - DNA, 20 bp, synthetic construct
  source 1..20: mol_type = other DNA
ttgagaagaaagccttcatg

SEQ ID NO: 667 - DNA, 20 bp, synthetic construct
  source 1..20: mol_type = other DNA
actatactgaaatgtaaata

SEQ ID NO: 668 - DNA, 20 bp, synthetic construct
  source 1..20: mol_type = other DNA
tatcaaactggaacacagga

SEQ ID NO: 669 - DNA, 20 bp, synthetic construct
  source 1..20: mol_type = other DNA
tgggcaaaagccttttaaaa

SEQ ID NO: 670 - DNA, 20 bp, synthetic construct
  source 1..20: mol_type = other DNA
gcaaacatagtaaaaaatta

SEQ ID NO: 671 - DNA, 20 bp, synthetic construct
  source 1..20: mol_type = other DNA
ttctcctgattttaagagtt

SEQ ID NO: 672 - DNA, 20 bp, synthetic construct
  source 1..20: mol_type = other DNA
aagaatgacttgcacttttc

SEQ ID NO: 673 - DNA, 20 bp, synthetic construct
  source 1..20: mol_type = other DNA
aaagataacttcacagaaaa

SEQ ID NO: 674 - DNA, 20 bp, synthetic construct
  source 1..20: mol_type = other DNA
ctttctactttagggaaaaa

SEQ ID NO: 675 - DNA, 20 bp, synthetic construct
  source 1..20: mol_type = other DNA
tttttcaatagacatgttct

SEQ ID NO: 676 - DNA, 20 bp, synthetic construct
  source 1..20: mol_type = other DNA
cttgtctttcctgagcaaga

SEQ ID NO: 677 - DNA, 20 bp, synthetic construct
  source 1..20: mol_type = other DNA
acctgatcttccattctctc

SEQ ID NO: 678 - DNA, 20 bp, synthetic construct
  source 1..20: mol_type = other DNA
ctccataaaagctccattaa

SEQ ID NO: 679 - DNA, 20 bp, synthetic construct
  source 1..20: mol_type = other DNA
tgtttactgatttaactctt

SEQ ID NO: 680 - DNA, 20 bp, synthetic construct
  source 1..20: mol_type = other DNA
aacagaaaaaaaaagggagc

SEQ ID NO: 681 - DNA, 20 bp, synthetic construct
  source 1..20: mol_type = other DNA
gtaccttaaagaacatatca

SEQ ID NO: 682 - DNA, 20 bp, synthetic construct
  source 1..20: mol_type = other DNA
aaatgtaaattgcatgagtc

SEQ ID NO: 683 - DNA, 20 bp, synthetic construct
  source 1..20: mol_type = other DNA
gggtaagaaatatcactgac

SEQ ID NO: 684 - DNA, 20 bp, synthetic construct
  source 1..20: mol_type = other DNA
aaccatgcttctcaaactct

SEQ ID NO: 685 - DNA, 20 bp, synthetic construct
  source 1..20: mol_type = other DNA
aagaacttctctgctttaca

SEQ ID NO: 686 - DNA, 20 bp, synthetic construct
  source 1..20: mol_type = other DNA
aatggaagtaaaagtgaaga

SEQ ID NO: 687 - DNA, 20 bp, synthetic construct
  source 1..20: mol_type = other DNA
aacagccatgtttaaaatat

SEQ ID NO: 688 - DNA, 20 bp, synthetic construct
  source 1..20: mol_type = other DNA
ttaaagtatcatctgtctca

SEQ ID NO: 689 - DNA, 20 bp, synthetic construct
  source 1..20: mol_type = other DNA
caatttggtaaaggagatca

SEQ ID NO: 690 - DNA, 20 bp, synthetic construct
  source 1..20: mol_type = other DNA
acacagaataactgtctctg

SEQ ID NO: 691 - DNA, 20 bp, synthetic construct
  source 1..20: mol_type = other DNA
gcttattgaccagcaaataa

SEQ ID NO: 692 - DNA, 20 bp, synthetic construct
  source 1..20: mol_type = other DNA
cccagtaaaagcagaatttt

SEQ ID NO: 693 - DNA, 20 bp, synthetic construct
  source 1..20: mol_type = other DNA
attaatagtagtcaacttaa

SEQ ID NO: 694 - DNA, 20 bp, synthetic construct
  source 1..20: mol_type = other DNA
acttgaacttctcagcagta

SEQ ID NO: 695 - DNA, 20 bp, synthetic construct
  source 1..20: mol_type = other DNA
agaagaggctctaaaagaaa

SEQ ID NO: 696 - DNA, 20 bp, synthetic construct
  source 1..20: mol_type = other DNA
aaaggcaactcctccttttc

SEQ ID NO: 697 - DNA, 20 bp, synthetic construct
  source 1..20: mol_type = other DNA
acagtattgttcaaaataaa

SEQ ID NO: 698 - DNA, 20 bp, synthetic construct
  source 1..20: mol_type = other DNA
cagatgacagctacaactga

SEQ ID NO: 699 - DNA, 20 bp, synthetic construct
  source 1..20: mol_type = other DNA
gaataatgactagatccgtg

SEQ ID NO: 700 - DNA, 20 bp, synthetic construct
  source 1..20: mol_type = other DNA
ataattatcatgcctgttta

SEQ ID NO: 701 - DNA, 20 bp, synthetic construct
  source 1..20: mol_type = other DNA
ctttagtaacctccacaact

SEQ ID NO: 702 - DNA, 20 bp, synthetic construct
  source 1..20: mol_type = other DNA
gaatttaaatgtgatgctac

SEQ ID NO: 703 - DNA, 20 bp, synthetic construct
  source 1..20: mol_type = other DNA
tgtcagacccagggccattt

SEQ ID NO: 704 - DNA, 20 bp, synthetic construct
  source 1..20: mol_type = other DNA
acttattttatgaaatgatt

SEQ ID NO: 705 - DNA, 20 bp, synthetic construct
  source 1..20: mol_type = other DNA
ttttagctaaacatattttt

SEQ ID NO: 706 - DNA, 20 bp, synthetic construct
  source 1..20: mol_type = other DNA
cagtctcatcagttttgtga

SEQ ID NO: 707 - DNA, 20 bp, synthetic construct
  source 1..20: mol_type = other DNA
tgtaaagtgtctcaaatatg

SEQ ID NO: 708 - DNA, 20 bp, synthetic construct
  source 1..20: mol_type = other DNA
cttgaaattgtaattttgaa

SEQ ID NO: 709 - DNA, 20 bp, synthetic construct
  source 1..20: mol_type = other DNA
aatcaaaatcagcacatata

SEQ ID NO: 710 - DNA, 20 bp, synthetic construct
  source 1..20: mol_type = other DNA
accaaataggtaaggaaaac

SEQ ID NO: 711 - DNA, 20 bp, synthetic construct
  source 1..20: mol_type = other DNA
aaagatctcctttaaaattt

SEQ ID NO: 712 - DNA, 20 bp, synthetic construct
  source 1..20: mol_type = other DNA
ctttagagagtatggaatca

SEQ ID NO: 713 - DNA, 20 bp, synthetic construct
  source 1..20: mol_type = other DNA
caaagctcacttttattctt

SEQ ID NO: 714 - DNA, 20 bp, synthetic construct
  source 1..20: mol_type = other DNA
acacagtatcaaacaagtct

SEQ ID NO: 715 - DNA, 20 bp, synthetic construct
  source 1..20: mol_type = other DNA
aagctgggcaataaaaaata

SEQ ID NO: 716 - DNA, 20 bp, synthetic construct
  source 1..20: mol_type = other DNA
ctgaccctgcacaataaagt

SEQ ID NO: 717 - DNA, 20 bp, synthetic construct
  source 1..20: mol_type = other DNA
catctatttcttcaggaaca

SEQ ID NO: 718 - DNA, 20 bp, synthetic construct
  source 1..20: mol_type = other DNA
gaatattaataatatacata

SEQ ID NO: 719 - DNA, 20 bp, synthetic construct
  source 1..20: mol_type = other DNA
aggattttgtgtgtgcttat

SEQ ID NO: 720 - DNA, 20 bp, synthetic construct
  source 1..20: mol_type = other DNA
ttttaggaattataaaagta

SEQ ID NO: 721 - DNA, 20 bp, synthetic construct
  source 1..20: mol_type = other DNA
acacagttttgtttcaaaag

SEQ ID NO: 722 - DNA, 20 bp, synthetic construct
  source 1..20: mol_type = other DNA
ggaaactaaatttgtgacta

SEQ ID NO: 723 - DNA, 20 bp, synthetic construct
  source 1..20: mol_type = other DNA
ctcttaacactcatagtgtg

SEQ ID NO: 724 - DNA, 20 bp, synthetic construct
  source 1..20: mol_type = other DNA
gagactaacctaaatgacaa

SEQ ID NO: 725 - DNA, 20 bp, synthetic construct
  source 1..20: mol_type = other DNA
caaatgtgaaagctggtcaa

SEQ ID NO: 726 - DNA, 20 bp, synthetic construct
  source 1..20: mol_type = other DNA
taacacactgccttcatttc

SEQ ID NO: 727 - DNA, 20 bp, synthetic construct
  source 1..20: mol_type = other DNA
tatctaaaatgcatcaaaaa

SEQ ID NO: 728 - DNA, 20 bp, synthetic construct
  source 1..20: mol_type = other DNA
cttgagaagaaagccttcat

SEQ ID NO: 729 - DNA, 20 bp, synthetic construct
  source 1..20: mol_type = other DNA
ccaaatcttgtcataggtga

SEQ ID NO: 730 - DNA, 20 bp, synthetic construct
  source 1..20: mol_type = other DNA
taacacaaatttaagcaaca

SEQ ID NO: 731 - DNA, 20 bp, synthetic construct
  source 1..20: mol_type = other DNA
aaatagcaaatggaataaca

SEQ ID NO: 732 - DNA, 20 bp, synthetic construct
  source 1..20: mol_type = other DNA
aaaccagaatcaagcaaggg

SEQ ID NO: 733 - DNA, 20 bp, synthetic construct
  source 1..20: mol_type = other DNA
catctacagtacaacttaat

SEQ ID NO: 734 - DNA, 20 bp, synthetic construct
  source 1..20: mol_type = other DNA
agatcagtataaatatgaat

SEQ ID NO: 735 - DNA, 20 bp, synthetic construct
  source 1..20: mol_type = other DNA
gtttaagggcacaaactctt

SEQ ID NO: 736 - DNA, 20 bp, synthetic construct
  source 1..20: mol_type = other DNA
aggtgtatagagaattcagg

SEQ ID NO: 737 - DNA, 20 bp, synthetic construct
  source 1..20: mol_type = other DNA
tactcaatgcttataacaac

SEQ ID NO: 738 - DNA, 20 bp, synthetic construct
  source 1..20: mol_type = other DNA
ggaactaacatgtaggcact

SEQ ID NO: 739 - DNA, 20 bp, synthetic construct
  source 1..20: mol_type = other DNA
cataaaagtgaatactttat

SEQ ID NO: 740 - DNA, 20 bp, synthetic construct
  source 1..20: mol_type = other DNA
aggctcttaggttaaacaca

SEQ ID NO: 741 - DNA, 20 bp, synthetic construct
  source 1..20: mol_type = other DNA
gctgacactgaacagataca

SEQ ID NO: 742 - DNA, 20 bp, synthetic construct
  source 1..20: mol_type = other DNA
catgtagagagattaagtga

SEQ ID NO: 743 - DNA, 20 bp, synthetic construct
  source 1..20: mol_type = other DNA
atcatttaattaatgtattt

SEQ ID NO: 744 - DNA, 18 bp, synthetic construct
  source 1..18: mol_type = other DNA
gtgagagcaagtagtggg

SEQ ID NO: 745 - DNA, 18 bp, synthetic construct
  source 1..18: mol_type = other DNA
tgtgagagcaagtagtgg

SEQ ID NO: 746 - DNA, 18 bp, synthetic construct
  source 1..18: mol_type = other DNA
ctgtgagagcaagtagtg

SEQ ID NO: 747 - DNA, 18 bp, synthetic construct
  source 1..18: mol_type = other DNA
actgtgagagcaagtagt

SEQ ID NO: 748 - DNA, 18 bp, synthetic construct
  source 1..18: mol_type = other DNA
tactgtgagagcaagtag

SEQ ID NO: 749 - DNA, 18 bp, synthetic construct
  source 1..18: mol_type = other DNA
gtactgtgagagcaagta

SEQ ID NO: 750 - DNA, 18 bp, synthetic construct
  source 1..18: mol_type = other DNA
agtactgtgagagcaagt

SEQ ID NO: 751 - DNA, 18 bp, synthetic construct
  source 1..18: mol_type = other DNA
gagtactgtgagagcaag

SEQ ID NO: 752 - DNA, 18 bp, synthetic construct
  source 1..18: mol_type = other DNA
cgagtactgtgagagcaa

SEQ ID NO: 753 - DNA, 18 bp, synthetic construct
  source 1..18: mol_type = other DNA
gcgagtactgtgagagca

SEQ ID NO: 754 - DNA, 18 bp, synthetic construct
  source 1..18: mol_type = other DNA
agcgagtactgtgagagc

SEQ ID NO: 755 - DNA, 18 bp, synthetic construct
  source 1..18: mol_type = other DNA
cagcgagtactgtgagag

SEQ ID NO: 756 - DNA, 18 bp, synthetic construct
  source 1..18: mol_type = other DNA
tcagcgagtactgtgaga

SEQ ID NO: 757 - DNA, 18 bp, synthetic construct
  source 1..18: mol_type = other DNA
ctcagcgagtactgtgag

SEQ ID NO: 758 - DNA, 18 bp, synthetic construct
  source 1..18: mol_type = other DNA
cctcagcgagtactgtga

SEQ ID NO: 759 - DNA, 18 bp, synthetic construct
  source 1..18: mol_type = other DNA
ccctcagcgagtactgtg

SEQ ID NO: 760 - DNA, 18 bp, synthetic construct
  source 1..18: mol_type = other DNA
accctcagcgagtactgt

SEQ ID NO: 761 - DNA, 18 bp, synthetic construct
  source 1..18: mol_type = other DNA
caccctcagcgagtactg

SEQ ID NO: 762 - DNA, 18 bp, synthetic construct
  source 1..18: mol_type = other DNA
tcaccctcagcgagtact

SEQ ID NO: 763 - DNA, 18 bp, synthetic construct
  source 1..18: mol_type = other DNA
ttcaccctcagcgagtac

SEQ ID NO: 764 - DNA, 18 bp, synthetic construct
  source 1..18: mol_type = other DNA
gttcaccctcagcgagta

SEQ ID NO: 765 - DNA, 18 bp, synthetic construct
  source 1..18: mol_type = other DNA
tgttcaccctcagcgagt

SEQ ID NO: 766 - DNA, 18 bp, synthetic construct
  source 1..18: mol_type = other DNA
ttgttcaccctcagcgag

SEQ ID NO: 767 - DNA, 18 bp, synthetic construct
  source 1..18: mol_type = other DNA
cttgttcaccctcagcga

SEQ ID NO: 768 - DNA, 18 bp, synthetic construct
  source 1..18: mol_type = other DNA
tcttgttcaccctcagcg

SEQ ID NO: 769 - DNA, 18 bp, synthetic construct
  source 1..18: mol_type = other DNA
ttcttgttcaccctcagc

SEQ ID NO: 770 - DNA, 18 bp, synthetic construct
  source 1..18: mol_type = other DNA
tttcttgttcaccctcag

SEQ ID NO: 771 - DNA, 18 bp, synthetic construct
  source 1..18: mol_type = other DNA
ttttcttgttcaccctca

SEQ ID NO: 772 - DNA, 18 bp, synthetic construct
  source 1..18: mol_type = other DNA
cttttcttgttcaccctc

SEQ ID NO: 773 - DNA, 18 bp, synthetic construct
  source 1..18: mol_type = other DNA
tcttttcttgttcaccct

SEQ ID NO: 774 - DNA, 18 bp, synthetic construct
  source 1..18: mol_type = other DNA
gtcttttcttgttcaccc

SEQ ID NO: 775 - DNA, 18 bp, synthetic construct
  source 1..18: mol_type = other DNA
ggtcttttcttgttcacc

SEQ ID NO: 776 - DNA, 18 bp, synthetic construct
  source 1..18: mol_type = other DNA
aggtcttttcttgttcac

SEQ ID NO: 777 - DNA, 18 bp, synthetic construct
  source 1..18: mol_type = other DNA
caggtcttttcttgttca

SEQ ID NO: 778 - DNA, 18 bp, synthetic construct
  source 1..18: mol_type = other DNA
tcaggtcttttcttgttc

SEQ ID NO: 779 - DNA, 18 bp, synthetic construct
  source 1..18: mol_type = other DNA
atcaggtcttttcttgtt

SEQ ID NO: 780 - DNA, 18 bp, synthetic construct
  source 1..18: mol_type = other DNA
tatcaggtcttttcttgt

SEQ ID NO: 781 - DNA, 18 bp, synthetic construct
  source 1..18: mol_type = other DNA
ttatcaggtcttttcttg

SEQ ID NO: 782 - DNA, 18 bp, synthetic construct
  source 1..18: mol_type = other DNA
tttatcaggtcttttctt

SEQ ID NO: 783 - DNA, 18 bp, synthetic construct
  source 1..18: mol_type = other DNA
aatctttatcaggtcttt

SEQ ID NO: 784 - DNA, 18 bp, synthetic construct
  source 1..18: mol_type = other DNA
taatctttatcaggtctt

SEQ ID NO: 785 - DNA, 18 bp, synthetic construct
  source 1..18: mol_type = other DNA
ttaatctttatcaggtct

SEQ ID NO: 786 - DNA, 18 bp, synthetic construct
  source 1..18: mol_type = other DNA
gttaatctttatcaggtc

SEQ ID NO: 787 - DNA, 18 bp, synthetic construct
  source 1..18: mol_type = other DNA
ggttaatctttatcaggt

SEQ ID NO: 788 - DNA, 18 bp, synthetic construct
  source 1..18: mol_type = other DNA
tggttaatctttatcagg

SEQ ID NO: 789 - DNA, 18 bp, synthetic construct
  source 1..18: mol_type = other DNA
ctggttaatctttatcag

SEQ ID NO: 790 - DNA, 18 bp, synthetic construct
  source 1..18: mol_type = other DNA
tctggttaatctttatca

SEQ ID NO: 791 - DNA, 18 bp, synthetic construct
  source 1..18: mol_type = other DNA
ttctggttaatctttatc

SEQ ID NO: 792 - DNA, 18 bp, synthetic construct
  source 1..18: mol_type = other DNA
tccctccttgttttcttc

SEQ ID NO: 793 - DNA, 18 bp, synthetic construct
  source 1..18: mol_type = other DNA
tttccctccttgttttct

SEQ ID NO: 794 - DNA, 18 bp, synthetic construct
  source 1..18: mol_type = other DNA
gtttccctccttgttttc

SEQ ID NO: 795 - DNA, 18 bp, synthetic construct
  source 1..18: mol_type = other DNA
tgtttccctccttgtttt

SEQ ID NO: 796 - DNA, 18 bp, synthetic construct
  source 1..18: mol_type = other DNA
ttgtttccctccttgttt

SEQ ID NO: 797 - DNA, 18 bp, synthetic construct
  source 1..18: mol_type = other DNA
gttgtttccctccttgtt

SEQ ID NO: 798 - DNA, 18 bp, synthetic construct
  source 1..18: mol_type = other DNA
ggttgtttccctccttgt

SEQ ID NO: 799 - DNA, 18 bp, synthetic construct
  source 1..18: mol_type = other DNA
cggttgtttccctccttg

SEQ ID NO: 800 - DNA, 18 bp, synthetic construct
  source 1..18: mol_type = other DNA
gcggttgtttccctcctt

SEQ ID NO: 801 - DNA, 18 bp, synthetic construct
  source 1..18: mol_type = other DNA
tgcggttgtttccctcct

SEQ ID NO: 802 - DNA, 18 bp, synthetic construct
  source 1..18: mol_type = other DNA
ctgcggttgtttccctcc

SEQ ID NO: 803 - DNA, 18 bp, synthetic construct
  source 1..18: mol_type = other DNA
gctgcggttgtttccctc

SEQ ID NO: 804 - DNA, 18 bp, synthetic construct
  source 1..18: mol_type = other DNA
ggctgcggttgtttccct

SEQ ID NO: 805 - DNA, 18 bp, synthetic construct
  source 1..18: mol_type = other DNA
aggctgcggttgtttccc

SEQ ID NO: 806 - DNA, 18 bp, synthetic construct
  source 1..18: mol_type = other DNA
caggctgcggttgtttcc

SEQ ID NO: 807 - DNA, 18 bp, synthetic construct
  source 1..18: mol_type = other DNA
acaggctgcggttgtttc

SEQ ID NO: 808 - DNA, 18 bp, synthetic construct
  source 1..18: mol_type = other DNA
tacaggctgcggttgttt

SEQ ID NO: 809 - DNA, 18 bp, synthetic construct
  source 1..18: mol_type = other DNA
ctacaggctgcggttgtt

SEQ ID NO: 810 - DNA, 18 bp, synthetic construct
  source 1..18: mol_type = other DNA
gctacaggctgcggttgt

SEQ ID NO: 811 - DNA, 18 bp, synthetic construct
  source 1..18: mol_type = other DNA
tgctacaggctgcggttg

SEQ ID NO: 812 - DNA, 18 bp, synthetic construct
  source 1..18: mol_type = other DNA
ttgctacaggctgcggtt

SEQ ID NO: 813 - DNA, 18 bp, synthetic construct
  source 1..18: mol_type = other DNA
cttgctacaggctgcggt

SEQ ID NO: 814 - DNA, 18 bp, synthetic construct
  source 1..18: mol_type = other DNA
gcttgctacaggctgcgg

SEQ ID NO: 815 - DNA, 18 bp, synthetic construct
  source 1..18: mol_type = other DNA
agcttgctacaggctgcg

SEQ ID NO: 816 - DNA, 18 bp, synthetic construct
  source 1..18: mol_type = other DNA
gagcttgctacaggctgc

SEQ ID NO: 817 - DNA, 18 bp, synthetic construct
  source 1..18: mol_type = other DNA
agagcttgctacaggctg

SEQ ID NO: 818 - DNA, 18 bp, synthetic construct
  source 1..18: mol_type = other DNA
cagagcttgctacaggct

SEQ ID NO: 819 - DNA, 18 bp, synthetic construct
  source 1..18: mol_type = other DNA
ccagagcttgctacaggc

SEQ ID NO: 820 - DNA, 18 bp, synthetic construct
  source 1..18: mol_type = other DNA
tccagagcttgctacagg

SEQ ID NO: 821 - DNA, 18 bp, synthetic construct
  source 1..18: mol_type = other DNA
ttccagagcttgctacag

SEQ ID NO: 822 - DNA, 18 bp, synthetic construct
  source 1..18: mol_type = other DNA
gttccagagcttgctaca

SEQ ID NO: 823 - DNA, 18 bp, synthetic construct
  source 1..18: mol_type = other DNA
agttccagagcttgctac

SEQ ID NO: 824 - DNA, 18 bp, synthetic construct
  source 1..18: mol_type = other DNA
gagttccagagcttgcta

SEQ ID NO: 825 - DNA, 18 bp, synthetic construct
  source 1..18: mol_type = other DNA
tgagttccagagcttgct

SEQ ID NO: 826 - DNA, 18 bp, synthetic construct
  source 1..18: mol_type = other DNA
ctgagttccagagcttgc

SEQ ID NO: 827 - DNA, 18 bp, synthetic construct
  source 1..18: mol_type = other DNA
cctgagttccagagcttg

SEQ ID NO: 828 - DNA, 18 bp, synthetic construct
  source 1..18: mol_type = other DNA
tcctgagttccagagctt

SEQ ID NO: 829 - DNA, 18 bp, synthetic construct
  source 1..18: mol_type = other DNA
ctcctgagttccagagct

SEQ ID NO: 830 - DNA, 18 bp, synthetic construct
  source 1..18: mol_type = other DNA
actcctgagttccagagc

SEQ ID NO: 831 - DNA, 18 bp, synthetic construct
  source 1..18: mol_type = other DNA
gactcctgagttccagag

SEQ ID NO: 832 - DNA, 18 bp, synthetic construct
  source 1..18: mol_type = other DNA
cgactcctgagttccaga

SEQ ID NO: 833 - DNA, 18 bp, synthetic construct
  source 1..18: mol_type = other DNA
gcgactcctgagttccag

SEQ ID NO: 834 - DNA, 18 bp, synthetic construct
  source 1..18: mol_type = other DNA
cgcgactcctgagttcca

SEQ ID NO: 835 - DNA, 18 bp, synthetic construct
  source 1..18: mol_type = other DNA
gcgcgactcctgagttcc

SEQ ID NO: 836 - DNA, 18 bp, synthetic construct
  source 1..18: mol_type = other DNA
cgcgcgactcctgagttc

SEQ ID NO: 837 - DNA, 18 bp, synthetic construct
  source 1..18: mol_type = other DNA
gcgcgcgactcctgagtt

SEQ ID NO: 838 - DNA, 18 bp, synthetic construct
  source 1..18: mol_type = other DNA
agcgcgcgactcctgagt

SEQ ID NO: 839 - DNA, 18 bp, synthetic construct
  source 1..18: mol_type = other DNA
tagcgcgcgactcctgag

SEQ ID NO: 840 - DNA, 18 bp, synthetic construct
  source 1..18: mol_type = other DNA
ctagcgcgcgactcctga

SEQ ID NO: 841 - DNA, 18 bp, synthetic construct
  source 1..18: mol_type = other DNA
cctagcgcgcgactcctg

SEQ ID NO: 842 - DNA, 18 bp, synthetic construct
  source 1..18: mol_type = other DNA
ccctagcgcgcgactcct

SEQ ID NO: 843 - DNA, 18 bp, synthetic construct
  source 1..18: mol_type = other DNA
cccctagcgcgcgactcc

SEQ ID NO: 844 - DNA, 18 bp, synthetic construct
  source 1..18: mol_type = other DNA
gcccctagcgcgcgactc

SEQ ID NO: 845 - DNA, 18 bp, synthetic construct
  source 1..18: mol_type = other DNA
ggcccctagcgcgcgact

SEQ ID NO: 846 - DNA, 18 bp, synthetic construct
  source 1..18: mol_type = other DNA
cggcccctagcgcgcgac

SEQ ID NO: 847 - DNA, 18 bp, synthetic construct
  source 1..18: mol_type = other DNA
ccggcccctagcgcgcga

SEQ ID NO: 848 - DNA, 18 bp, synthetic construct
  source 1..18: mol_type = other DNA
cccggcccctagcgcgcg

SEQ ID NO: 849 - DNA, 18 bp, synthetic construct
  source 1..18: mol_type = other DNA
ccccggcccctagcgcgc

SEQ ID NO: 850 - DNA, 18 bp, synthetic construct
  source 1..18: mol_type = other DNA
gccccggcccctagcgcg

SEQ ID NO: 851 - DNA, 18 bp, synthetic construct
  source 1..18: mol_type = other DNA
ggccccggcccctagcgc

SEQ ID NO: 852 - DNA, 18 bp, synthetic construct
  source 1..18: mol_type = other DNA
cggccccggcccctagcg

SEQ ID NO: 853 - DNA, 18 bp, synthetic construct
  source 1..18: mol_type = other DNA
ccggccccggcccctagc

SEQ ID NO: 854 - DNA, 18 bp, synthetic construct
  source 1..18: mol_type = other DNA
cccggccccggcccctag

SEQ ID NO: 855 - DNA, 18 bp, synthetic construct
  source 1..18: mol_type = other DNA
ccccggccccggccccta

SEQ ID NO: 856 - DNA, 18 bp, synthetic construct
  source 1..18: mol_type = other DNA
acgccccggccccggccc

SEQ ID NO: 857 - DNA, 18 bp, synthetic construct
  source 1..18: mol_type = other DNA
cacgccccggccccggcc

SEQ ID NO: 858 - DNA, 18 bp, synthetic construct
  source 1..18: mol_type = other DNA
ccacgccccggccccggc

SEQ ID NO: 859 - DNA, 18 bp, synthetic construct
  source 1..18: mol_type = other DNA
accacgccccggccccgg

SEQ ID NO: 860 - DNA, 18 bp, synthetic construct
  source 1..18: mol_type = other DNA
gaccacgccccggccccg

SEQ ID NO: 861 - DNA, 18 bp, synthetic construct
  source 1..18: mol_type = other DNA
cgaccacgccccggcccc

SEQ ID NO: 862 - DNA, 18 bp, synthetic construct
  source 1..18: mol_type = other DNA
ccgaccacgccccggccc

SEQ ID NO: 863 - DNA, 18 bp, synthetic construct
  source 1..18: mol_type = other DNA
cccgaccacgccccggcc

SEQ ID NO: 864 - DNA, 18 bp, synthetic construct
  source 1..18: mol_type = other DNA
ccccgaccacgccccggc

SEQ ID NO: 865 - DNA, 18 bp, synthetic construct
  source 1..18: mol_type = other DNA
gccccgaccacgccccgg

SEQ ID NO: 866 - DNA, 18 bp, synthetic construct
  source 1..18: mol_type = other DNA
cgccccgaccacgccccg

SEQ ID NO: 867 - DNA, 18 bp, synthetic construct
  source 1..18: mol_type = other DNA
ccgccccgaccacgcccc

SEQ ID NO: 868 - DNA, 18 bp, synthetic construct
  source 1..18: mol_type = other DNA
cccgccccgaccacgccc

SEQ ID NO: 869 - DNA, 18 bp, synthetic construct
  source 1..18: mol_type = other DNA
gcccgccccgaccacgcc

SEQ ID NO: 870 - DNA, 18 bp, synthetic construct
  source 1..18: mol_type = other DNA
ggcccgccccgaccacgc

SEQ ID NO: 871 - DNA, 18 bp, synthetic construct
  source 1..18: mol_type = other DNA
gggcccgccccgaccacg

SEQ ID NO: 872 - DNA, 18 bp, synthetic construct
  source 1..18: mol_type = other DNA
cgggcccgccccgaccac

SEQ ID NO: 873 - DNA, 18 bp, synthetic construct
  source 1..18: mol_type = other DNA
ccgggcccgccccgacca

SEQ ID NO: 874 - DNA, 18 bp, synthetic construct
  source 1..18: mol_type = other DNA
cccgggcccgccccgacc

SEQ ID NO: 875 - DNA, 18 bp, synthetic construct
  source 1..18: mol_type = other DNA
ccccgggcccgccccgac

SEQ ID NO: 876 - DNA, 18 bp, synthetic construct
  source 1..18: mol_type = other DNA
agccccgccccgggcccg

SEQ ID NO: 877 - DNA, 18 bp, synthetic construct
  source 1..18: mol_type = other DNA
cagccccgccccgggccc

SEQ ID NO: 878 - DNA, 18 bp, synthetic construct
  source 1..18: mol_type = other DNA
gcagccccgccccgggcc

SEQ ID NO: 879 - DNA, 18 bp, synthetic construct
  source 1..18: mol_type = other DNA
cgcagccccgccccgggc

SEQ ID NO: 880 - DNA, 18 bp, synthetic construct
  source 1..18: mol_type = other DNA
ccgcagccccgccccggg

SEQ ID NO: 881 - DNA, 18 bp, synthetic construct
  source 1..18: mol_type = other DNA
accgcagccccgccccgg

SEQ ID NO: 882 - DNA, 18 bp, synthetic construct
  source 1..18: mol_type = other DNA
aaccgcagccccgccccg

SEQ ID NO: 883 - DNA, 18 bp, synthetic construct
  source 1..18: mol_type = other DNA
caaccgcagccccgcccc

SEQ ID NO: 884 - DNA, 18 bp, synthetic construct
  source 1..18: mol_type = other DNA
gcaaccgcagccccgccc

SEQ ID NO: 885 - DNA, 18 bp, synthetic construct
  source 1..18: mol_type = other DNA
cgcaaccgcagccccgcc

SEQ ID NO: 886 - DNA, 18 bp, synthetic construct
  source 1..18: mol_type = other DNA
ccgcaaccgcagccccgc

SEQ ID NO: 887 - DNA, 18 bp, synthetic construct
  source 1..18: mol_type = other DNA
accgcaaccgcagccccg

SEQ ID NO: 888 - DNA, 18 bp, synthetic construct
  source 1..18: mol_type = other DNA
caccgcaaccgcagcccc

SEQ ID NO: 889 - DNA, 18 bp, synthetic construct
  source 1..18: mol_type = other DNA
gcaccgcaaccgcagccc

SEQ ID NO: 890 - DNA, 18 bp, synthetic construct
  source 1..18: mol_type = other DNA
ggcaccgcaaccgcagcc

SEQ ID NO: 891 - DNA, 18 bp, synthetic construct
  source 1..18: mol_type = other DNA
aggcaccgcaaccgcagc

SEQ ID NO: 892 - DNA, 18 bp, synthetic construct
  source 1..18: mol_type = other DNA
caggcaccgcaaccgcag

SEQ ID NO: 893 - DNA, 18 bp, synthetic construct
  source 1..18: mol_type = other DNA
gcaggcaccgcaaccgca

SEQ ID NO: 894 - DNA, 18 bp, synthetic construct
  source 1..18: mol_type = other DNA
cgcaggcaccgcaaccgc

SEQ ID NO: 895 - DNA, 18 bp, synthetic construct
  source 1..18: mol_type = other DNA
gcgcaggcaccgcaaccg

SEQ ID NO: 896 - DNA, 18 bp, synthetic construct
  source 1..18: mol_type = other DNA
ggcgcaggcaccgcaacc

SEQ ID NO: 897 - DNA, 18 bp, synthetic construct
  source 1..18: mol_type = other DNA
gggcgcaggcaccgcaac

SEQ ID NO: 898 - DNA, 17 bp, synthetic construct
  source 1..17: mol_type = other DNA
tgagagcaagtagtggg

SEQ ID NO: 899 - DNA, 17 bp, synthetic construct
  source 1..17: mol_type = other DNA
gtgagagcaagtagtgg

SEQ ID NO: 900 - DNA, 17 bp, synthetic construct
  source 1..17: mol_type = other DNA
tgtgagagcaagtagtg

SEQ ID NO: 901 - DNA, 17 bp, synthetic construct
  source 1..17: mol_type = other DNA
ctgtgagagcaagtagt

SEQ ID NO: 902 - DNA, 17 bp, synthetic construct
  source 1..17: mol_type = other DNA
actgtgagagcaagtag

SEQ ID NO: 903 - DNA, 17 bp, synthetic construct
  source 1..17: mol_type = other DNA
tactgtgagagcaagta

SEQ ID NO: 904 - DNA, 17 bp, synthetic construct
  source 1..17: mol_type = other DNA
gtactgtgagagcaagt

SEQ ID NO: 905 - DNA, 17 bp, synthetic construct
  source 1..17: mol_type = other DNA
agtactgtgagagcaag

SEQ ID NO: 906 - DNA, 17 bp, synthetic construct
  source 1..17: mol_type = other DNA
gagtactgtgagagcaa

SEQ ID NO: 907 - DNA, 17 bp, synthetic construct
  source 1..17: mol_type = other DNA
cgagtactgtgagagca

SEQ ID NO: 908 - DNA, 17 bp, synthetic construct
  source 1..17: mol_type = other DNA
gcgagtactgtgagagc

SEQ ID NO: 909 - DNA, 17 bp, synthetic construct
  source 1..17: mol_type = other DNA
agcgagtactgtgagag

SEQ ID NO: 910 - DNA, 17 bp, synthetic construct
  source 1..17: mol_type = other DNA
cagcgagtactgtgaga

SEQ ID NO: 911 - DNA, 17 bp, synthetic construct
  source 1..17: mol_type = other DNA
tcagcgagtactgtgag

SEQ ID NO: 912 - DNA, 17 bp, synthetic construct
  source 1..17: mol_type = other DNA
ctcagcgagtactgtga

SEQ ID NO: 913 - DNA, 17 bp, synthetic construct
  source 1..17: mol_type = other DNA
cctcagcgagtactgtg

SEQ ID NO: 914 - DNA, 17 bp, synthetic construct
  source 1..17: mol_type = other DNA
ccctcagcgagtactgt

SEQ ID NO: 915 - DNA, 17 bp, synthetic construct
  source 1..17: mol_type = other DNA
accctcagcgagtactg

SEQ ID NO: 916 - DNA, 17 bp, synthetic construct
  source 1..17: mol_type = other DNA
caccctcagcgagtact

SEQ ID NO: 917 - DNA, 17 bp, synthetic construct
  source 1..17: mol_type = other DNA
tcaccctcagcgagtac

SEQ ID NO: 918 - DNA, 17 bp, synthetic construct
  source 1..17: mol_type = other DNA
ttcaccctcagcgagta

SEQ ID NO: 919 - DNA, 17 bp, synthetic construct
  source 1..17: mol_type = other DNA
gttcaccctcagcgagt

SEQ ID NO: 920 - DNA, 17 bp, synthetic construct
  source 1..17: mol_type = other DNA
tgttcaccctcagcgag

SEQ ID NO: 921 - DNA, 17 bp, synthetic construct
  source 1..17: mol_type = other DNA
ttgttcaccctcagcga

SEQ ID NO: 922 - DNA, 17 bp, synthetic construct
  source 1..17: mol_type = other DNA
cttgttcaccctcagcg

SEQ ID NO: 923 - DNA, 17 bp, synthetic construct
  source 1..17: mol_type = other DNA
tcttgttcaccctcagc

SEQ ID NO: 924 - DNA, 17 bp, synthetic construct
  source 1..17: mol_type = other DNA
ttcttgttcaccctcag

SEQ ID NO: 925 - DNA, 17 bp, synthetic construct
  source 1..17: mol_type = other DNA
tttcttgttcaccctca

SEQ ID NO: 926 - DNA, 17 bp, synthetic construct
  source 1..17: mol_type = other DNA
ttttcttgttcaccctc

SEQ ID NO: 927 - DNA, 17 bp, synthetic construct
  source 1..17: mol_type = other DNA
cttttcttgttcaccct

SEQ ID NO: 928 - DNA, 17 bp, synthetic construct
  source 1..17: mol_type = other DNA
tcttttcttgttcaccc

SEQ ID NO: 929 - DNA, 17 bp, synthetic construct
  source 1..17: mol_type = other DNA
gtcttttcttgttcacc

SEQ ID NO: 930 - DNA, 17 bp, synthetic construct
  source 1..17: mol_type = other DNA
ggtcttttcttgttcac

SEQ ID NO: 931 - DNA, 17 bp, synthetic construct
  source 1..17: mol_type = other DNA
aggtcttttcttgttca

SEQ ID NO: 932 - DNA, 17 bp, synthetic construct
  source 1..17: mol_type = other DNA
caggtcttttcttgttc

SEQ ID NO: 933 - DNA, 17 bp, synthetic construct
  source 1..17: mol_type = other DNA
tcaggtcttttcttgtt

SEQ ID NO: 934 - DNA, 17 bp, synthetic construct
  source 1..17: mol_type = other DNA
atcaggtcttttcttgt

SEQ ID NO: 935 - DNA, 17 bp, synthetic construct
  source 1..17: mol_type = other DNA
tatcaggtcttttcttg

SEQ ID NO: 936 - DNA, 17 bp, synthetic construct
  source 1..17: mol_type = other DNA
ttatcaggtcttttctt

SEQ ID NO: 937 - DNA, 17 bp, synthetic construct
  source 1..17: mol_type = other DNA
atctttatcaggtcttt

SEQ ID NO: 938 - DNA, 17 bp, synthetic construct
  source 1..17: mol_type = other DNA
aatctttatcaggtctt

SEQ ID NO: 939 - DNA, 17 bp, synthetic construct
  source 1..17: mol_type = other DNA
taatctttatcaggtct

SEQ ID NO: 940 - DNA, 17 bp, synthetic construct
  source 1..17: mol_type = other DNA
ttaatctttatcaggtc

SEQ ID NO: 941 - DNA, 17 bp, synthetic construct
  source 1..17: mol_type = other DNA
gttaatctttatcaggt

SEQ ID NO: 942 - DNA, 17 bp, synthetic construct
  source 1..17: mol_type = other DNA
ggttaatctttatcagg

SEQ ID NO: 943 - DNA, 17 bp, synthetic construct
  source 1..17: mol_type = other DNA
tggttaatctttatcag

SEQ ID NO: 944 - DNA, 17 bp, synthetic construct
  source 1..17: mol_type = other DNA
ctggttaatctttatca

SEQ ID NO: 945 - DNA, 17 bp, synthetic construct
  source 1..17: mol_type = other DNA
tctggttaatctttatc

SEQ ID NO: 946 - DNA, 17 bp, synthetic construct
  source 1..17: mol_type = other DNA
ccctccttgttttcttc

SEQ ID NO: 947 - DNA, 17 bp, synthetic construct
  source 1..17: mol_type = other DNA
tccctccttgttttctt

SEQ ID NO: 948 - DNA, 17 bp, synthetic construct
  source 1..17: mol_type = other DNA
ttccctccttgttttct

SEQ ID NO: 949 - DNA, 17 bp, synthetic construct
  source 1..17: mol_type = other DNA
tttccctccttgttttc

SEQ ID NO: 950 - DNA, 17 bp, synthetic construct
  source 1..17: mol_type = other DNA
gtttccctccttgtttt

SEQ ID NO: 951 - DNA, 17 bp, synthetic construct
  source 1..17: mol_type = other DNA
tgtttccctccttgttt

SEQ ID NO: 952 - DNA, 17 bp, synthetic construct
  source 1..17: mol_type = other DNA
ttgtttccctccttgtt

SEQ ID NO: 953 - DNA, 17 bp, synthetic construct
  source 1..17: mol_type = other DNA
ggttgtttccctccttg

SEQ ID NO: 954 - DNA, 17 bp, synthetic construct
  source 1..17: mol_type = other DNA
cggttgtttccctcctt

SEQ ID NO: 955 - DNA, 17 bp, synthetic construct
  source 1..17: mol_type = other DNA
gcggttgtttccctcct

SEQ ID NO: 956 - DNA, 17 bp, synthetic construct
  source 1..17: mol_type = other DNA
tgcggttgtttccctcc

SEQ ID NO: 957 - DNA, 17 bp, synthetic construct
  source 1..17: mol_type = other DNA
ctgcggttgtttccctc

SEQ ID NO: 958 - DNA, 17 bp, synthetic construct
  source 1..17: mol_type = other DNA
gctgcggttgtttccct

SEQ ID NO: 959 - DNA, 17 bp, synthetic construct
  source 1..17: mol_type = other DNA
ggctgcggttgtttccc

SEQ ID NO: 960 - DNA, 17 bp, synthetic construct
  source 1..17: mol_type = other DNA
aggctgcggttgtttcc

SEQ ID NO: 961 - DNA, 17 bp, synthetic construct
  source 1..17: mol_type = other DNA
caggctgcggttgtttc

SEQ ID NO: 962 - DNA, 17 bp, synthetic construct
  source 1..17: mol_type = other DNA
acaggctgcggttgttt

SEQ ID NO: 963 - DNA, 17 bp, synthetic construct
  source 1..17: mol_type = other DNA
tacaggctgcggttgtt

SEQ ID NO: 964 - DNA, 17 bp, synthetic construct
  source 1..17: mol_type = other DNA
ctacaggctgcggttgt

SEQ ID NO: 965 - DNA, 17 bp, synthetic construct
  source 1..17: mol_type = other DNA
gctacaggctgcggttg

SEQ ID NO: 966 - DNA, 17 bp, synthetic construct
  source 1..17: mol_type = other DNA
tgctacaggctgcggtt

SEQ ID NO: 967 - DNA, 17 bp, synthetic construct
  source 1..17: mol_type = other DNA
ttgctacaggctgcggt

SEQ ID NO: 968 - DNA, 17 bp, synthetic construct
  source 1..17: mol_type = other DNA
cttgctacaggctgcgg

SEQ ID NO: 969 - DNA, 17 bp, synthetic construct
  source 1..17: mol_type = other DNA
gcttgctacaggctgcg

SEQ ID NO: 970 - DNA, 17 bp, synthetic construct
  source 1..17: mol_type = other DNA
agcttgctacaggctgc

SEQ ID NO: 971 - DNA, 17 bp, synthetic construct
  source 1..17: mol_type = other DNA
gagcttgctacaggctg

SEQ ID NO: 972 - DNA, 17 bp, synthetic construct
  source 1..17: mol_type = other DNA
agagcttgctacaggct

SEQ ID NO: 973 - DNA, 17 bp, synthetic construct
  source 1..17: mol_type = other DNA
cagagcttgctacaggc

SEQ ID NO: 974 - DNA, 17 bp, synthetic construct
  source 1..17: mol_type = other DNA
ccagagcttgctacagg

SEQ ID NO: 975 - DNA, 17 bp, synthetic construct
  source 1..17: mol_type = other DNA
tccagagcttgctacag

SEQ ID NO: 976 - DNA, 17 bp, synthetic construct
  source 1..17: mol_type = other DNA
ttccagagcttgctaca

SEQ ID NO: 977 - DNA, 17 bp, synthetic construct
  source 1..17: mol_type = other DNA
gttccagagcttgctac

SEQ ID NO: 978 - DNA, 17 bp, synthetic construct
  source 1..17: mol_type = other DNA
agttccagagcttgcta

SEQ ID NO: 979 - DNA, 17 bp, synthetic construct
  source 1..17: mol_type = other DNA
gagttccagagcttgct

SEQ ID NO: 980 - DNA, 17 bp, synthetic construct
  source 1..17: mol_type = other DNA
tgagttccagagcttgc

SEQ ID NO: 981 - DNA, 17 bp, synthetic construct
  source 1..17: mol_type = other DNA
ctgagttccagagcttg

SEQ ID NO: 982 - DNA, 17 bp, synthetic construct
  source 1..17: mol_type = other DNA
cctgagttccagagctt

SEQ ID NO: 983 - DNA, 17 bp, synthetic construct
  source 1..17: mol_type = other DNA
tcctgagttccagagct

SEQ ID NO: 984 - DNA, 17 bp, synthetic construct
  source 1..17: mol_type = other DNA
ctcctgagttccagagc

SEQ ID NO: 985 - DNA, 17 bp, synthetic construct
  source 1..17: mol_type = other DNA
actcctgagttccagag

SEQ ID NO: 986 - DNA, 17 bp, synthetic construct
  source 1..17: mol_type = other DNA
gactcctgagttccaga

SEQ ID NO: 987 - DNA, 17 bp, synthetic construct
  source 1..17: mol_type = other DNA
cgactcctgagttccag

SEQ ID NO: 988 - DNA, 17 bp, synthetic construct
  source 1..17: mol_type = other DNA
gcgactcctgagttcca

SEQ ID NO: 989 - DNA, 17 bp, synthetic construct
  source 1..17: mol_type = other DNA
cgcgactcctgagttcc

SEQ ID NO: 990 - DNA, 17 bp, synthetic construct
  source 1..17: mol_type = other DNA
gcgcgactcctgagttc

SEQ ID NO: 991 - DNA, 17 bp, synthetic construct
  source 1..17: mol_type = other DNA
cgcgcgactcctgagtt

SEQ ID NO: 992 - DNA, 17 bp, synthetic construct
  source 1..17: mol_type = other DNA
gcgcgcgactcctgagt

SEQ ID NO: 993 - DNA, 17 bp, synthetic construct
  source 1..17: mol_type = other DNA
agcgcgcgactcctgag

SEQ ID NO: 994 - DNA, 17 bp, synthetic construct
  source 1..17: mol_type = other DNA
tagcgcgcgactcctga

SEQ ID NO: 995 - DNA, 17 bp, synthetic construct
  source 1..17: mol_type = other DNA
ctagcgcgcgactcctg

SEQ ID NO: 996 - DNA, 17 bp, synthetic construct
  source 1..17: mol_type = other DNA
cctagcgcgcgactcct

SEQ ID NO: 997 - DNA, 17 bp, synthetic construct
  source 1..17: mol_type = other DNA
ccctagcgcgcgactcc

SEQ ID NO: 998 - DNA, 17 bp, synthetic construct
  source 1..17: mol_type = other DNA
cccctagcgcgcgactc

SEQ ID NO: 999 - DNA, 17 bp, synthetic construct
  source 1..17: mol_type = other DNA
gcccctagcgcgcgact

SEQ ID NO: 1000 - DNA, 17 bp, synthetic construct
  source 1..17: mol_type = other DNA
ggcccctagcgcgcgac

SEQ ID NO: 1001 - DNA, 17 bp, synthetic construct
  source 1..17: mol_type = other DNA
cggcccctagcgcgcga

SEQ ID NO: 1002 - DNA, 17 bp, synthetic construct
  source 1..17: mol_type = other DNA
ccggcccctagcgcgcg

SEQ ID NO: 1003 - DNA, 17 bp, synthetic construct
  source 1..17: mol_type = other DNA
cccggcccctagcgcgc

SEQ ID NO: 1004 - DNA, 17 bp, synthetic construct
  source 1..17: mol_type = other DNA
ccccggcccctagcgcg

SEQ ID NO: 1005 - DNA, 17 bp, synthetic construct
  source 1..17: mol_type = other DNA
gccccggcccctagcgc

SEQ ID NO: 1006 - DNA, 17 bp, synthetic construct
  source 1..17: mol_type = other DNA
ggccccggcccctagcg

SEQ ID NO: 1007 - DNA, 17 bp, synthetic construct
  source 1..17: mol_type = other DNA
cggccccggcccctagc

SEQ ID NO: 1008 - DNA, 17 bp, synthetic construct
  source 1..17: mol_type = other DNA
ccggccccggcccctag

SEQ ID NO: 1009 - DNA, 17 bp, synthetic construct
  source 1..17: mol_type = other DNA
cccggccccggccccta

SEQ ID NO: 1010 - DNA, 17 bp, synthetic construct
  source 1..17: mol_type = other DNA
acgccccggccccggcc

SEQ ID NO: 1011 - DNA, 17 bp, synthetic construct
  source 1..17: mol_type = other DNA
cacgccccggccccggc

SEQ ID NO: 1012 - DNA, 17 bp, synthetic construct
  source 1..17: mol_type = other DNA
ccacgccccggccccgg

SEQ ID NO: 1013 - DNA, 17 bp, synthetic construct
  source 1..17: mol_type = other DNA
accacgccccggccccg

SEQ ID NO: 1014 - DNA, 17 bp, synthetic construct
  source 1..17: mol_type = other DNA
gaccacgccccggcccc

SEQ ID NO: 1015 - DNA, 17 bp, synthetic construct
  source 1..17: mol_type = other DNA
cgaccacgccccggccc

SEQ ID NO: 1016 - DNA, 17 bp, synthetic construct
  source 1..17: mol_type = other DNA
ccgaccacgccccggcc

SEQ ID NO: 1017 - DNA, 17 bp, synthetic construct
  source 1..17: mol_type = other DNA
cccgaccacgccccggc

SEQ ID NO: 1018 - DNA, 17 bp, synthetic construct
  source 1..17: mol_type = other DNA
ccccgaccacgccccgg

SEQ ID NO: 1019 - DNA, 17 bp, synthetic construct
  source 1..17: mol_type = other DNA
gccccgaccacgccccg

SEQ ID NO: 1020 - DNA, 17 bp, synthetic construct
  source 1..17: mol_type = other DNA
cgccccgaccacgcccc

SEQ ID NO: 1021 - DNA, 17 bp, synthetic construct
  source 1..17: mol_type = other DNA
ccgccccgaccacgccc

SEQ ID NO: 1022 - DNA, 17 bp, synthetic construct
  source 1..17: mol_type = other DNA
cccgccccgaccacgcc

SEQ ID NO: 1023 - DNA, 17 bp, synthetic construct
  source 1..17: mol_type = other DNA
gcccgccccgaccacgc

SEQ ID NO: 1024 - DNA, 17 bp, synthetic construct
  source 1..17: mol_type = other DNA
ggcccgccccgaccacg

SEQ ID NO: 1025 - DNA, 17 bp, synthetic construct
  source 1..17: mol_type = other DNA
gggcccgccccgaccac

SEQ ID NO: 1026 - DNA, 17 bp, synthetic construct
  source 1..17: mol_type = other DNA
cgggcccgccccgacca

SEQ ID NO: 1027 - DNA, 17 bp, synthetic construct
  source 1..17: mol_type = other DNA
ccgggcccgccccgacc

SEQ ID NO: 1028 - DNA, 17 bp, synthetic construct
  source 1..17: mol_type = other DNA
cccgggcccgccccgac

SEQ ID NO: 1029 - DNA, 17 bp, synthetic construct
  source 1..17: mol_type = other DNA
gcagccccgccccgggc

SEQ ID NO: 1030 - DNA, 17 bp, synthetic construct
  source 1..17: mol_type = other DNA
cgcagccccgccccggg

SEQ ID NO: 1031 - DNA, 17 bp, synthetic construct
  source 1..17: mol_type = other DNA
ccgcagccccgccccgg

SEQ ID NO: 1032 - DNA, 17 bp, synthetic construct
  source 1..17: mol_type = other DNA
accgcagccccgccccg

SEQ ID NO: 1033 - DNA, 17 bp, synthetic construct
  source 1..17: mol_type = other DNA
aaccgcagccccgcccc

SEQ ID NO: 1034 - DNA, 17 bp, synthetic construct
  source 1..17: mol_type = other DNA
caaccgcagccccgccc

SEQ ID NO: 1035 - DNA, 17 bp, synthetic construct
  source 1..17: mol_type = other DNA
gcaaccgcagccccgcc

SEQ ID NO: 1036 - DNA, 17 bp, synthetic construct
  source 1..17: mol_type = other DNA
cgcaaccgcagccccgc

SEQ ID NO: 1037 - DNA, 17 bp, synthetic construct
  source 1..17: mol_type = other DNA
ccgcaaccgcagccccg

SEQ ID NO: 1038 - DNA, 17 bp, synthetic construct
  source 1..17: mol_type = other DNA
accgcaaccgcagcccc

SEQ ID NO: 1039 - DNA, 17 bp, synthetic construct
  source 1..17: mol_type = other DNA
caccgcaaccgcagccc

SEQ ID NO: 1040 - DNA, 17 bp, synthetic construct
  source 1..17: mol_type = other DNA
gcaccgcaaccgcagcc

SEQ ID NO: 1041 - DNA, 17 bp, synthetic construct
  source 1..17: mol_type = other DNA
ggcaccgcaaccgcagc

SEQ ID NO: 1042 - DNA, 17 bp, synthetic construct
  source 1..17: mol_type = other DNA
aggcaccgcaaccgcag

SEQ ID NO: 1043 - DNA, 17 bp, synthetic construct
  source 1..17: mol_type = other DNA
caggcaccgcaaccgca

SEQ ID NO: 1044 - DNA, 17 bp, synthetic construct
  source 1..17: mol_type = other DNA
gcaggcaccgcaaccgc

SEQ ID NO: 1045 - DNA, 17 bp, synthetic construct
  source 1..17: mol_type = other DNA
cgcaggcaccgcaaccg

SEQ ID NO: 1046 - DNA, 17 bp, synthetic construct
  source 1..17: mol_type = other DNA
gcgcaggcaccgcaacc

SEQ ID NO: 1047 - DNA, 17 bp, synthetic construct
  source 1..17: mol_type = other DNA
ggcgcaggcaccgcaac

SEQ ID NO: 1048 - DNA, 20 bp, synthetic construct
  source 1..20: mol_type = other DNA
ccactcgccaccgcctgcgc

SEQ ID NO: 1049 - DNA, 20 bp, synthetic construct
  source 1..20: mol_type = other DNA
tgcattcctaagcaatgtgt

SEQ ID NO: 1050 - DNA, 20 bp, synthetic construct
  source 1..20: mol_type = other DNA
cccggccccggccccggccc

SEQ ID NO: 1051 - DNA, 20 bp, synthetic construct
  source 1..20: mol_type = other DNA
ccccggccccggccccggcc

SEQ ID NO: 1052 - DNA, 20 bp, synthetic construct
  source 1..20: mol_type = other DNA
ttacatctatagcaccactc

SEQ ID NO: 1053 - DNA, 20 bp, synthetic construct
  source 1..20: mol_type = other DNA
tcactcccttttcagacaag

SEQ ID NO: 1054 - DNA, 20 bp, synthetic construct
  source 1..20: mol_type = other DNA
aactaagttctgtctgtgga

SEQ ID NO: 1055 - DNA, 20 bp, synthetic construct
  source 1..20: mol_type = other DNA
atacaggactaaagtgcttc

SEQ ID NO: 1056 - DNA, 20 bp, synthetic construct
  source 1..20: mol_type = other DNA
ctctgaccctgatcttccat

SEQ ID NO: 1057 - DNA, 18 bp, synthetic construct
  source 1..18: mol_type = other DNA
aacagctggagatggcgg

SEQ ID NO: 1058 - DNA, 18 bp, synthetic construct
  source 1..18: mol_type = other DNA
caacagctggagatggcg

SEQ ID NO: 1059 - DNA, 18 bp, synthetic construct
  source 1..18: mol_type = other DNA
gcaacagctggagatggc

SEQ ID NO: 1060 - DNA, 18 bp, synthetic construct
  source 1..18: mol_type = other DNA
ggcaacagctggagatgg

SEQ ID NO: 1061 - DNA, 18 bp, synthetic construct
  source 1..18: mol_type = other DNA
tggcaacagctggagatg

SEQ ID NO: 1062 - DNA, 18 bp, synthetic construct
  source 1..18: mol_type = other DNA
ttggcaacagctggagat

SEQ ID NO: 1063 - DNA, 18 bp, synthetic construct
  source 1..18: mol_type = other DNA
cttggcaacagctggaga

SEQ ID NO: 1064 - DNA, 18 bp, synthetic construct
  source 1..18: mol_type = other DNA
tcttggcaacagctggag

SEQ ID NO: 1065 - DNA, 18 bp, synthetic construct
  source 1..18: mol_type = other DNA
gtcttggcaacagctgga

SEQ ID NO: 1066 - DNA, 18 bp, synthetic construct
  source 1..18: mol_type = other DNA
tgtcttggcaacagctgg

SEQ ID NO: 1067 - DNA, 18 bp, synthetic construct
  source 1..18: mol_type = other DNA
ctgtcttggcaacagctg

SEQ ID NO: 1068 - DNA, 18 bp, synthetic construct
  source 1..18: mol_type = other DNA
tctgtcttggcaacagct

SEQ ID NO: 1069 - DNA, 18 bp, synthetic construct
  source 1..18: mol_type = other DNA
ctctgtcttggcaacagc

SEQ ID NO: 1070 - DNA, 18 bp, synthetic construct
  source 1..18: mol_type = other DNA
tctctgtcttggcaacag

SEQ ID NO: 1071 - DNA, 18 bp, synthetic construct
  source 1..18: mol_type = other DNA
atctctgtcttggcaaca

SEQ ID NO: 1072 - DNA, 18 bp, synthetic construct
  source 1..18: mol_type = other DNA
aatctctgtcttggcaac

SEQ ID NO: 1073 - DNA, 18 bp, synthetic construct
  source 1..18: mol_type = other DNA
caatctctgtcttggcaa

SEQ ID NO: 1074 - DNA, 18 bp, synthetic construct
  source 1..18: mol_type = other DNA
gcaatctctgtcttggca

SEQ ID NO: 1075 - DNA, 18 bp, synthetic construct
  source 1..18: mol_type = other DNA
agcaatctctgtcttggc

SEQ ID NO: 1076 - DNA, 18 bp, synthetic construct
  source 1..18: mol_type = other DNA
aagcaatctctgtcttgg

SEQ ID NO: 1077 - DNA, 18 bp, synthetic construct
  source 1..18: mol_type = other DNA
aaagcaatctctgtcttg

SEQ ID NO: 1078 - DNA, 18 bp, synthetic construct
  source 1..18: mol_type = other DNA
taaagcaatctctgtctt

SEQ ID NO: 1079 - DNA, 18 bp, synthetic construct
  source 1..18: mol_type = other DNA
ttaaagcaatctctgtct

SEQ ID NO: 1080 - DNA, 18 bp, synthetic construct
  source 1..18: mol_type = other DNA
cttaaagcaatctctgtc

SEQ ID NO: 1081 - DNA, 18 bp, synthetic construct
  source 1..18: mol_type = other DNA
acttaaagcaatctctgt

SEQ ID NO: 1082 - DNA, 18 bp, synthetic construct
  source 1..18: mol_type = other DNA
cacttaaagcaatctctg

SEQ ID NO: 1083 - DNA, 18 bp, synthetic construct
  source 1..18: mol_type = other DNA
ccacttaaagcaatctct

SEQ ID NO: 1084 - DNA, 18 bp, synthetic construct
  source 1..18: mol_type = other DNA
ctgctaataaaggtgatt

SEQ ID NO: 1085 - DNA, 18 bp, synthetic construct
  source 1..18: mol_type = other DNA
gctgctaataaaggtgat

SEQ ID NO: 1086 - DNA, 18 bp, synthetic construct
  source 1..18: mol_type = other DNA
agctgctaataaaggtga

SEQ ID NO: 1087 - DNA, 18 bp, synthetic construct
  source 1..18: mol_type = other DNA
tagctgctaataaaggtg

SEQ ID NO: 1088 - DNA, 18 bp, synthetic construct
  source 1..18: mol_type = other DNA
gtagctgctaataaaggt

SEQ ID NO: 1089 - DNA, 18 bp, synthetic construct
  source 1..18: mol_type = other DNA
agtagctgctaataaagg

SEQ ID NO: 1090 - DNA, 18 bp, synthetic construct
  source 1..18: mol_type = other DNA
aagtagctgctaataaag

SEQ ID NO: 1091 - DNA, 18 bp, synthetic construct
  source 1..18: mol_type = other DNA
aaagtagctgctaataaa

SEQ ID NO: 1092 - DNA, 18 bp, synthetic construct
  source 1..18: mol_type = other DNA
aaaagtagctgctaataa

SEQ ID NO: 1093 - DNA, 18 bp, synthetic construct
  source 1..18: mol_type = other DNA
caaaagtagctgctaata

SEQ ID NO: 1094 - DNA, 18 bp, synthetic construct
  source 1..18: mol_type = other DNA
gcaaaagtagctgctaat

SEQ ID NO: 1095 - DNA, 18 bp, synthetic construct
  source 1..18: mol_type = other DNA
agcaaaagtagctgctaa

SEQ ID NO: 1096 - DNA, 18 bp, synthetic construct
  source 1..18: mol_type = other DNA
aagcaaaagtagctgcta

SEQ ID NO: 1097 - DNA, 18 bp, synthetic construct
  source 1..18: mol_type = other DNA
taagcaaaagtagctgct

SEQ ID NO: 1098 - DNA, 18 bp, synthetic construct
  source 1..18: mol_type = other DNA
gtaagcaaaagtagctgc

SEQ ID NO: 1099 - DNA, 18 bp, synthetic construct
  source 1..18: mol_type = other DNA
agtaagcaaaagtagctg

SEQ ID NO: 1100 - DNA, 18 bp, synthetic construct
  source 1..18: mol_type = other DNA
cagtaagcaaaagtagct

SEQ ID NO: 1101 - DNA, 18 bp, synthetic construct
  source 1..18: mol_type = other DNA
ccagtaagcaaaagtagc

SEQ ID NO: 1102 - DNA, 18 bp, synthetic construct
  source 1..18: mol_type = other DNA
cccagtaagcaaaagtag

SEQ ID NO: 1103 - DNA, 18 bp, synthetic construct
  source 1..18: mol_type = other DNA
tcccagtaagcaaaagta

SEQ ID NO: 1104 - DNA, 18 bp, synthetic construct
  source 1..18: mol_type = other DNA
gtcccagtaagcaaaagt

SEQ ID NO: 1105 - DNA, 18 bp, synthetic construct
  source 1..18: mol_type = other DNA
tgtcccagtaagcaaaag

SEQ ID NO: 1106 - DNA, 18 bp, synthetic construct
  source 1..18: mol_type = other DNA
ttgtcccagtaagcaaaa

SEQ ID NO: 1107 - DNA, 18 bp, synthetic construct
  source 1..18: mol_type = other DNA
attgtcccagtaagcaaa

SEQ ID NO: 1108 - DNA, 18 bp, synthetic construct
  source 1..18: mol_type = other DNA
tattgtcccagtaagcaa

SEQ ID NO: 1109 - DNA, 18 bp, synthetic construct
  source 1..18: mol_type = other DNA
atattgtcccagtaagca

SEQ ID NO: 1110 - DNA, 18 bp, synthetic construct
  source 1..18: mol_type = other DNA
aatattgtcccagtaagc

SEQ ID NO: 1111 - DNA, 18 bp, synthetic construct
  source 1..18: mol_type = other DNA
gaatattgtcccagtaag

SEQ ID NO: 1112 - DNA, 18 bp, synthetic construct
  source 1..18: mol_type = other DNA
agaatattgtcccagtaa

SEQ ID NO: 1113 - DNA, 18 bp, synthetic construct
  source 1..18: mol_type = other DNA
aagaatattgtcccagta

SEQ ID NO: 1114 - DNA, 18 bp, synthetic construct
  source 1..18: mol_type = other DNA
caagaatattgtcccagt

SEQ ID NO: 1115 - DNA, 18 bp, synthetic construct
  source 1..18: mol_type = other DNA
ccaagaatattgtcccag

SEQ ID NO: 1116 - DNA, 18 bp, synthetic construct
  source 1..18: mol_type = other DNA
accaagaatattgtccca

SEQ ID NO: 1117 - DNA, 18 bp, synthetic construct
  source 1..18: mol_type = other DNA
gaccaagaatattgtccc

SEQ ID NO: 1118 - DNA, 18 bp, synthetic construct
  source 1..18: mol_type = other DNA
ggaccaagaatattgtcc

SEQ ID NO: 1119 - DNA, 18 bp, synthetic construct
  source 1..18: mol_type = other DNA
aggaccaagaatattgtc

SEQ ID NO: 1120 - DNA, 18 bp, synthetic construct
  source 1..18: mol_type = other DNA
taggaccaagaatattgt

SEQ ID NO: 1121 - DNA, 18 bp, synthetic construct
  source 1..18: mol_type = other DNA
ctaggaccaagaatattg

SEQ ID NO: 1122 - DNA, 18 bp, synthetic construct
  source 1..18: mol_type = other DNA
tctaggaccaagaatatt

SEQ ID NO: 1123 - DNA, 18 bp, synthetic construct
  source 1..18: mol_type = other DNA
ctctaggaccaagaatat

SEQ ID NO: 1124 - DNA, 18 bp, synthetic construct
  source 1..18: mol_type = other DNA
actctaggaccaagaata

SEQ ID NO: 1125 - DNA, 18 bp, synthetic construct
  source 1..18: mol_type = other DNA
tactctaggaccaagaat

SEQ ID NO: 1126 - DNA, 18 bp, synthetic construct
  source 1..18: mol_type = other DNA
ttactctaggaccaagaa

SEQ ID NO: 1127 - DNA, 18 bp, synthetic construct
  source 1..18: mol_type = other DNA
cttactctaggaccaaga

SEQ ID NO: 1128 - DNA, 18 bp, synthetic construct
  source 1..18: mol_type = other DNA
ccttactctaggaccaag

SEQ ID NO: 1129 - DNA, 18 bp, synthetic construct
  source 1..18: mol_type = other DNA
gccttactctaggaccaa

SEQ ID NO: 1130 - DNA, 18 bp, synthetic construct
  source 1..18: mol_type = other DNA
tgccttactctaggacca

SEQ ID NO: 1131 - DNA, 18 bp, synthetic construct
  source 1..18: mol_type = other DNA
gtgccttactctaggacc

SEQ ID NO: 1132 - DNA, 18 bp, synthetic construct
  source 1..18: mol_type = other DNA
tgtgccttactctaggac

SEQ ID NO: 1133 - DNA, 18 bp, synthetic construct
  source 1..18: mol_type = other DNA
atgtgccttactctagga

SEQ ID NO: 1134 - DNA, 18 bp, synthetic construct
  source 1..18: mol_type = other DNA
aatgtgccttactctagg

SEQ ID NO: 1135 - DNA, 18 bp, synthetic construct
  source 1..18: mol_type = other DNA
aaatgtgccttactctag

SEQ ID NO: 1136 - DNA, 18 bp, synthetic construct
  source 1..18: mol_type = other DNA
caaatgtgccttactcta

SEQ ID NO: 1137 - DNA, 18 bp, synthetic construct
  source 1..18: mol_type = other DNA
ccaaatgtgccttactct

SEQ ID NO: 1138 - DNA, 18 bp, synthetic construct
  source 1..18: mol_type = other DNA
cccaaatgtgccttactc

SEQ ID NO: 1139 - DNA, 18 bp, synthetic construct
  source 1..18: mol_type = other DNA
gcccaaatgtgccttact

SEQ ID NO: 1140 - DNA, 18 bp, synthetic construct
  source 1..18: mol_type = other DNA
agcccaaatgtgccttac

SEQ ID NO: 1141 - DNA, 18 bp, synthetic construct
  source 1..18: mol_type = other DNA
gagcccaaatgtgcctta

SEQ ID NO: 1142 - DNA, 18 bp, synthetic construct
  source 1..18: mol_type = other DNA
ggagcccaaatgtgcctt

SEQ ID NO: 1143 - DNA, 18 bp, synthetic construct
  source 1..18: mol_type = other DNA
tggagcccaaatgtgcct

SEQ ID NO: 1144 - DNA, 18 bp, synthetic construct
  source 1..18: mol_type = other DNA
ttggagcccaaatgtgcc

SEQ ID NO: 1145 - DNA, 18 bp, synthetic construct
  source 1..18: mol_type = other DNA
tttggagcccaaatgtgc

SEQ ID NO: 1146 - DNA, 18 bp, synthetic construct
  source 1..18: mol_type = other DNA
ctttggagcccaaatgtg

SEQ ID NO: 1147 - DNA, 18 bp, synthetic construct
  source 1..18: mol_type = other DNA
tctttggagcccaaatgt

SEQ ID NO: 1148 - DNA, 18 bp, synthetic construct
  source 1..18: mol_type = other DNA
gtctttggagcccaaatg

SEQ ID NO: 1149 - DNA, 18 bp, synthetic construct
  source 1..18: mol_type = other DNA
tgtctttggagcccaaat

SEQ ID NO: 1150 - DNA, 18 bp, synthetic construct
  source 1..18: mol_type = other DNA
ctgtctttggagcccaaa

SEQ ID NO: 1151 - DNA, 18 bp, synthetic construct
  source 1..18: mol_type = other DNA
tctgtctttggagcccaa

SEQ ID NO: 1152 - DNA, 18 bp, synthetic construct
  source 1..18: mol_type = other DNA
ttctgtctttggagccca

SEQ ID NO: 1153 - DNA, 18 bp, synthetic construct
  source 1..18: mol_type = other DNA
gttctgtctttggagccc

SEQ ID NO: 1154 - DNA, 18 bp, synthetic construct
  source 1..18: mol_type = other DNA
tgttctgtctttggagcc

SEQ ID NO: 1155 - DNA, 18 bp, synthetic construct
  source 1..18: mol_type = other DNA
ctgttctgtctttggagc

SEQ ID NO: 1156 - DNA, 18 bp, synthetic construct
  source 1..18: mol_type = other DNA
cctgttctgtctttggag

SEQ ID NO: 1157 - DNA, 18 bp, synthetic construct
  source 1..18: mol_type = other DNA
acctgttctgtctttgga

SEQ ID NO: 1158 - DNA, 18 bp, synthetic construct
  source 1..18: mol_type = other DNA
tacctgttctgtctttgg

SEQ ID NO: 1159 - DNA, 18 bp, synthetic construct
  source 1..18: mol_type = other DNA
gtacctgttctgtctttg

SEQ ID NO: 1160 - DNA, 18 bp, synthetic construct
  source 1..18: mol_type = other DNA
agtacctgttctgtcttt

SEQ ID NO: 1161 - DNA, 18 bp, synthetic construct
  source 1..18: mol_type = other DNA
aagtacctgttctgtctt

SEQ ID NO: 1162 - DNA, 18 bp, synthetic construct
  source 1..18: mol_type = other DNA
gaagtacctgttctgtct

SEQ ID NO: 1163 - DNA, 18 bp, synthetic construct
  source 1..18: mol_type = other DNA
agaagtacctgttctgtc

SEQ ID NO: 1164 - DNA, 18 bp, synthetic construct
  source 1..18: mol_type = other DNA
gagaagtacctgttctgt

SEQ ID NO: 1165 - DNA, 18 bp, synthetic construct
  source 1..18: mol_type = other DNA
tgagaagtacctgttctg

SEQ ID NO: 1166 - DNA, 18 bp, synthetic construct
  source 1..18: mol_type = other DNA
ctgagaagtacctgttct

SEQ ID NO: 1167 - DNA, 18 bp, synthetic construct
  source 1..18: mol_type = other DNA
actgagaagtacctgttc

SEQ ID NO: 1168 - DNA, 18 bp, synthetic construct
  source 1..18: mol_type = other DNA
cactgagaagtacctgtt

SEQ ID NO: 1169 - DNA, 18 bp, synthetic construct
  source 1..18: mol_type = other DNA
tcactgagaagtacctgt

SEQ ID NO: 1170 - DNA, 18 bp, synthetic construct
  source 1..18: mol_type = other DNA
atcactgagaagtacctg

SEQ ID NO: 1171 - DNA, 18 bp, synthetic construct
  source 1..18: mol_type = other DNA
catcactgagaagtacct

SEQ ID NO: 1172 - DNA, 18 bp, synthetic construct
  source 1..18: mol_type = other DNA
ccatcactgagaagtacc

SEQ ID NO: 1173 - DNA, 18 bp, synthetic construct
  source 1..18: mol_type = other DNA
tccatcactgagaagtac

SEQ ID NO: 1174 - DNA, 18 bp, synthetic construct
  source 1..18: mol_type = other DNA
ctccatcactgagaagta

SEQ ID NO: 1175 - DNA, 18 bp, synthetic construct
  source 1..18: mol_type = other DNA
tctccatcactgagaagt

SEQ ID NO: 1176 - DNA, 18 bp, synthetic construct
  source 1..18: mol_type = other DNA
ttctccatcactgagaag

SEQ ID NO: 1177 - DNA, 18 bp, synthetic construct
  source 1..18: mol_type = other DNA
tttctccatcactgagaa

SEQ ID NO: 1178 - DNA, 18 bp, synthetic construct
  source 1..18: mol_type = other DNA
atttctccatcactgaga

SEQ ID NO: 1179 - DNA, 18 bp, synthetic construct
  source 1..18: mol_type = other DNA
tatttctccatcactgag

SEQ ID NO: 1180 - DNA, 18 bp, synthetic construct
  source 1..18: mol_type = other DNA
gttatttctccatcactg

SEQ ID NO: 1181 - DNA, 18 bp, synthetic construct
  source 1..18: mol_type = other DNA
agttatttctccatcact

SEQ ID NO: 1182 - DNA, 18 bp, synthetic construct
  source 1..18: mol_type = other DNA
aagttatttctccatcac

SEQ ID NO: 1183 - DNA, 18 bp, synthetic construct
  source 1..18: mol_type = other DNA
aaagttatttctccatca

SEQ ID NO: 1184 - DNA, 18 bp, synthetic construct
  source 1..18: mol_type = other DNA
aaaagttatttctccatc

SEQ ID NO: 1185 - DNA, 18 bp, synthetic construct
  source 1..18: mol_type = other DNA
gaaaagttatttctccat

SEQ ID NO: 1186 - DNA, 18 bp, synthetic construct
  source 1..18: mol_type = other DNA
aagaaaagttatttctcc

SEQ ID NO: 1187 - DNA, 18 bp, synthetic construct
  source 1..18: mol_type = other DNA
caagaaaagttatttctc

SEQ ID NO: 1188 - DNA, 18 bp, synthetic construct
  source 1..18: mol_type = other DNA
gcaagaaaagttatttct

SEQ ID NO: 1189 - DNA, 18 bp, synthetic construct
  source 1..18: mol_type = other DNA
ggcaagaaaagttatttc

SEQ ID NO: 1190 - DNA, 18 bp, synthetic construct
  source 1..18: mol_type = other DNA
tggcaagaaaagttattt

SEQ ID NO: 1191 - DNA, 18 bp, synthetic construct
  source 1..18: mol_type = other DNA
ttggcaagaaaagttatt

SEQ ID NO: 1192 - DNA, 18 bp, synthetic construct
  source 1..18: mol_type = other DNA
gttggcaagaaaagttat

SEQ ID NO: 1193 - DNA, 18 bp, synthetic construct
  source 1..18: mol_type = other DNA
ggttggcaagaaaagtta

SEQ ID NO: 1194 - DNA, 18 bp, synthetic construct
  source 1..18: mol_type = other DNA
tggttggcaagaaaagtt

SEQ ID NO: 1195 - DNA, 18 bp, synthetic construct
  source 1..18: mol_type = other DNA
gtggttggcaagaaaagt

SEQ ID NO: 1196 - DNA, 18 bp, synthetic construct
  source 1..18: mol_type = other DNA
tgtggttggcaagaaaag

SEQ ID NO: 1197 - DNA, 18 bp, synthetic construct
  source 1..18: mol_type = other DNA
gtgtggttggcaagaaaa

SEQ ID NO: 1198 - DNA, 18 bp, synthetic construct
  source 1..18: mol_type = other DNA
agtgtggttggcaagaaa

SEQ ID NO: 1199 - DNA, 18 bp, synthetic construct
  source 1..18: mol_type = other DNA
gagtgtggttggcaagaa

SEQ ID NO: 1200 - DNA, 18 bp, synthetic construct
  source 1..18: mol_type = other DNA
agagtgtggttggcaaga

SEQ ID NO: 1201 - DNA, 18 bp, synthetic construct
  source 1..18: mol_type = other DNA
tagagtgtggttggcaag

SEQ ID NO: 1202 - DNA, 18 bp, synthetic construct
  source 1..18: mol_type = other DNA
ttagagtgtggttggcaa

SEQ ID NO: 1203 - DNA, 18 bp, synthetic construct
  source 1..18: mol_type = other DNA
tttagagtgtggttggca

SEQ ID NO: 1204 - DNA, 18 bp, synthetic construct
  source 1..18: mol_type = other DNA
atttagagtgtggttggc

SEQ ID NO: 1205 - DNA, 18 bp, synthetic construct
  source 1..18: mol_type = other DNA
catttagagtgtggttgg

SEQ ID NO: 1206 - DNA, 18 bp, synthetic construct
  source 1..18: mol_type = other DNA
ccatttagagtgtggttg

SEQ ID NO: 1207 - DNA, 18 bp, synthetic construct
  source 1..18: mol_type = other DNA
tccatttagagtgtggtt

SEQ ID NO: 1208 - DNA, 18 bp, synthetic construct
  source 1..18: mol_type = other DNA
ctccatttagagtgtggt

SEQ ID NO: 1209 - DNA, 18 bp, synthetic construct
  source 1..18: mol_type = other DNA
tctccatttagagtgtgg

SEQ ID NO: 1210 - DNA, 18 bp, synthetic construct
  source 1..18: mol_type = other DNA
ttctccatttagagtgtg

SEQ ID NO: 1211 - DNA, 18 bp, synthetic construct
  source 1..18: mol_type = other DNA
tttctccatttagagtgt

SEQ ID NO: 1212 - DNA, 18 bp, synthetic construct
  source 1..18: mol_type = other DNA
atttctccatttagagtg

SEQ ID NO: 1213 - DNA, 18 bp, synthetic construct
  source 1..18: mol_type = other DNA
gatttctccatttagagt

SEQ ID NO: 1214 - DNA, 18 bp, synthetic construct
  source 1..18: mol_type = other DNA
ggatttctccatttagag

SEQ ID NO: 1215 - DNA, 18 bp, synthetic construct
  source 1..18: mol_type = other DNA
aggatttctccatttaga

SEQ ID NO: 1216 - DNA, 18 bp, synthetic construct
  source 1..18: mol_type = other DNA
aaggatttctccatttag

SEQ ID NO: 1217 - DNA, 18 bp, synthetic construct
  source 1..18: mol_type = other DNA
gaaggatttctccattta

SEQ ID NO: 1218 - DNA, 18 bp, synthetic construct
  source 1..18: mol_type = other DNA
cgaaggatttctccattt

SEQ ID NO: 1219 - DNA, 18 bp, synthetic construct
  source 1..18: mol_type = other DNA
tcgaaggatttctccatt

SEQ ID NO: 1220 - DNA, 18 bp, synthetic construct
  source 1..18: mol_type = other DNA
ttcgaaggatttctccat

SEQ ID NO: 1221 - DNA, 18 bp, synthetic construct
  source 1..18: mol_type = other DNA
tttcgaaggatttctcca

SEQ ID NO: 1222 - DNA, 18 bp, synthetic construct
  source 1..18: mol_type = other DNA
atttcgaaggatttctcc

SEQ ID NO: 1223 - DNA, 18 bp, synthetic construct
  source 1..18: mol_type = other DNA
catttcgaaggatttctc

SEQ ID NO: 1224 - DNA, 18 bp, synthetic construct
  source 1..18: mol_type = other DNA
gcatttcgaaggatttct

SEQ ID NO: 1225 - DNA, 18 bp, synthetic construct
  source 1..18: mol_type = other DNA
tgcatttcgaaggatttc

SEQ ID NO: 1226 - DNA, 18 bp, synthetic construct
  source 1..18: mol_type = other DNA
ctgcatttcgaaggattt

SEQ ID NO: 1227 - DNA, 18 bp, synthetic construct
  source 1..18: mol_type = other DNA
tctgcatttcgaaggatt

SEQ ID NO: 1228 - DNA, 18 bp, synthetic construct
  source 1..18: mol_type = other DNA
ctctgcatttcgaaggat

SEQ ID NO: 1229 - DNA, 18 bp, synthetic construct
  source 1..18: mol_type = other DNA
tctctgcatttcgaagga

SEQ ID NO: 1230 - DNA, 18 bp, synthetic construct
  source 1..18: mol_type = other DNA
ctctctgcatttcgaagg

SEQ ID NO: 1231 - DNA, 18 bp, synthetic construct
  source 1..18: mol_type = other DNA
actctctgcatttcgaag

SEQ ID NO: 1232 - DNA, 18 bp, synthetic construct
  source 1..18: mol_type = other DNA
cactctctgcatttcgaa

SEQ ID NO: 1233 - DNA, 18 bp, synthetic construct
  source 1..18: mol_type = other DNA
ccactctctgcatttcga

SEQ ID NO: 1234 - DNA, 18 bp, synthetic construct
  source 1..18: mol_type = other DNA
accactctctgcatttcg

SEQ ID NO: 1235 - DNA, 18 bp, synthetic construct
  source 1..18: mol_type = other DNA
caccactctctgcatttc

SEQ ID NO: 1236 - DNA, 18 bp, synthetic construct
  source 1..18: mol_type = other DNA
gcaccactctctgcattt

SEQ ID NO: 1237 - DNA, 18 bp, synthetic construct
  source 1..18: mol_type = other DNA
agcaccactctctgcatt

SEQ ID NO: 1238 - DNA, 18 bp, synthetic construct
  source 1..18: mol_type = other DNA
tagcaccactctctgcat

SEQ ID NO: 1239 - DNA, 18 bp, synthetic construct
  source 1..18: mol_type = other DNA
atagcaccactctctgca

SEQ ID NO: 1240 - DNA, 18 bp, synthetic construct
  source 1..18: mol_type = other DNA
tatagcaccactctctgc

SEQ ID NO: 1241 - DNA, 18 bp, synthetic construct
  source 1..18: mol_type = other DNA
ctatagcaccactctctg

SEQ ID NO: 1242 - DNA, 18 bp, synthetic construct
  source 1..18: mol_type = other DNA
tctatagcaccactctct

SEQ ID NO: 1243 - DNA, 18 bp, synthetic construct
  source 1..18: mol_type = other DNA
atctatagcaccactctc

SEQ ID NO: 1244 - DNA, 18 bp, synthetic construct
  source 1..18: mol_type = other DNA
catctatagcaccactct

SEQ ID NO: 1245 - DNA, 18 bp, synthetic construct
  source 1..18: mol_type = other DNA
acatctatagcaccactc

SEQ ID NO: 1246 - DNA, 18 bp, synthetic construct
  source 1..18: mol_type = other DNA
tacatctatagcaccact

SEQ ID NO: 1247 - DNA, 18 bp, synthetic construct
  source 1..18: mol_type = other DNA
ttacatctatagcaccac

SEQ ID NO: 1248 - DNA, 18 bp, synthetic construct
  source 1..18: mol_type = other DNA
tttacatctatagcacca

SEQ ID NO: 1249 - DNA, 18 bp, synthetic construct
  source 1..18: mol_type = other DNA
ctttacatctatagcacc

SEQ ID NO: 1250 - DNA, 18 bp, synthetic construct
  source 1..18: mol_type = other DNA
actttacatctatagcac

SEQ ID NO: 1251 - DNA, 18 bp, synthetic construct
  source 1..18: mol_type = other DNA
aactttacatctatagca

SEQ ID NO: 1252 - DNA, 18 bp, synthetic construct
  source 1..18: mol_type = other DNA
aaactttacatctatagc

SEQ ID NO: 1253 - DNA, 18 bp, synthetic construct
  source 1..18: mol_type = other DNA
aaaactttacatctatag

SEQ ID NO: 1254 - DNA, 18 bp, synthetic construct
  source 1..18: mol_type = other DNA
aaaaaactttacatctat

SEQ ID NO: 1255 - DNA, 18 bp, synthetic construct
  source 1..18: mol_type = other DNA
caaaaaactttacatcta

SEQ ID NO: 1256 - DNA, 18 bp, synthetic construct
  source 1..18: mol_type = other DNA
acaaaaaactttacatct

SEQ ID NO: 1257 - DNA, 18 bp, synthetic construct
  source 1..18: mol_type = other DNA
gacaaaaaactttacatc

SEQ ID NO: 1258 - DNA, 18 bp, synthetic construct
  source 1..18: mol_type = other DNA
caagacaaaaaactttac

SEQ ID NO: 1259 - DNA, 18 bp, synthetic construct
  source 1..18: mol_type = other DNA
gacaagacaaaaaacttt

SEQ ID NO: 1260 - DNA, 18 bp, synthetic construct
  source 1..18: mol_type = other DNA
agacaagacaaaaaactt

SEQ ID NO: 1261 - DNA, 18 bp, synthetic construct
  source 1..18: mol_type = other DNA
cagacaagacaaaaaact

SEQ ID NO: 1262 - DNA, 18 bp, synthetic construct
  source 1..18: mol_type = other DNA
tcagacaagacaaaaaac

SEQ ID NO: 1263 - DNA, 18 bp, synthetic construct
  source 1..18: mol_type = other DNA
ttcagacaagacaaaaaa

SEQ ID NO: 1264 - DNA, 18 bp, synthetic construct
  source 1..18: mol_type = other DNA
ttttcagacaagacaaaa

SEQ ID NO: 1265 - DNA, 18 bp, synthetic construct
  source 1..18: mol_type = other DNA
cttttcagacaagacaaa

SEQ ID NO: 1266 - DNA, 18 bp, synthetic construct
  source 1..18: mol_type = other DNA
ccttttcagacaagacaa

SEQ ID NO: 1267 - DNA, 18 bp, synthetic construct
  source 1..18: mol_type = other DNA
cccttttcagacaagaca

SEQ ID NO: 1268 - DNA, 18 bp, synthetic construct
  source 1..18: mol_type = other DNA
tcccttttcagacaagac

SEQ ID NO: 1269 - DNA, 18 bp, synthetic construct
  source 1..18: mol_type = other DNA
ctcccttttcagacaaga

SEQ ID NO: 1270 - DNA, 18 bp, synthetic construct
  source 1..18: mol_type = other DNA
actcccttttcagacaag

SEQ ID NO: 1271 - DNA, 18 bp, synthetic construct
  source 1..18: mol_type = other DNA
cactcccttttcagacaa

SEQ ID NO: 1272 - DNA, 18 bp, synthetic construct
  source 1..18: mol_type = other DNA
tcactcccttttcagaca

SEQ ID NO: 1273 - DNA, 18 bp, synthetic construct
  source 1..18: mol_type = other DNA
atcactcccttttcagac

SEQ ID NO: 1274 - DNA, 18 bp, synthetic construct
  source 1..18: mol_type = other DNA
aatcactcccttttcaga

SEQ ID NO: 1275 - DNA, 18 bp, synthetic construct
  source 1..18: mol_type = other DNA
taatcactcccttttcag

SEQ ID NO: 1276 - DNA, 18 bp, synthetic construct
  source 1..18: mol_type = other DNA
ataatcactcccttttca

SEQ ID NO: 1277 - DNA, 18 bp, synthetic construct
  source 1..18: mol_type = other DNA
aataatcactcccttttc

SEQ ID NO: 1278 - DNA, 18 bp, synthetic construct
  source 1..18: mol_type = other DNA
caataatcactccctttt

SEQ ID NO: 1279 - DNA, 18 bp, synthetic construct
  source 1..18: mol_type = other DNA
acaataatcactcccttt

SEQ ID NO: 1280 - DNA, 18 bp, synthetic construct
  source 1..18: mol_type = other DNA
aacaataatcactccctt

SEQ ID NO: 1281 - DNA, 18 bp, synthetic construct
  source 1..18: mol_type = other DNA
aaacaataatcactccct

SEQ ID NO: 1282 - DNA, 18 bp, synthetic construct
  source 1..18: mol_type = other DNA
gaaacaataatcactccc

SEQ ID NO: 1283 - DNA, 18 bp, synthetic construct
  source 1..18: mol_type = other DNA
tgaaacaataatcactcc

SEQ ID NO: 1284 - DNA, 18 bp, synthetic construct
  source 1..18: mol_type = other DNA
atgaaacaataatcactc

SEQ ID NO: 1285 - DNA, 18 bp, synthetic construct
  source 1..18: mol_type = other DNA
aatgaaacaataatcact

SEQ ID NO: 1286 - DNA, 18 bp, synthetic construct
  source 1..18: mol_type = other DNA
taatgaaacaataatcac

SEQ ID NO: 1287 - DNA, 18 bp, synthetic construct
  source 1..18: mol_type = other DNA
ttaatgaaacaataatca

SEQ ID NO: 1288 - DNA, 18 bp, synthetic construct
  source 1..18: mol_type = other DNA
attaatgaaacaataatc

SEQ ID NO: 1289 - DNA, 18 bp, synthetic construct
  source 1..18: mol_type = other DNA
atcaaagattaatgaaac

SEQ ID NO: 1290 - DNA, 18 bp, synthetic construct
  source 1..18: mol_type = other DNA
catcaaagattaatgaaa

SEQ ID NO: 1291 - DNA, 18 bp, synthetic construct
  source 1..18: mol_type = other DNA
ccatcaaagattaatgaa

SEQ ID NO: 1292 - DNA, 18 bp, synthetic construct
  source 1..18: mol_type = other DNA
tccatcaaagattaatga

SEQ ID NO: 1293 - DNA, 18 bp, synthetic construct
  source 1..18: mol_type = other DNA
ttccatcaaagattaatg

SEQ ID NO: 1294 - DNA, 18 bp, synthetic construct
  source 1..18: mol_type = other DNA
tttccatcaaagattaat

SEQ ID NO: 1295 - DNA, 18 bp, synthetic construct
  source 1..18: mol_type = other DNA
gtttccatcaaagattaa

SEQ ID NO: 1296 - DNA, 18 bp, synthetic construct
  source 1..18: mol_type = other DNA
agtttccatcaaagatta

SEQ ID NO: 1297 - DNA, 18 bp, synthetic construct
  source 1..18: mol_type = other DNA
cagtttccatcaaagatt

SEQ ID NO: 1298 - DNA, 18 bp, synthetic construct
  source 1..18: mol_type = other DNA
ccagtttccatcaaagat

SEQ ID NO: 1299 - DNA, 18 bp, synthetic construct
  source 1..18: mol_type = other DNA
tccagtttccatcaaaga

SEQ ID NO: 1300 - DNA, 18 bp, synthetic construct
  source 1..18: mol_type = other DNA
ttccagtttccatcaaag

SEQ ID NO: 1301 - DNA, 18 bp, synthetic construct
  source 1..18: mol_type = other DNA
attccagtttccatcaaa

SEQ ID NO: 1302 - DNA, 18 bp, synthetic construct
  source 1..18: mol_type = other DNA
cattccagtttccatcaa

SEQ ID NO: 1303 - DNA, 18 bp, synthetic construct
  source 1..18: mol_type = other DNA
ccattccagtttccatca

SEQ ID NO: 1304 - DNA, 18 bp, synthetic construct
  source 1..18: mol_type = other DNA
cccattccagtttccatc

SEQ ID NO: 1305 - DNA, 18 bp, synthetic construct
  source 1..18: mol_type = other DNA
ccccattccagtttccat

SEQ ID NO: 1306 - DNA, 18 bp, synthetic construct
  source 1..18: mol_type = other DNA
tccccattccagtttcca

SEQ ID NO: 1307 - DNA, 18 bp, synthetic construct
  source 1..18: mol_type = other DNA
atccccattccagtttcc

SEQ ID NO: 1308 - DNA, 18 bp, synthetic construct
  source 1..18: mol_type = other DNA
gatccccattccagtttc

SEQ ID NO: 1309 - DNA, 18 bp, synthetic construct
  source 1..18: mol_type = other DNA
cgatccccattccagttt

SEQ ID NO: 1310 - DNA, 18 bp, synthetic construct
  source 1..18: mol_type = other DNA
gcgatccccattccagtt

SEQ ID NO: 1311 - DNA, 18 bp, synthetic construct
  source 1..18: mol_type = other DNA
tgcgatccccattccagt

SEQ ID NO: 1312 - DNA, 18 bp, synthetic construct
  source 1..18: mol_type = other DNA
ctgcgatccccattccag

SEQ ID NO: 1313 - DNA, 18 bp, synthetic construct
  source 1..18: mol_type = other DNA
gctgcgatccccattcca

SEQ ID NO: 1314 - DNA, 18 bp, synthetic construct
  source 1..18: mol_type = other DNA
tgctgcgatccccattcc

SEQ ID NO: 1315 - DNA, 18 bp, synthetic construct
  source 1..18: mol_type = other DNA
gtgctgcgatccccattc

SEQ ID NO: 1316 - DNA, 18 bp, synthetic construct
  source 1..18: mol_type = other DNA
tgtgctgcgatccccatt

SEQ ID NO: 1317 - DNA, 18 bp, synthetic construct
  source 1..18: mol_type = other DNA
atgtgctgcgatccccat

SEQ ID NO: 1318 - DNA, 18 bp, synthetic construct
  source 1..18: mol_type = other DNA
tatgtgctgcgatcccca

SEQ ID NO: 1319 - DNA, 18 bp, synthetic construct
  source 1..18: mol_type = other DNA
aagtataattgatagtcc

SEQ ID NO: 1320 - DNA, 18 bp, synthetic construct
  source 1..18: mol_type = other DNA
gaagtataattgatagtc

SEQ ID NO: 1321 - DNA, 18 bp, synthetic construct
  source 1..18: mol_type = other DNA
ggaagtataattgatagt

SEQ ID NO: 1322 - DNA, 18 bp, synthetic construct
  source 1..18: mol_type = other DNA
tggaagtataattgatag

SEQ ID NO: 1323 - DNA, 18 bp, synthetic construct
  source 1..18: mol_type = other DNA
gtggaagtataattgata

SEQ ID NO: 1324 - DNA, 18 bp, synthetic construct
  source 1..18: mol_type = other DNA
tgtggaagtataattgat

SEQ ID NO: 1325 - DNA, 18 bp, synthetic construct
  source 1..18: mol_type = other DNA
ctgtggaagtataattga

SEQ ID NO: 1326 - DNA, 18 bp, synthetic construct
  source 1..18: mol_type = other DNA
tctgtggaagtataattg

SEQ ID NO: 1327 - DNA, 18 bp, synthetic construct
  source 1..18: mol_type = other DNA
gtctgtggaagtataatt

SEQ ID NO: 1328 - DNA, 18 bp, synthetic construct
  source 1..18: mol_type = other DNA
tgtctgtggaagtataat

SEQ ID NO: 1329 - DNA, 18 bp, synthetic construct
  source 1..18: mol_type = other DNA
ctgtctgtggaagtataa

SEQ ID NO: 1330 - DNA, 18 bp, synthetic construct
  source 1..18: mol_type = other DNA
tctgtctgtggaagtata

SEQ ID NO: 1331 - DNA, 18 bp, synthetic construct
  source 1..18: mol_type = other DNA
ttctgtctgtggaagtat

SEQ ID NO: 1332 - DNA, 18 bp, synthetic construct
  source 1..18: mol_type = other DNA
gttctgtctgtggaagta

SEQ ID NO: 1333 - DNA, 18 bp, synthetic construct
  source 1..18: mol_type = other DNA
agttctgtctgtggaagt

SEQ ID NO: 1334 - DNA, 18 bp, synthetic construct
  source 1..18: mol_type = other DNA
aagttctgtctgtggaag

SEQ ID NO: 1335 - DNA, 18 bp, synthetic construct
  source 1..18: mol_type = other DNA
taagttctgtctgtggaa

SEQ ID NO: 1336 - DNA, 18 bp, synthetic construct
  source 1..18: mol_type = other DNA
ctaagttctgtctgtgga

SEQ ID NO: 1337 - DNA, 18 bp, synthetic construct
  source 1..18: mol_type = other DNA
actaagttctgtctgtgg

SEQ ID NO: 1338 - DNA, 18 bp, synthetic construct
  source 1..18: mol_type = other DNA
aactaagttctgtctgtg

SEQ ID NO: 1339 - DNA, 18 bp, synthetic construct
  source 1..18: mol_type = other DNA
aaactaagttctgtctgt

SEQ ID NO: 1340 - DNA, 18 bp, synthetic construct
  source 1..18: mol_type = other DNA
gaaactaagttctgtctg

SEQ ID NO: 1341 - DNA, 18 bp, synthetic construct
  source 1..18: mol_type = other DNA
agaaactaagttctgtct

SEQ ID NO: 1342 - DNA, 18 bp, synthetic construct
  source 1..18: mol_type = other DNA
tagaaactaagttctgtc

SEQ ID NO: 1343 - DNA, 18 bp, synthetic construct
  source 1..18: mol_type = other DNA
gtagaaactaagttctgt

SEQ ID NO: 1344 - DNA, 18 bp, synthetic construct
  source 1..18: mol_type = other DNA
ggtagaaactaagttctg

SEQ ID NO: 1345 - DNA, 18 bp, synthetic construct
  source 1..18: mol_type = other DNA
aggtagaaactaagttct

SEQ ID NO: 1346 - DNA, 18 bp, synthetic construct
  source 1..18: mol_type = other DNA
gaggtagaaactaagttc

SEQ ID NO: 1347 - DNA, 18 bp, synthetic construct
  source 1..18: mol_type = other DNA
ggaggtagaaactaagtt

SEQ ID NO: 1348 - DNA, 18 bp, synthetic construct
  source 1..18: mol_type = other DNA
gggaggtagaaactaagt

SEQ ID NO: 1349 - DNA, 18 bp, synthetic construct
  source 1..18: mol_type = other DNA
tgggaggtagaaactaag

SEQ ID NO: 1350 - DNA, 18 bp, synthetic construct
  source 1..18: mol_type = other DNA
gtgggaggtagaaactaa

SEQ ID NO: 1351 - DNA, 18 bp, synthetic construct
  source 1..18: mol_type = other DNA
agtgggaggtagaaacta

SEQ ID NO: 1352 - DNA, 18 bp, synthetic construct
  source 1..18: mol_type = other DNA
aagtgggaggtagaaact

SEQ ID NO: 1353 - DNA, 18 bp, synthetic construct
  source 1..18: mol_type = other DNA
gaagtgggaggtagaaac

SEQ ID NO: 1354 - DNA, 18 bp, synthetic construct
  source 1..18: mol_type = other DNA
tgaagtgggaggtagaaa

SEQ ID NO: 1355 - DNA, 18 bp, synthetic construct
  source 1..18: mol_type = other DNA
atgaagtgggaggtagaa

SEQ ID NO: 1356 - DNA, 18 bp, synthetic construct
  source 1..18: mol_type = other DNA
tatgaagtgggaggtaga

SEQ ID NO: 1357 - DNA, 18 bp, synthetic construct
  source 1..18: mol_type = other DNA
ctatgaagtgggaggtag

SEQ ID NO: 1358 - DNA, 18 bp, synthetic construct
  source 1..18: mol_type = other DNA
tctatgaagtgggaggta

SEQ ID NO: 1359 - DNA, 18 bp, synthetic construct
  source 1..18: mol_type = other DNA
ctctatgaagtgggaggt

SEQ ID NO: 1360 - DNA, 18 bp, synthetic construct
  source 1..18: mol_type = other DNA
actctatgaagtgggagg

SEQ ID NO: 1361 - DNA, 18 bp, synthetic construct
  source 1..18: mol_type = other DNA
cactctatgaagtgggag

SEQ ID NO: 1362 - DNA, 18 bp, synthetic construct
  source 1..18: mol_type = other DNA
acactctatgaagtggga

SEQ ID NO: 1363 - DNA, 18 bp, synthetic construct
  source 1..18: mol_type = other DNA
cacactctatgaagtggg

SEQ ID NO: 1364 - DNA, 18 bp, synthetic construct
  source 1..18: mol_type = other DNA
acacactctatgaagtgg

SEQ ID NO: 1365 - DNA, 18 bp, synthetic construct
  source 1..18: mol_type = other DNA
cacacactctatgaagtg

SEQ ID NO: 1366 - DNA, 18 bp, synthetic construct
  source 1..18: mol_type = other DNA
acacacactctatgaagt

SEQ ID NO: 1367 - DNA, 18 bp, synthetic construct
  source 1..18: mol_type = other DNA
ccctgatcttccattctc

SEQ ID NO: 1368 - DNA, 18 bp, synthetic construct
  source 1..18: mol_type = other DNA
accctgatcttccattct

SEQ ID NO: 1369 - DNA, 18 bp, synthetic construct
  source 1..18: mol_type = other DNA
gaccctgatcttccattc

SEQ ID NO: 1370 - DNA, 18 bp, synthetic construct
  source 1..18: mol_type = other DNA
tgaccctgatcttccatt

SEQ ID NO: 1371 - DNA, 18 bp, synthetic construct
  source 1..18: mol_type = other DNA
ctgaccctgatcttccat

SEQ ID NO: 1372 - DNA, 18 bp, synthetic construct
  source 1..18: mol_type = other DNA
tctgaccctgatcttcca

SEQ ID NO: 1373 - DNA, 18 bp, synthetic construct
  source 1..18: mol_type = other DNA
ctctgaccctgatcttcc

SEQ ID NO: 1374 - DNA, 18 bp, synthetic construct
  source 1..18: mol_type = other DNA
actctgaccctgatcttc

SEQ ID NO: 1375 - DNA, 18 bp, synthetic construct
  source 1..18: mol_type = other DNA
tactctgaccctgatctt

SEQ ID NO: 1376 - DNA, 18 bp, synthetic construct
  source 1..18: mol_type = other DNA
atactctgaccctgatct

SEQ ID NO: 1377 - DNA, 18 bp, synthetic construct
  source 1..18: mol_type = other DNA
aatactctgaccctgatc

SEQ ID NO: 1378 - DNA, 18 bp, synthetic construct
  source 1..18: mol_type = other DNA
atgatttcttgtctggga

SEQ ID NO: 1379 - DNA, 18 bp, synthetic construct
  source 1..18: mol_type = other DNA
catgatttcttgtctggg

SEQ ID NO: 1380 - DNA, 18 bp, synthetic construct
  source 1..18: mol_type = other DNA
ccatgatttcttgtctgg

SEQ ID NO: 1381 - DNA, 18 bp, synthetic construct
  source 1..18: mol_type = other DNA
gccatgatttcttgtctg

SEQ ID NO: 1382 - DNA, 18 bp, synthetic construct
  source 1..18: mol_type = other DNA
ggccatgatttcttgtct

SEQ ID NO: 1383 - DNA, 18 bp, synthetic construct
  source 1..18: mol_type = other DNA
gggccatgatttcttgtc

SEQ ID NO: 1384 - DNA, 18 bp, synthetic construct
  source 1..18: mol_type = other DNA
aactaacatgtaggcact

SEQ ID NO: 1385 - DNA, 18 bp, synthetic construct
  source 1..18: mol_type = other DNA
gaactaacatgtaggcac

SEQ ID NO: 1386 - DNA, 18 bp, synthetic construct
  source 1..18: mol_type = other DNA
ggaactaacatgtaggca

SEQ ID NO: 1387 - DNA, 18 bp, synthetic construct
  source 1..18: mol_type = other DNA
aggaactaacatgtaggc

SEQ ID NO: 1388 - DNA, 18 bp, synthetic construct
  source 1..18: mol_type = other DNA
cttctgattcaagccatt

SEQ ID NO: 1389 - DNA, 18 bp, synthetic construct
  source 1..18: mol_type = other DNA
gcttctgattcaagccat

SEQ ID NO: 1390 - DNA, 18 bp, synthetic construct
  source 1..18: mol_type = other DNA
tgcttctgattcaagcca

SEQ ID NO: 1391 - DNA, 18 bp, synthetic construct
  source 1..18: mol_type = other DNA
gtgcttctgattcaagcc

SEQ ID NO: 1392 - DNA, 18 bp, synthetic construct
  source 1..18: mol_type = other DNA
agtgcttctgattcaagc

SEQ ID NO: 1393 - DNA, 18 bp, synthetic construct
  source 1..18: mol_type = other DNA
aagtgcttctgattcaag

SEQ ID NO: 1394 - DNA, 18 bp, synthetic construct
  source 1..18: mol_type = other DNA
aaagtgcttctgattcaa

SEQ ID NO: 1395 - DNA, 18 bp, synthetic construct
  source 1..18: mol_type = other DNA
taaagtgcttctgattca

SEQ ID NO: 1396 - DNA, 18 bp, synthetic construct
  source 1..18: mol_type = other DNA
ctaaagtgcttctgattc

SEQ ID NO: 1397 - DNA, 18 bp, synthetic construct
  source 1..18: mol_type = other DNA
actaaagtgcttctgatt

SEQ ID NO: 1398 - DNA, 18 bp, synthetic construct
  source 1..18: mol_type = other DNA
gactaaagtgcttctgat

SEQ ID NO: 1399 - DNA, 18 bp, synthetic construct
  source 1..18: mol_type = other DNA
ggactaaagtgcttctga

SEQ ID NO: 1400 - DNA, 18 bp, synthetic construct
  source 1..18: mol_type = other DNA
aggactaaagtgcttctg

SEQ ID NO: 1401 - DNA, 18 bp, synthetic construct
  source 1..18: mol_type = other DNA
caggactaaagtgcttct

SEQ ID NO: 1402 - DNA, 18 bp, synthetic construct
  source 1..18: mol_type = other DNA
acaggactaaagtgcttc

SEQ ID NO: 1403 - DNA, 18 bp, synthetic construct
  source 1..18: mol_type = other DNA
tacaggactaaagtgctt

SEQ ID NO: 1404 - DNA, 18 bp, synthetic construct
  source 1..18: mol_type = other DNA
atacaggactaaagtgct

SEQ ID NO: 1405 - DNA, 18 bp, synthetic construct
  source 1..18: mol_type = other DNA
gatacaggactaaagtgc

SEQ ID NO: 1406 - DNA, 18 bp, synthetic construct
  source 1..18: mol_type = other DNA
agatacaggactaaagtg

SEQ ID NO: 1407 - DNA, 18 bp, synthetic construct
  source 1..18: mol_type = other DNA
cagatacaggactaaagt

SEQ ID NO: 1408 - DNA, 18 bp, synthetic construct
  source 1..18: mol_type = other DNA
acagatacaggactaaag

SEQ ID NO: 1409 - DNA, 18 bp, synthetic construct
  source 1..18: mol_type = other DNA
aacagatacaggactaaa

SEQ ID NO: 1410 - DNA, 18 bp, synthetic construct
  source 1..18: mol_type = other DNA
gaacagatacaggactaa

SEQ ID NO: 1411 - DNA, 18 bp, synthetic construct
  source 1..18: mol_type = other DNA
tgaacagatacaggacta

SEQ ID NO: 1412 - DNA, 18 bp, synthetic construct
  source 1..18: mol_type = other DNA
ctgaacagatacaggact

SEQ ID NO: 1413 - DNA, 18 bp, synthetic construct
  source 1..18: mol_type = other DNA
actgaacagatacaggac

SEQ ID NO: 1414 - DNA, 18 bp, synthetic construct
  source 1..18: mol_type = other DNA
cactgaacagatacagga

SEQ ID NO: 1415 - DNA, 18 bp, synthetic construct
  source 1..18: mol_type = other DNA
acactgaacagatacagg

SEQ ID NO: 1416 - DNA, 18 bp, synthetic construct
  source 1..18: mol_type = other DNA
gacactgaacagatacag

SEQ ID NO: 1417 - DNA, 18 bp, synthetic construct
  source 1..18: mol_type = other DNA
tgacactgaacagataca

SEQ ID NO: 1418 - DNA, 18 bp, synthetic construct
  source 1..18: mol_type = other DNA
ctgacactgaacagatac

SEQ ID NO: 1419 - DNA, 18 bp, synthetic construct
  source 1..18: mol_type = other DNA
gctgacactgaacagata

SEQ ID NO: 1420 - DNA, 18 bp, synthetic construct
  source 1..18: mol_type = other DNA
ggctgacactgaacagat

SEQ ID NO: 1421 - DNA, 18 bp, synthetic construct
  source 1..18: mol_type = other DNA
aggctgacactgaacaga

SEQ ID NO: 1422 - DNA, 18 bp, synthetic construct
  source 1..18: mol_type = other DNA
aaggctgacactgaacag

SEQ ID NO: 1423 - DNA, 18 bp, synthetic construct
  source 1..18: mol_type = other DNA
aaaggctgacactgaaca

SEQ ID NO: 1424 - DNA, 18 bp, synthetic construct
  source 1..18: mol_type = other DNA
gaaaggctgacactgaac

SEQ ID NO: 1425 - DNA, 18 bp, synthetic construct
  source 1..18: mol_type = other DNA
tgaaaggctgacactgaa

SEQ ID NO: 1426 - DNA, 18 bp, synthetic construct
  source 1..18: mol_type = other DNA
tgggatttaaaatgatgt

SEQ ID NO: 1427 - DNA, 18 bp, synthetic construct
  source 1..18: mol_type = other DNA
atgggatttaaaatgatg

SEQ ID NO: 1428 - DNA, 18 bp, synthetic construct
  source 1..18: mol_type = other DNA
cttgagaagaaagccttc

SEQ ID NO: 1429 - DNA, 18 bp, synthetic construct
  source 1..18: mol_type = other DNA
attaaggctcttaggtta

SEQ ID NO: 1430 - DNA, 18 bp, synthetic construct
  source 1..18: mol_type = other DNA
gtagacagtctgttattt

SEQ ID NO: 1431 - DNA, 18 bp, synthetic construct
  source 1..18: mol_type = other DNA
tgacatgtagagagatta

SEQ ID NO: 1432 - DNA, 18 bp, synthetic construct
  source 1..18: mol_type = other DNA
tggtttaagggcacaaac

SEQ ID NO: 1433 - DNA, 18 bp, synthetic construct
  source 1..18: mol_type = other DNA
acttgagaagaaagcctt

SEQ ID NO: 1434 - DNA, 18 bp, synthetic construct
  source 1..18: mol_type = other DNA
cctctgatactccatcat

SEQ ID NO: 1435 - DNA, 18 bp, synthetic construct
  source 1..18: mol_type = other DNA
aaatcttgtcataggtga

SEQ ID NO: 1436 - DNA, 18 bp, synthetic construct
  source 1..18: mol_type = other DNA
aattcttacttgagaaga

SEQ ID NO: 1437 - DNA, 18 bp, synthetic construct
  source 1..18: mol_type = other DNA
ggtgtatagagaattcag

SEQ ID NO: 1438 - DNA, 18 bp, synthetic construct
  source 1..18: mol_type = other DNA
tactccatcatgagccta

SEQ ID NO: 1439 - DNA, 18 bp, synthetic construct
  source 1..18: mol_type = other DNA
gctggatggaaaaagatc

SEQ ID NO: 1440 - DNA, 18 bp, synthetic construct
  source 1..18: mol_type = other DNA
gtccctagaacaatctaa

SEQ ID NO: 1441 - DNA, 18 bp, synthetic construct
  source 1..18: mol_type = other DNA
gaagaaattgacatgtag

SEQ ID NO: 1442 - DNA, 18 bp, synthetic construct
  source 1..18: mol_type = other DNA
catctacagtacaactta

SEQ ID NO: 1443 - DNA, 20 bp, synthetic construct
  source 1..20: mol_type = other DNA
atctctgtcttggcaacagc

SEQ ID NO: 1444 - DNA, 20 bp, synthetic construct
  source 1..20: mol_type = other DNA
aatctctgtcttggcaacag

SEQ ID NO: 1445 - DNA, 20 bp, synthetic construct
  source 1..20: mol_type = other DNA
caatctctgtcttggcaaca

SEQ ID NO: 1446 - DNA, 20 bp, synthetic construct
  source 1..20: mol_type = other DNA
aagcaatctctgtcttggca

SEQ ID NO: 1447 - DNA, 20 bp, synthetic construct
  source 1..20: mol_type = other DNA
ttactctaggaccaagaata

SEQ ID NO: 1448 - DNA, 20 bp, synthetic construct
  source 1..20: mol_type = other DNA
cttactctaggaccaagaat

SEQ ID NO: 1449 - DNA, 20 bp, synthetic construct
  source 1..20: mol_type = other DNA
tgccttactctaggaccaag

SEQ ID NO: 1450 - DNA, 20 bp, synthetic construct
  source 1..20: mol_type = other DNA
tgtgccttactctaggacca

SEQ ID NO: 1451 - DNA, 20 bp, synthetic construct
  source 1..20: mol_type = other DNA
atgtgccttactctaggacc

SEQ ID NO: 1452 - DNA, 20 bp, synthetic construct
  source 1..20: mol_type = other DNA
cccaaatgtgccttactcta

SEQ ID NO: 1453 - DNA, 20 bp, synthetic construct
  source 1..20: mol_type = other DNA
gcccaaatgtgccttactct

SEQ ID NO: 1454 - DNA, 20 bp, synthetic construct
  source 1..20: mol_type = other DNA
gagcccaaatgtgccttact

SEQ ID NO: 1455 - DNA, 20 bp, synthetic construct
  source 1..20: mol_type = other DNA
ggagcccaaatgtgccttac

SEQ ID NO: 1456 - DNA, 20 bp, synthetic construct
  source 1..20: mol_type = other DNA
ttggagcccaaatgtgcctt

SEQ ID NO: 1457 - DNA, 20 bp, synthetic construct
  source 1..20: mol_type = other DNA
tttggagcccaaatgtgcct

SEQ ID NO: 1458 - DNA, 20 bp, synthetic construct
  source 1..20: mol_type = other DNA
ctgtctttggagcccaaatg

SEQ ID NO: 1459 - DNA, 20 bp, synthetic construct
  source 1..20: mol_type = other DNA
tgttctgtctttggagccca

SEQ ID NO: 1460 - DNA, 20 bp, synthetic construct
  source 1..20: mol_type = other DNA
cctgttctgtctttggagcc

SEQ ID NO: 1461 - DNA, 20 bp, synthetic construct
  source 1..20: mol_type = other DNA
acctgttctgtctttggagc

SEQ ID NO: 1462 - DNA, 20 bp, synthetic construct
  source 1..20: mol_type = other DNA
agtacctgttctgtctttgg

SEQ ID NO: 1463 - DNA, 20 bp, synthetic construct
  source 1..20: mol_type = other DNA
catcactgagaagtacctgt

SEQ ID NO: 1464 - DNA, 20 bp, synthetic construct
  source 1..20: mol_type = other DNA
ctccatcactgagaagtacc

SEQ ID NO: 1465 - DNA, 20 bp, synthetic construct
  source 1..20: mol_type = other DNA
ccactctctgcatttcgaag

SEQ ID NO: 1466 - DNA, 20 bp, synthetic construct
  source 1..20: mol_type = other DNA
accactctctgcatttcgaa

SEQ ID NO: 1467 - DNA, 20 bp, synthetic construct
  source 1..20: mol_type = other DNA
gcaccactctctgcatttcg

SEQ ID NO: 1468 - DNA, 20 bp, synthetic construct
  source 1..20: mol_type = other DNA
atagcaccactctctgcatt

SEQ ID NO: 1469 - DNA, 20 bp, synthetic construct
  source 1..20: mol_type = other DNA
tatagcaccactctctgcat

SEQ ID NO: 1470 - DNA, 20 bp, synthetic construct
  source 1..20: mol_type = other DNA
acatctatagcaccactctc

SEQ ID NO: 1471 - DNA, 20 bp, synthetic construct
  source 1..20: mol_type = other DNA
tacatctatagcaccactct

SEQ ID NO: 1472 - DNA, 20 bp, synthetic construct
  source 1..20: mol_type = other DNA
tttacatctatagcaccact

SEQ ID NO: 1473 - DNA, 20 bp, synthetic construct
  source 1..20: mol_type = other DNA
ctttacatctatagcaccac

SEQ ID NO: 1474 - DNA, 20 bp, synthetic construct
  source 1..20: mol_type = other DNA
aactttacatctatagcacc

SEQ ID NO: 1475 - DNA, 20 bp, synthetic construct
  source 1..20: mol_type = other DNA
aaactttacatctatagcac

SEQ ID NO: 1476 - DNA, 20 bp, synthetic construct
  source 1..20: mol_type = other DNA
ctcccttttcagacaagaca

SEQ ID NO: 1477 - DNA, 20 bp, synthetic construct
  source 1..20: mol_type = other DNA
actcccttttcagacaagac

SEQ ID NO: 1478 - DNA, 20 bp, synthetic construct
  source 1..20: mol_type = other DNA
atcactcccttttcagacaa

SEQ ID NO: 1479 - DNA, 20 bp, synthetic construct
  source 1..20: mol_type = other DNA
taatcactcccttttcagac

SEQ ID NO: 1480 - DNA, 20 bp, synthetic construct
  source 1..20: mol_type = other DNA
ataatcactcccttttcaga

SEQ ID NO: 1481 - DNA, 20 bp, synthetic construct
  source 1..20: mol_type = other DNA
atccccattccagtttccat

SEQ ID NO: 1482 - DNA, 20 bp, synthetic construct
  source 1..20: mol_type = other DNA
gatccccattccagtttcca

SEQ ID NO: 1483 - DNA, 20 bp, synthetic construct
  source 1..20: mol_type = other DNA
gcgatccccattccagtttc

SEQ ID NO: 1484 - DNA, 20 bp, synthetic construct
  source 1..20: mol_type = other DNA
tgcgatccccattccagttt

SEQ ID NO: 1485 - DNA, 20 bp, synthetic construct
  source 1..20: mol_type = other DNA
gctgcgatccccattccagt

SEQ ID NO: 1486 - DNA, 20 bp, synthetic construct
  source 1..20: mol_type = other DNA
tgctgcgatccccattccag

SEQ ID NO: 1487 - DNA, 20 bp, synthetic construct
  source 1..20: mol_type = other DNA
tgtgctgcgatccccattcc

SEQ ID NO: 1488 - DNA, 20 bp, synthetic construct
  source 1..20: mol_type = other DNA
atgtgctgcgatccccattc

SEQ ID NO: 1489 - DNA, 20 bp, synthetic construct
  source 1..20: mol_type = other DNA
actaagttctgtctgtggaa

SEQ ID NO: 1490 - DNA, 20 bp, synthetic construct
  source 1..20: mol_type = other DNA
gaaactaagttctgtctgtg

SEQ ID NO: 1491 - DNA, 20 bp, synthetic construct
  source 1..20: mol_type = other DNA
agaaactaagttctgtctgt

SEQ ID NO: 1492 - DNA, 20 bp, synthetic construct
  source 1..20: mol_type = other DNA
tgaccctgatcttccattct

SEQ ID NO: 1493 - DNA, 20 bp, synthetic construct
  source 1..20: mol_type = other DNA
ctgaccctgatcttccattc

SEQ ID NO: 1494 - DNA, 20 bp, synthetic construct
  source 1..20: mol_type = other DNA
actctgaccctgatcttcca

SEQ ID NO: 1495 - DNA, 20 bp, synthetic construct
  source 1..20: mol_type = other DNA
atactctgaccctgatcttc

SEQ ID NO: 1496 - DNA, 20 bp, synthetic construct
  source 1..20: mol_type = other DNA
aatactctgaccctgatctt

SEQ ID NO: 1497 - DNA, 20 bp, synthetic construct
  source 1..20: mol_type = other DNA
ccatgatttcttgtctggga

SEQ ID NO: 1498 - DNA, 20 bp, synthetic construct
  source 1..20: mol_type = other DNA
ggccatgatttcttgtctgg

SEQ ID NO: 1499 - DNA, 20 bp, synthetic construct
  source 1..20: mol_type = other DNA
gggccatgatttcttgtctg

SEQ ID NO: 1500 - DNA, 20 bp, synthetic construct
  source 1..20: mol_type = other DNA
acttaagttcatctacagta

SEQ ID NO: 1501 - DNA, 20 bp, synthetic construct
  source 1..20: mol_type = other DNA
tccactgctggatggaaaaa

SEQ ID NO: 1502 - DNA, 20 bp, synthetic construct
  source 1..20: mol_type = other DNA
atattatttatcttactcaa

SEQ ID NO: 1503 - DNA, 20 bp, synthetic construct
  source 1..20: mol_type = other DNA
gttctaagtgctttatatta

SEQ ID NO: 1504 - DNA, 20 bp, synthetic construct
  source 1..20: mol_type = other DNA
aggaactaacatgtaggcac

SEQ ID NO: 1505 - DNA, 20 bp, synthetic construct
  source 1..20: mol_type = other DNA
atataagataatacatgtaa

SEQ ID NO: 1506 - DNA, 20 bp, synthetic construct
  source 1..20: mol_type = other DNA
catcatgagcctaaaggaaa

SEQ ID NO: 1507 - DNA, 20 bp, synthetic construct
  source 1..20: mol_type = other DNA
ccatcatgagcctaaaggaa

SEQ ID NO: 1508 - DNA, 20 bp, synthetic construct
  source 1..20: mol_type = other DNA
cttctgattcaagccattaa

SEQ ID NO: 1509 - DNA, 20 bp, synthetic construct
  source 1..20: mol_type = other DNA
tgcttctgattcaagccatt

SEQ ID NO: 1510 - DNA, 20 bp, synthetic construct
  source 1..20: mol_type = other DNA
gtgcttctgattcaagccat

SEQ ID NO: 1511 - DNA, 20 bp, synthetic construct
  source 1..20: mol_type = other DNA
agtgcttctgattcaagcca

SEQ ID NO: 1512 - DNA, 20 bp, synthetic construct
  source 1..20: mol_type = other DNA
aagtgcttctgattcaagcc

SEQ ID NO: 1513 - DNA, 20 bp, synthetic construct
  source 1..20: mol_type = other DNA
aaagtgcttctgattcaagc

SEQ ID NO: 1514 - DNA, 20 bp, synthetic construct
  source 1..20: mol_type = other DNA
taaagtgcttctgattcaag

SEQ ID NO: 1515 - DNA, 20 bp, synthetic construct
  source 1..20: mol_type = other DNA
ctaaagtgcttctgattcaa

SEQ ID NO: 1516 - DNA, 20 bp, synthetic construct
  source 1..20: mol_type = other DNA
actaaagtgcttctgattca

SEQ ID NO: 1517 - DNA, 20 bp, synthetic construct
  source 1..20: mol_type = other DNA
gactaaagtgcttctgattc

SEQ ID NO: 1518 - DNA, 20 bp, synthetic construct
  source 1..20: mol_type = other DNA
ggactaaagtgcttctgatt

SEQ ID NO: 1519 - DNA, 20 bp, synthetic construct
  source 1..20: mol_type = other DNA
aggactaaagtgcttctgat

SEQ ID NO: 1520 - DNA, 20 bp, synthetic construct
  source 1..20: mol_type = other DNA
caggactaaagtgcttctga

SEQ ID NO: 1521 - DNA, 20 bp, synthetic construct
  source 1..20: mol_type = other DNA
acaggactaaagtgcttctg

SEQ ID NO: 1522 - DNA, 20 bp, synthetic construct
  source 1..20: mol_type = other DNA
tacaggactaaagtgcttct

SEQ ID NO: 1523 - DNA, 20 bp, synthetic construct
  source 1..20: mol_type = other DNA
gatacaggactaaagtgctt

SEQ ID NO: 1524 - DNA, 20 bp, synthetic construct
  source 1..20: mol_type = other DNA
agatacaggactaaagtgct

SEQ ID NO: 1525 - DNA, 20 bp, synthetic construct
  source 1..20: mol_type = other DNA
cagatacaggactaaagtgc

SEQ ID NO: 1526 - DNA, 20 bp, synthetic construct
  source 1..20: mol_type = other DNA
acagatacaggactaaagtg

SEQ ID NO: 1527 - DNA, 20 bp, synthetic construct
  source 1..20: mol_type = other DNA
aacagatacaggactaaagt

SEQ ID NO: 1528 - DNA, 20 bp, synthetic construct
  source 1..20: mol_type = other DNA
gaacagatacaggactaaag

SEQ ID NO: 1529 - DNA, 20 bp, synthetic construct
  source 1..20: mol_type = other DNA
tgaacagatacaggactaaa

SEQ ID NO: 1530 - DNA, 20 bp, synthetic construct
  source 1..20: mol_type = other DNA
ctgaacagatacaggactaa

SEQ ID NO: 1531 - DNA, 20 bp, synthetic construct
  source 1..20: mol_type = other DNA
actgaacagatacaggacta

SEQ ID NO: 1532 - DNA, 20 bp, synthetic construct
  source 1..20: mol_type = other DNA
cactgaacagatacaggact

SEQ ID NO: 1533 - DNA, 20 bp, synthetic construct
  source 1..20: mol_type = other DNA
acactgaacagatacaggac

SEQ ID NO: 1534 - DNA, 20 bp, synthetic construct
  source 1..20: mol_type = other DNA
gacactgaacagatacagga

SEQ ID NO: 1535 - DNA, 20 bp, synthetic construct
  source 1..20: mol_type = other DNA
tgacactgaacagatacagg

SEQ ID NO: 1536 - DNA, 20 bp, synthetic construct
  source 1..20: mol_type = other DNA
ctgacactgaacagatacag

SEQ ID NO: 1537 - DNA, 20 bp, synthetic construct
  source 1..20: mol_type = other DNA
ggctgacactgaacagatac

SEQ ID NO: 1538 - DNA, 20 bp, synthetic construct
  source 1..20: mol_type = other DNA
aggctgacactgaacagata

SEQ ID NO: 1539 - DNA, 20 bp, synthetic construct
  source 1..20: mol_type = other DNA
aaggctgacactgaacagat

SEQ ID NO: 1540 - DNA, 20 bp, synthetic construct
  source 1..20: mol_type = other DNA
aaaggctgacactgaacaga

SEQ ID NO: 1541 - DNA, 20 bp, synthetic construct
  source 1..20: mol_type = other DNA
gaaaggctgacactgaacag

SEQ ID NO: 1542 - DNA, 20 bp, synthetic construct
  source 1..20: mol_type = other DNA
tgaaaggctgacactgaaca

SEQ ID NO: 1543 - DNA, 20 bp, synthetic construct
  source 1..20: mol_type = other DNA
aatgggatttaaaatgatgt

SEQ ID NO: 1544 - DNA, 20 bp, synthetic construct
  source 1..20: mol_type = other DNA
aaatgggatttaaaatgatg

SEQ ID NO: 1545 - DNA, 20 bp, synthetic construct
  source 1..20: mol_type = other DNA
caaatgggatttaaaatgat

SEQ ID NO: 1546 - DNA, 24 bp, synthetic construct
  source 1..24: mol_type = other DNA
ttccaatgcttactggagaagtga

SEQ ID NO: 1547 - DNA, 26 bp, synthetic construct
  source 1..26: mol_type = other DNA
ggaacactgtgtgatttcatagatga

SEQ ID NO: 1548 - DNA, 17 bp, synthetic construct
  source 1..17: mol_type = other DNA
tcctgtaatggaactgc